European Patent Specification EP 2 570 423 B1, published May 3, 2023. Title: HEPATITIS C. VIRUS NUCLEIC ACID VACCINE. Applicant: Istituto di Ricerche di Biologia Molecolare P. Angeletti S.p.A. Application PCT/EP2006/005697. The sequence listing filed with the application follows.

SEQUENCE LISTING (33 sequences)

SEQ ID NO: 1 - protein, 2675 aa, Artificial Sequence
  Chimeric HCV polypeptide
MAPITAYAQQTRGLLGTIVTSLTGRDKNVVAGEVQVLSTATQTFLGTTVGGVMWTVYHGAGSRTLAGVKHPALQMYTNVDQDLVGWPAPPGAKSLEPCTCGSADLYLVTRDADVIPARRRGDSTASLLSPRPLARLKGSSGGPVMCPSGHVAGIFRAAVCTRGVAKALQFIPVETLSTQARSPSFSDNSTPPAVPQSYQVGYLHAPTGSGKSTKVPAAYVAQGYNVLVLNPSVAATLGFGSFMSRAYGIDPNIRTGNRTVTTGAKLTYSTYGKFLAGGGCSGGAYDVIICDDCHAQDATSILGIGTVLDQAETAGVRLTVLATATPPGSITVPHSNIEEVALGSEGEIPFYGKAIPIACIKGGRHLIFCHSKKKCDKMASKLRGMGLNAVAYYRGLDVSVIPTTGDVVVCATDALMTGFTGDFDSVIDCNVAVEQYVDFSLDPTFSIETCTAPQDAVSRSQRRGRTGRGRLGTYRYVTPGERPSGMFDSVVLCECYDAGCSWYDLQPAETTVRLRAYLSTPGLPVCQDHLDLWESVFTGLTHIDAHFLSQTKQAGLNFSYLTAYQATVCARAQAPPPSWDETWKCLVRLKPTLHGPTPLLYRLGPVQNEICLTHPITKYVMACMSADLEVTTSTWVLLGGVLAAVAAYCLSVGCVVIVGHIELGGKPALVPDKEVLYQQYDEMEECSQARMAPITAYSQQTRGLLGCIITSLTGRDKNQVEGEVQVVSTATQSFLATCVNGVCWTVYHGAGSKTLAGPKGPITQMYTNVDQDLVGWQAPPGARSLTPCTCGSSDLYLVTRHADVIPVRRRGDSRGSLLSPRPVSYLKGSSGGPLLCPSGHAVGIFRAAVCTRGVAKAVDFVPVESMETTMRSPVFTDNSSPPAVPQSFQVAHLHAPTGSGKSTKVPAAYAAQGYKVLVLNPSVAATLGFGAYMSKAHGIDPNIRTGVRTITTGAPVTYSTYGKFLADGGCSGGAYDIIICDECHSTDSTTILGIGTVLDQAETAGARLVVLATATPPGSVTVPHPNIEEVALSNTGEIPFYGKAIPIEAIRGGRHLIFCHSKKKCDELAAKLSGLGINAVAYYRGLDVSVIPTIGDVVVVATDALMTGYTGDFDSVIDCNTCVTQTVDFSLDPTFTIETTTVPQDAVSRSQRRGRTGRGRRGIYRFVTPGERPSGMFDSSVLCECYDAGCAWYELTPAETSVRLRAYLNTPGLPVCQDHLEFWESVFTGLTHIDAHFLSQTKQAGDNFPYLVAYQATVCARAQAPPPSWDQMWKCLIRLKPTLHGPTPLLYRLGAVQNEVTLTHPITKYIMACMSADLEVVTSTWVLVGGVLAALAAYCLTTGSVVIVGRIILSGRPAIVPDREFLYQEFDEMEECASHLPYIEQGMQLAEQFKQKALGLLQTATKQAEAAAPVVESKWRALETFWAKHMWNFISGIQYLAGLSTLPGNPAIASLMAFTASITSPLTTQSTLLFNILGGWVAAQLAPPSAASAFVGAGIAGAAVGSIGLGKVLVDILAGYGAGVAGALVAFKVMSGEMPSTEDLVNLLPAILSPGALVVGVVCAAILRRHVGPGEGAVQWMNRLIAFASRGNHVSPTHYVPESDAAARVTQILSSLTITQLLKRLHQWINEDCSTPCSGSWLRDVWDWICTVLTDFKTWLQSKLLPQLPGVPFFSCQRGYKGVWRGDGIMQTTCPCGAQITGHVKNGSMRIVGPKTCSNTWHGTFPINAYTTGPCTPSPAPNYSRALWRVAAEEYVEVTRVGDFHYVTGMTTDNVKCPCQVPAPEFFTEVDGVRLHRYAPACRPLLREEVTFQVGLNQYLVGSQLPCEPEPDVAVLTSMLTDPSHITAETAKRRLARGSPPSLASSSASQLSAPSLKATCTTHHVSPDADLIEANLLWRQEMGGNITRVESENKVVVLDSFDPLRAEEDEREVSVPAEILRKSKKFPAAMPIWARPDYNPPLLESWKDPDYVPPVVHGCPLPPIKAPPIPPPRRKRTVVLTESSVSSALAELATKTFGSSESSAVDSGTATALPDQASDDGDKGSDVESYSSMPPLEGEPGDPDLSDGSWSTVSEEASEDVVCCSMSYTWTGALITPCAAEESKLPINALSNSLLRHHNMVYATTSRSAGLRQKKVTFDRLQVLDDHYRDVLKEMKAKASTVKAKLLSVEEACKLTPPHSAKSKFGYGAKDVRNLSSKAVNHIHSVWKDLLEDTVTPIDTTIMAKNEVFCVQPEKGGRKPARLIVFPDLGVRVCEKMALYDVVSTLPQVVMGSSYGFQYSPGQRVEFLVNTWKSKKNPMGFSYDTRCFDSTVTENDIRVEESIYQCCDLAPEARQAIKSLTERLYIGGPLTNSKGQNCGYRRCRASGVLTTSCGNTLTCYLKASAACRAAKLQDCTMLVNAAGLVVICESAGTQEDAASLRVFTEAMTRYSAPPGDPPQPEYDLELITSCSSNVSVAHDASGKRVYYLTRDPTTPLARAAWETARHTPVNSWLGNIIMYAPTLWARMILMTHFFSILLAQEQLEKALDCQIYGACYSIEPLDLPQIIERLHGLSAFSLHSYSPGEINRVASCLRKLGVPPLRVWRHRARSVRARLLSQGGRAATCGKYLFNWAVKTKLKLTPIPAASQLDLSGWFVAGYSGGDIYHSLSRARPRWFMLCLLLLSVGVGIYLLPNR

SEQ ID NO: 2 - DNA, 12939 bp, Artificial Sequence
  Plasmid containing an expression cassette encoding a chimeric HCV polypeptide
tcgcgcgtttcggtgatgacggtgaaaacctctgacacatgcagctcccggagacggtcacagcttgtctgtaagcggatgccgggagcagacaagcccgtcagggcgcgtcagcgggtgttggcgggtgtcggggctggcttaactatgcggcatcagagcagattgtactgagagtgcaccatatgcggtgtgaaataccgcacagatgcgtaaggagaaaataccgcatcagattggctattggccattgcatacgttgtatccatatcataatatgtacatttatattggctcatgtccaacattaccgccatgttgacattgattattgactagttattaatagtaatcaattacggggtcattagttcatagcccatatatggagttccgcgttacataacttacggtaaatggcccgcctggctgaccgcccaacgacccccgcccattgacgtcaataatgacgtatgttcccatagtaacgccaatagggactttccattgacgtcaatgggtggagtatttacggtaaactgcccacttggcagtacatcaagtgtatcatatgccaagtacgccccctattgacgtcaatgacggtaaatggcccgcctggcattatgcccagtacatgaccttatgggactttcctacttggcagtacatctacgtattagtcatcgctattaccatggtgatgcggttttggcagtacatcaatgggcgtggatagcggtttgactcacggggatttccaagtctccaccccattgacgtcaatgggagtttgttttggcaccaaaatcaacgggactttccaaaatgtcgtaacaactccgccccattgacgcaaatgggcggtaggcgtgtacggtgggaggtctatataagcagagctcgtttagtgaaccgtcagatcgcctggagacgccatccacgctgttttgacctccatagaagacaccgggaccgatccagcctccgcggccgggaacggtgcattggaacgcggattccccgtgccaagagtgacgtaagtaccgcctatagactctataggcacacccctttggctcttatgcatgctatactgtttttggcttggggcctatacacccccgcttccttatgctataggtgatggtatagcttagcctataggtgtgggttattgaccattattgaccactcccctattggtgacgatactttccattactaatccataacatggctctttgccacaactatctctattggctatatgccaatactctgtccttcagagactgacacggactctgtatttttacaggatggggtcccatttattatttacaaattcacatatacaacaacgccgtcccccgtgcccgcagtttttattaaacatagcgtgggatctccacgcgaatctcgggtacgtgttccggacatgggctcttctccggtagcggcggagcttccacatccgagccctggtcccatgcctccagcggctcatggtcgctcggcagctccttgctcctaacagtggaggccagacttaggcacagcacaatgcccaccaccaccagtgtgccgcacaaggccgtggcggtagggtatgtgtctgaaaatgagcgtggagattgggctcgcacggctgacgcagatggaagacttaaggcagcggcagaagaagatgcaggcagctgagttgttgtattctgataagagtcagaggtaactcccgttgcggtgctgttaacggtggagggcagtgtagtctgagcagtactcgttgctgccgcgcgcgccaccagacataatagctgacagactaacagactgttcctttccatgggtcttttctgcagtcaccgtccttagaattccgccaccatggcccctatcaccgcctatgcccagcagacaagaggcctgctgggcaccatcgtgacaagcctgaccggcagagacaagaatgtggtggccggcgaagtgcaggtgctgagcaccgccacccagacatttctgggcaccacagtgggcggcgtgatgtggacagtgtaccacggagccggctctagaacactggccggcgtgaagcaccctgccctgcagatgtataccaacgtggatcaggatcttgtggggtggcctgcccctcctggcgccaagtctctggagccttgtacctgcggcagcgccgatctgtacctggtgaccagggacgccgatgtgatccccgccagaagaagaggcgatagcaccgccagcctgctgtctccgcggccgctggccagactgaagggaagcagcggcggacctgtgatgtgtcctagcggccacgtggccggcatctttagagccgccgtgtgtacaagaggcgtggccaaggccctgcagtttatccctgtggagaccctgagcacccaggccagaagccctagcttcagcgacaacagcacccctcctgccgtgcctcagagctaccaagtgggctacctgcacgcccctacaggctctggcaagtccaccaaagtgcctgccgcctatgtggcccagggctacaatgtgctggtgctgaacccttctgtggccgccacactgggctttggcagcttcatgagcagggcctacggcatcgaccccaatatccggaccggcaacagaaccgtgacaaccggcgccaagctgacctacagcacctacggcaagttcctggccggaggaggatgtagcggcggagcctacgacgtgatcatctgcgacgattgccacgcccaggatgccacaagcatcctgggcatcgggaccgtgctggatcaggccgaaacagccggagtgagactgacagtgctggccacagccacacctcctggcagcatcacagtgccccacagcaatatcgaagaagtggccctgggcagcgagggcgagatccctttttacgggaaggccatccctatcgcctgtatcaagggcggcaggcacctgatcttctgccacagcaagaaaaagtgtgacaagatggccagcaagctgagaggcatgggcctgaatgccgtggcctactacagaggcctggacgtgtctgtgatccctaccaccggcgatgtggtggtgtgtgccaccgatgccctgatgaccggcttcaccggcgatttcgacagcgtgatcgattgcaacgtggccgtggagcagtacgtggacttcagcctggaccctacattcagcatcgagacctgcacagctcctcaggatgccgtgtcccggtctcagagaagaggcagaaccggcagaggcagactgggcacctacagatacgtgacccctggcgagagacctagcggcatgtttgacagcgtggtgctgtgcgagtgttacgatgccggctgctcctggtacgatctgcagcctgccgagaccactgtgaggctgagagcctacctgtctacccctggcctgcctgtgtgtcaggatcacctggacctgtgggagagcgtgtttaccggcctgacacacatcgacgcccactttctgagccagacaaaacaggccggcctgaacttcagctacctgaccgcctaccaggccacagtgtgtgctagagcccaggcccctcctcctagctgggatgagacctggaagtgccttgtgagactgaagccaaccctgcacggacctaccccactgctgtatagactgggccccgtgcagaacgagatctgcctgacccaccctatcaccaagtacgtgatggcctgcatgagcgctgatctggaagtgaccacctccacttgggtgctgctggggggcgtgctagccgccgtggccgcctattgtctgtctgtgggctgcgtggtgattgtgggccacatcgagctgggaggaaagcctgccctggtgcccgataaggaagtgctctaccagcagtacgacgagatggaggagtgtagccaggctagaatggcccccatcaccgcctacagccagcagacccgcggcctgctgggctgcatcatcaccagcctgaccggccgcgacaagaaccaggtggagggcgaggtgcaggtggtgagcaccgccacccagagcttcctggccacctgcgtgaacggcgtgtgctggaccgtgtaccacggcgccggcagcaagaccctggccggccccaagggccccatcacccagatgtacaccaacgtggaccaggacctggtgggctggcaggccccccccggcgcccgcagcctgaccccctgcacctgcggcagcagcgacctgtacctggtgacccgccacgccgacgtgatccccgtgcgccgccgcggcgacagccgcggcagcctgctgagcccccgccccgtgagctacctgaagggcagcagcggcggccccctgctgtgccccagcggccacgccgtgggcatcttccgcgccgccgtgtgcacccgcggcgtggccaaggccgtggacttcgtgcccgtggagagcatggagaccaccatgcgcagccccgtgttcaccgacaacagcagcccccccgccgtgccccagagcttccaggtggcccacctgcacgcccccaccggcagcggcaagagcaccaaggtgcccgccgcctacgccgcccagggctacaaggtgctggtgctgaaccccagcgtggccgccaccctgggcttcggcgcctacatgagcaaggcccacggcatcgaccccaacatccgcaccggcgtgcgcaccatcaccaccggcgcccccgtgacctacagcacctacggcaagttcctggccgacggcggctgcagcggcggcgcctacgacatcatcatctgcgacgagtgccacagcaccgacagcaccaccatcctgggcatcggcaccgtgctggaccaggccgagaccgccggcgcccgcctggtggtgctggccaccgccaccccccccggcagcgtgaccgtgccccaccccaacatcgaggaggtggccctgagcaacaccggcgagatccccttctacggcaaggccatccccatcgaggccatccgcggcggccgccacctgatcttctgccacagcaagaagaagtgcgacgagctggccgccaagctgagcggcctgggcatcaacgccgtggcctactaccgcggcctggacgtgagcgtgatccccaccatcggcgacgtggtggtggtggccaccgacgccctgatgaccggctacaccggcgacttcgacagcgtgatcgactgcaacacctgcgtgacccagaccgtggacttcagcctggaccccaccttcaccatcgagaccaccaccgtgccccaggacgccgtgagccgcagccagcgccgcggccgcaccggccgcggccgccgcggcatctaccgcttcgtgacccccggcgagcgccccagcggcatgttcgacagcagcgtgctgtgcgagtgctacgacgccggctgcgcctggtacgagctgacccccgccgagaccagcgtgcgcctgcgcgcctacctgaacacccccggcctgcccgtgtgccaggaccacctggagttctgggagagcgtgttcaccggcctgacccacatcgacgcccacttcctgagccagaccaagcaggccggcgacaacttcccctacctggtggcctaccaggccaccgtgtgcgcccgcgcccaggcccccccccccagctgggaccagatgtggaagtgcctgatccgcctgaagcccaccctgcacggccccacccccctgctgtaccgcctgggcgccgtgcagaacgaggtgaccctgacccaccccatcaccaagtacatcatggcctgcatgagcgccgacctggaggtggtgaccagcacctgggtgctggtgggcggcgtgctggccgccctggccgcctactgcctgaccaccggcagcgtggtgatcgtgggccgcatcatcctgagcggccgccccgccatcgtgcccgaccgcgagttcctgtaccaggagttcgacgagatggaggagtgcgccagccacctgccctacatcgagcagggcatgcagctggccgagcagttcaagcagaaggccctgggcctgctgcagaccgccaccaagcaggccgaggccgccgcccccgtggtggagagcaagtggcgcgccctggagaccttctgggccaagcacatgtggaacttcatcagcggcatccagtacctggccggcctgagcaccctgcccggcaaccccgccatcgccagcctgatggccttcaccgccagcatcaccagccccctgaccacccagagcaccctgctgttcaacatcctgggcggctgggtggccgcccagctggccccccccagcgccgccagcgccttcgtgggcgccggcatcgccggcgccgccgtgggcagcatcggcctgggcaaggtgctggtggacatcctggccggctacggcgccggcgtggccggcgccctggtggccttcaaggtgatgagcggcgagatgcccagcaccgaggacctggtgaacctgctgcccgccatcctgagccccggcgccctggtggtgggcgtggtgtgcgccgccatcctgcgccgccacgtgggccccggcgagggcgccgtgcagtggatgaaccgcctgatcgccttcgccagccgcggcaaccacgtgagccccacccactacgtgcccgagagcgacgccgccgcccgcgtgacccagatcctgagcagcctgaccatcacccagctgctgaagcgcctgcaccagtggatcaacgaggactgcagcaccccctgcagcggcagctggctgcgcgacgtgtgggactggatctgcaccgtgctgaccgacttcaagacctggctgcagagcaagctgctgccccagctgcccggcgtgcccttcttcagctgccagcgcggctacaagggcgtgtggcgcggcgacggcatcatgcagaccacctgcccctgcggcgcccagatcaccggccacgtgaagaacggcagcatgcgcatcgtgggccccaagacctgcagcaacacctggcacggcaccttccccatcaacgcctacaccaccggcccctgcacccccagccccgcccccaactacagccgcgccctgtggcgcgtggccgccgaggagtacgtggaggtgacccgcgtgggcgacttccactacgtgaccggcatgaccaccgacaacgtgaagtgcccctgccaggtgcccgcccccgagttcttcaccgaggtggacggcgtgcgcctgcaccgctacgcccccgcctgccgccccctgctgcgcgaggaggtgaccttccaggtgggcctgaaccagtacctggtgggcagccagctgccctgcgagcccgagcccgacgtggccgtgctgaccagcatgctgaccgaccccagccacatcaccgccgagaccgccaagcgccgcctggcccgcggcagcccccccagcctggccagcagcagcgccagccagctgagcgcccccagcctgaaggccacctgcaccacccaccacgtgagccccgacgccgacctgatcgaggccaacctgctgtggcgccaggagatgggcggcaacatcacccgcgtggagagcgagaacaaggtggtggtgctggacagcttcgaccccctgcgcgccgaggaggacgagcgcgaggtgagcgtgcccgccgagatcctgcgcaagagcaagaagttccccgccgccatgcccatctgggcccgccccgactacaacccccccctgctggagagctggaaggaccccgactacgtgccccccgtggtgcacggctgccccctgccccccatcaaggccccccccatcccccccccccgccgcaagcgcaccgtggtgctgaccgagagcagcgtgagcagcgccctggccgagctggccaccaagaccttcggcagcagcgagagcagcgccgtggacagcggcaccgccaccgccctgcccgaccaggccagcgacgacggcgacaagggcagcgacgtggagagctacagcagcatgccccccctggagggcgagcccggcgaccccgacctgagcgacggcagctggagcaccgtgagcgaggaggccagcgaggacgtggtgtgctgcagcatgagctacacctggaccggcgccctgatcaccccctgcgccgccgaggagagcaagctgcccatcaacgccctgagcaacagcctgctgcgccaccacaacatggtgtacgccaccaccagccgcagcgccggcctgcgccagaagaaggtgaccttcgaccgcctgcaggtgctggacgaccactaccgcgacgtgctgaaggagatgaaggccaaggccagcaccgtgaaggccaagctgctgagcgtggaggaggcctgcaagctgacccccccccacagcgccaagagcaagttcggctacggcgccaaggacgtgcgcaacctgagcagcaaggccgtgaaccacatccacagcgtgtggaaggacctgctggaggacaccgtgacccccatcgacaccaccatcatggccaagaacgaggtgttctgcgtgcagcccgagaagggcggccgcaagcccgcccgcctgatcgtgttccccgacctgggcgtgcgcgtgtgcgagaagatggccctgtacgacgtggtgagcaccctgccccaggtggtgatgggcagcagctacggcttccagtacagccccggccagcgcgtggagttcctggtgaacacctggaagagcaagaagaaccccatgggcttcagctacgacacccgctgcttcgacagcaccgtgaccgagaacgacatccgcgtggaggagagcatctaccagtgctgcgacctggcccccgaggcccgccaggccatcaagagcctgaccgagcgcctgtacatcggcggccccctgaccaacagcaagggccagaactgcggctaccgccgctgccgcgccagcggcgtgctgaccaccagctgcggcaacaccctgacctgctacctgaaggccagcgccgcctgccgcgccgccaagctgcaggactgcaccatgctggtgaacgccgccggcctggtggtgatctgcgagagcgccggcacccaggaggacgccgccagcctgcgcgtgttcaccgaggccatgacccgctacagcgccccccccggcgaccccccccagcccgagtacgacctggagctgatcaccagctgcagcagcaacgtgagcgtggcccacgacgccagcggcaagcgcgtgtactacctgacccgcgaccccaccacccccctggcccgcgccgcctgggagaccgcccgccacacccccgtgaacagctggctgggcaacatcatcatgtacgcccccaccctgtgggcccgcatgatcctgatgacccacttcttcagcatcctgctggcccaggagcagctggagaaggccctggactgccagatctacggcgcctgctacagcatcgagcccctggacctgccccagatcatcgagcgcctgcacggcctgagcgccttcagcctgcacagctacagccccggcgagatcaaccgcgtggccagctgcctgcgcaagctgggcgtgccccccctgcgcgtgtggcgccaccgcgcccgcagcgtgcgcgcccgcctgctgagccagggcggccgcgccgccacctgcggcaagtacctgttcaactgggccgtgaagaccaagctgaagctgacccccatccccgccgccagccagctggacctgagcggctggttcgtggccggctacagcggcggcgacatctaccacagcctgagccgcgcccgcccccgctggttcatgctgtgcctgctgctgctgagcgtgggcgtgggcatctacctgctgcccaaccgctaaatttaaatgtttaaacgtcgacagcggccgcgatctgctgtgccttctagttgccagccatctgttgtttgcccctcccccgtgccttccttgaccctggaaggtgccactcccactgtcctttcctaataaaatgaggaaattgcatcgcattgtctgagtaggtgtcattctattctggggggtggggtggggcaggacagcaagggggaggattgggaagacaatagcaggcatgctggggatgcggtgggctctatggccgcagcggccaggtgctgaagaattgacccggttcctcctgggccagaaagaagcaggcacatccccttctctgtgacacaccctgtccacgcccctggttcttagttccagccccactcataggacactcatagctcaggagggctccgccttcaatcccacccgctaaagtacttggagcggtctctccctccctcatcagcccaccaaaccaaacctagcctccaagagtgggaagaaattaaagcaagataggctattaagtgcagagggagagaaaatgcctccaacatgtgaggaagtaatgagagaaatcatagaatttcttccgcttcctcgctcactgactcgctgcgctcggtcgttcggctgcggcgagcggtatcagctcactcaaaggcggtaatacggttatccacagaatcaggggataacgcaggaaagaacatgtgagcaaaaggccagcaaaaggccaggaaccgtaaaaaggccgcgttgctggcgtttttccataggctccgcccccctgacgagcatcacaaaaatcgacgctcaagtcagaggtggcgaaacccgacaggactataaagataccaggcgtttccccctggaagctccctcgtgcgctctcctgttccgaccctgccgcttaccggatacctgtccgcctttctcccttcgggaagcgtggcgctttctcatagctcacgctgtaggtatctcagttcggtgtaggtcgttcgctccaagctgggctgtgtgcacgaaccccccgttcagcccgaccgctgcgccttatccggtaactatcgtcttgagtccaacccggtaagacacgacttatcgccactggcagcagccactggtaacaggattagcagagcgaggtatgtaggcggtgctacagagttcttgaagtggtggcctaactacggctacactagaagaacagtatttggtatctgcgctctgctgaagccagttaccttcggaaaaagagttggtagctcttgatccggcaaacaaaccaccgctggtagcggtggtttttttgtttgcaagcagcagattacgcgcagaaaaaaaggatctcaagaagatcctttgatcttttctacggggtctgacgctcagtggaacgaaaactcacgttaagggattttggtcatgagattatcaaaaaggatcttcacctagatccttttaaattaaaaatgaagttttaaatcaatctaaagtatatatgagtaaacttggtctgacagttaccaatgcttaatcagtgaggcacctatctcagcgatctgtctatttcgttcatccatagttgcctgactcggggggggggggcgctgaggtctgcctcgtgaagaaggtgttgctgactcataccaggcctgaatcgccccatcatccagccagaaagtgagggagccacggttgatgagagctttgttgtaggtggaccagttggtgattttgaacttttgctttgccacggaacggtctgcgttgtcgggaagatgcgtgatctgatccttcaactcagcaaaagttcgatttattcaacaaagccgccgtcccgtcaagtcagcgtaatgctctgccagtgttacaaccaattaaccaattctgattagaaaaactcatcgagcatcaaatgaaactgcaatttattcatatcaggattatcaataccatatttttgaaaaagccgtttctgtaatgaaggagaaaactcaccgaggcagttccataggatggcaagatcctggtatcggtctgcgattccgactcgtccaacatcaatacaacctattaatttcccctcgtcaaaaataaggttatcaagtgagaaatcaccatgagtgacgactgaatccggtgagaatggcaaaagcttatgcatttctttccagacttgttcaacaggccagccattacgctcgtcatcaaaatcactcgcatcaaccaaaccgttattcattcgtgattgcgcctgagcgagacgaaatacgcgatcgctgttaaaaggacaattacaaacaggaatcgaatgcaaccggcgcaggaacactgccagcgcatcaacaatattttcacctgaatcaggatattcttctaatacctggaatgctgttttcccggggatcgcagtggtgagtaaccatgcatcatcaggagtacggataaaatgcttgatggtcggaagaggcataaattccgtcagccagtttagtctgaccatctcatctgtaacatcattggcaacgctacctttgccatgtttcagaaacaactctggcgcatcgggcttcccatacaatcgatagattgtcgcacctgattgcccgacattatcgcgagcccatttatacccatataaatcagcatccatgttggaatttaatcgcggcctcgagcaagacgtttcccgttgaatatggctcataacaccccttgtattactgtttatgtaagcagacagttttattgttcatgatgatatatttttatcttgtgcaatgtaacatcagagattttgagacacaacgtggctttccccccccccccattattgaagcatttatcagggttattgtctcatgagcggatacatatttgaatgtatttagaaaaataaacaaataggggttccgcgcacatttccccgaaaagtgccacctgacgtctaagaaaccattattatcatgacattaacctataaaaataggcgtatcacgaggccctttcgtc

SEQ ID NO: 3 - protein, 543 aa, Chimpanzee adenovirus type 3
MKRTKTSDESFNPVYPYDTESGPPSVPFLTPPFVSPDGFQESPPGVLSLNLAEPLVTSHGMLALKMGSGLSLDDAGNLTSQDITTASPPLKKTKTNLSLETSSPLTVSTSGALTVAAAAPLAVAGTSLTMQSEAPLTVQDAKLTLATKGPLTVSEGKLALQTSAPLTAADSSTLTVSATPPINVSSGSLGLDMEDPMYTHDGKLGIRIGGPLRVVDSLHTLTVVTGNGLTVDNNALQTRVTGALGYDTSGNLQLRAAGGMRIDANGQLILNVAYPFDAQNNLSLRLGQGPLYINTDHNLDLNCNRGLTTTTTNNTKKLETKISSGLDYDTNGAVIIKLGTGLSFDNTGALTVGNTGDDKLTLWTTPDPSPNCRIHSDKDCKFTLVLTKCGSQILASVAALAVSGNLASITGTVASVTIFLRFDQNGVLMENSSLDRQYWNFRNGNSTNAAPYTNAVGFMPNLAAYPKTQSQTAKNNIVSQVYLNGDKSKPMTLTITLNGTNESSETSQVSHYSMSFTWAWESGQYATETFATNSFTFSYIAEQ

SEQ ID NO: 4 - DNA, 1683 bp, Chimpanzee adenovirus type 3
atgtcagattcttgctcctgtccctccgcacccactatcttcatgttgttgcagatgaagcgcaccaaaacgtctgacgagagcttcaaccccgtgtacccctatgacacggaaagcggccctccctccgtccctttcctcacccctcccttcgtgtctcccgatggattccaagaaagcccccccggggtcctgtctctgaacctggccgagcccctggtcacttcccacggcatgctcgccctgaaaatgggaagtggcctctccctggacgacgctggcaacctcacctctcaagatatcaccaccgctagccctcccctcaaaaaaaccaagaccaacctcagcctagaaacctcatcccccctaactgtaagcacctcaggcgccctcaccgtagcagccgccgctcccctggcagtggccggcacctccctcaccatgcaatcagaggcccccctgacagtacaggatgcaaaactcaccctggccaccaaaggccccctgaccgtgtctgaaggcaaactggccttgcaaacatcggccccgctgacggccgctgacagcagcaccctcaccgttagcgccacaccaccaattaatgtaagcagtggaagtttaggcttagacatggaagaccctatgtatactcacgatggaaaactgggaataagaattgggggtccactaagagtagtagacagcttgcacacactcactgtagttaccggaaatggactaactgtagataacaatgccctccaaactagagttacgggcgccctaggttatgacacatcaggaaatctacaattgagagctgcaggaggtatgcgaattgatgcaaatggccaacttatccttaatgtggcatacccatttgatgctcagaacaatctcagccttagacttggtcagggacccctgtatataaacacagaccacaacctggatttgaattgcaacagaggtctaaccacaactaccaccaacaacacaaaaaaacttgagactaaaattagctcaggcttagactatgacaccaatggtgctgtcattattaaacttggcactggtctaagcttcgacaacacaggcgccctaactgtgggaaacactggtgatgataaactgactctgtggacgaccccagacccatctccaaattgcagaattcactcagacaaagactgcaagtttactctagtcctaactaagtgtggaagccaaatcctggcctctgtcgccgccctagcggtatcaggaaatctggcttcgataacaggcaccgttgccagcgttaccatctttctcagatttgatcagaatggagtgcttatggaaaactcctcgctagacaggcagtactggaacttcagaaatggcaactcaactaacgctgccccctacaccaatgcagttgggttcatgccaaacctcgcagcataccccaaaacgcaaagccagactgctaaaaacaacattgtaagtcaggtttacttgaatggagacaaatccaaacccatgacccttaccatcaccctcaatggaactaatgaatccagtgaaactagccaggtgagtcactactccatgtcatttacatgggcttgggaaagtgggcaatatgccactgaaacctttgccaccaactccttcaccttttcttacattgctgaacaa

SEQ ID NO: 5 - protein, 960 aa, Chimpanzee adenovirus type 3
MATPSMMPQWSYMHISGQDASEYLSPGLVQFARATESYFSLSNKFRNPTVAPTHDVTTDRSQRLTLRFIPVDREDTAYSYKARFTLAVGDNRVLDMASTYFDIRGVLDRGPTFKPYSGTAYNSLAPKGAPNSCEWEQEETQAVEEAAEEEEEDADGQAEEEQAATKKTHVYAQAPLSGEKISKDGLQIGTDATATEQKPIYADPTFQPEPQIGESQWNEADATVAGGRVLKKSTPMKPCYGSYARPTNANGGQGVLTANAQGQLESQVEMQFFSTSENARNEANNIQPKLVLYSEDVHMETPDTHLSYKPAKSDDNSKIMLGQQSMPNRPNYIGFRDNFIGLMYYNSTGNMGVLAGQASQLNAVVDLQDRNTELSYQLLLDSMGDRTRYFSMWNQAVDSYDPDVRIIENHGTEDELPNYCFPLGGIGVTDTYQAVKTNNGNNGGQVTWTKDETFADRNEIGVGNNFAMEINLSANLWRNFLYSNVALYLPDKLKYNPSNVDISDNPNTYDYMNKRVVAPGLVDCYINLGARWSLDYMDNVNPFNHHRNAGLRYRSMLLGNGRYVPFHIQVPQKFFAIKNLLLLPGSYTYEWNFRKDVNMVLQSSLGNDLRVDGASIKFESICLYATFFPMAHNTASTLEAMLRNDTNDQSFNDYLSAANMLYPIPANATNVPISIPSRNWAAFRGWAFTRLKTKETPSLGSGFDPYYTYSGSIPYLDGTFYLNHTFKKVSVTFDSSVSWPGNDRLLTPNEFEIKRSVDGEGYNVAQCNMTKDWFLVQMLANYNIGYQGFYIPESYKDRMYSFFRNFQPMSRQVVDQTKYKDYQEVGIIHQHNNSGFVGYLAPTMREGQAYPANFPYPLIGKTAVDSITQKKFLCDRTLWRIPFSSNFMSMGALSDLGQNLLYANSAHALDMTFEVDPMDEPTLLYVLFEVFDVVRVHQPHRGVIETVYLRTPFSAGNATT

SEQ ID NO: 6 - DNA, 2880 bp, Chimpanzee adenovirus type 3
atggcgaccccatcgatgatgccgcagtggtcgtacatgcacatctcgggccaggacgcctcggagtacctgagccccgggctggtgcagttcgcccgcgccaccgagagctacttcagcctgagtaacaagtttaggaaccccacggtggcgcccacgcacgatgtgaccaccgaccggtctcagcgcctgacgctgcggttcattcccgtggaccgcgaggacaccgcgtactcgtacaaggcgcggttcaccctggccgtgggcgacaaccgcgtgctggacatggcctccacctactttgacatccgcggggtgctggaccggggtcccactttcaagccctactctggcaccgcctacaactccctggcccccaagggcgctcccaactcctgcgagtgggagcaagaggaaactcaggcagttgaagaagcagcagaagaggaagaagaagatgctgacggtcaagctgaggaagagcaagcagctaccaaaaagactcatgtatatgctcaggctcccctttctggcgaaaaaattagtaaagatggtctgcaaataggaacggacgctacagctacagaacaaaaacctatttatgcagaccctacattccagcccgaaccccaaatcggggagtcccagtggaatgaggcagatgctacagtcgccggcggtagagtgctaaagaaatctactcccatgaaaccatgctatggttcctatgcaagacccacaaatgctaatggaggtcagggtgtactaacggcaaatgcccagggacagctagaatctcaggttgaaatgcaattcttttcaacttctgaaaacgcccgtaacgaggctaacaacattcagcccaaattggtgctgtatagtgaggatgtgcacatggagaccccggatacgcacctttcttacaagcccgcaaaaagcgatgacaattcaaaaatcatgctgggtcagcagtccatgcccaacagacctaattacatcggcttcagagacaactttatcggcctcatgtattacaatagcactggcaacatgggagtgcttgcaggtcaggcctctcagttgaatgcagtggtggacttgcaagacagaaacacagaactgtcctaccagctcttgcttgattccatgggtgacagaaccagatacttttccatgtggaatcaggcagtggacagttatgacccagatgttagaattattgaaaatcatggaactgaagacgagctccccaactattgtttccctctgggtggcataggggtaactgacacttaccaggctgttaaaaccaacaatggcaataacgggggccaggtgacttggacaaaagatgaaacttttgcagatcgcaatgaaataggggtgggaaacaatttcgctatggagatcaacctcagtgccaacctgtggagaaacttcctgtactccaacgtggcgctgtacctaccagacaagcttaagtacaacccctccaatgtggacatctctgacaaccccaacacctacgattacatgaacaagcgagtggtggccccggggctggtggactgctacatcaacctgggcgcgcgctggtcgctggactacatggacaacgtcaaccccttcaaccaccaccgcaatgcgggcctgcgctaccgctccatgctcctgggcaacgggcgctacgtgcccttccacatccaggtgccccagaagttctttgccatcaagaacctcctcctcctgccgggctcctacacctacgagtggaacttcaggaaggatgtcaacatggtcctccagagctctctgggtaacgatctcagggtggacggggccagcatcaagttcgagagcatctgcctctacgccaccttcttccccatggcccacaacacggcctccacgctcgaggccatgctcaggaacgacaccaacgaccagtccttcaatgactacctttccgccgccaacatgctctaccccatacccgccaacgccaccaacgtccccatctccatcccctcgcgcaactgggcggccttccgcggctgggccttcacccgcctcaagaccaaggagaccccctccctgggctcgggattcgacccctactacacctactcgggctctattccctacctggacggcaccttctacctcaaccacactttcaagaaggtctcggtcaccttcgactcctcggtcagctggccgggcaacgaccgtctgctcacccccaacgagttcgagatcaagcgctcggtcgacggggaaggctacaacgtggcccagtgcaacatgaccaaggactggttcctggtccagatgctggccaactacaacatcggctaccagggcttctacatcccagagagctacaaggacaggatgtactccttcttcaggaacttccagcccatgagccggcaggtggtggaccagaccaagtacaaggactaccaggaggtgggcatcatccaccagcacaacaactcgggcttcgtgggctacctcgcccccaccatgcgcgagggacaggcctaccccgccaacttcccctacccgctcataggcaagaccgcggtcgacagcatcacccagaaaaagttcctctgcgaccgcaccctctggcgcatccccttctccagcaacttcatgtccatgggtgcgctctcggacctgggccagaacttgctctacgccaactccgcccacgccctcgacatgaccttcgaggtcgaccccatggacgagcccacccttctctatgttctgttcgaagtctttgacgtggtccgggtccaccagccgcaccgcggcgtcatcgagaccgtgtacctgcgtacgcccttctcggccggcaacgccaccacc

SEQ ID NO: 7 - protein, 593 aa, Chimpanzee adenovirus type 3
MRRAAMYQEGPPPSYESVVGAAAAAPSSPFASQLLEPPYVPPRYLRPTGGRNSIRYSELAPLFDTTRVYLVDNKSADVASLNYQNDHSNFLTTVIQNNDYSPSEASTQTINLDDRSHWGGDLKTILHTNMPNVNEFMFTNKFKARVMVSRSHTKEDRVELKYEWVEFELPEGNYSETMTIDLMNNAIVEHYLKVGRQNGVLESDIGVKFDTRNFRLGLDPVTGLVMPGVYTNEAFHPDIILLPGCGVDFTYSRLSNLLGIRKRQPFQEGFRITYEDLEGGNIPALLDVEAYQDSLKENEAGQEDTTPAASAAAEQGEDAADTAAADGAEADPAMVVEAPEQEEDMNDSAVRGDTFVTRGEEKQAEAEAAAEEKQLAAAAAAAALAAAEAESEGTKPAKEPVIKPLTEDSKKRSYNLLKDSTNTAYRSWYLAYNYGDPSTGVRSWTLLCTPDVTCGSEQVYWSLPDMMQDPVTFRSTRQVSNFPVVGAELLPVHSKSFYNDQAVYSQLIRQFTSLTHVFNRFPENQILARPPAPTITTVSENVPALTDHGTLPLRNSIGGVQRVTVTDARRRTCPYVYKALGIVSPRVLSSRTF

SEQ ID NO: 8 - DNA, 1779 bp, Chimpanzee adenovirus type 3
atgcggcgcgcggcgatgtaccaggagggacctcctccctcttacgagagcgtggtgggcgcggcggcggcggcgccctcttctccctttgcgtcgcagctgctggagccgccgtacgtgcctccgcgctacctgcggcctacgggggggagaaacagcatccgttactcggagctggcgcccctgttcgacaccacccgggtgtacctggtggacaacaagtcggcggacgtggcctccctgaactaccagaacgaccacagcaattttttgaccacggtcatccagaacaatgactacagcccgagcgaggccagcacccagaccatcaatctggatgaccggtcgcactggggcggcgacctgaaaaccatcctgcacaccaacatgcccaacgtgaacgagttcatgttcaccaataagttcaaggcgcgggtgatggtgtcgcgctcgcacaccaaggaagaccgggtggagctgaagtacgagtgggtggagttcgagctgccagagggcaactactccgagaccatgaccattgacctgatgaacaacgcgatcgtggagcactatctgaaagtgggcaggcaaaacggggtcctggagagcgacatcggggtcaagttcgacaccaggaacttccgcctggggctggaccccgtgaccgggctggttatgcccggggtgtacaccaacgaggccttccatcccgacatcatcctgctgcccggctgcggggtggacttcacttacagccgcctgagcaacctcctgggcatccgcaagcggcagcccttccaggagggcttcaggatcacctacgaggacctggaggggggcaacatccccgcgctcctcgatgtggaggcctaccaggatagcttgaaggaaaatgaggcgggacaggaggataccacccccgccgcctccgccgccgccgagcagggcgaggatgctgctgacaccgcggccgcggacggggcagaggccgaccccgctatggtggtggaggctcccgagcaggaggaggatatgaatgacagtgcggtgcgcggagacaccttcgtcacccggggggaggaaaagcaagcggaggccgaggccgcggccgaggaaaagcaactggcggcagcagcggcggcggcggcgttggccgcggcggaggctgagtctgaggggaccaagcccgccaaggagcccgtgattaagcccctgaccgaagatagcaagaagcgcagttacaacctgctcaaggacagcaccaacaccgcgtaccgcagctggtacctggcctacaactacggcgacccgtcgacgggggtgcgctcctggaccctgctgtgcacgccggacgtgacctgcggctcggagcaggtgtactggtcgctgcccgacatgatgcaagaccccgtgaccttccgctccacgcggcaggtcagcaacttcccggtggtgggcgccgagctgctgcccgtgcactccaagagcttctacaacgaccaggccgtctactcccagctcatccgccagttcacctctctgacccacgtgttcaatcgctttcctgagaaccagattctggcgcgcccgcccgcccccaccatcaccaccgtcagtgaaaacgttcctgctctcacagatcacgggacgctaccgctgcgcaacagcatcggaggagtccagcgagtgaccgttactgacgccagacgccgcacctgcccctacgtttacaaggccttgggcatagtctcgccgcgcgtcctttccagccgcactttt

SEQ ID NO: 9 - protein, 425 aa, Chimpanzee adenovirus type 63
MSKKRVRVDDDFDPVYPYDADNAPTVPFINPPFVSSDGFQEKPLGVLSLRLADPVTTKNGEITLKLGEGVDLDSSGKLISNTATKAAAPLSFSNNTISLNMDHPFYTKDGKLSLQVSPPLNILRTSILNTLALGFGSGLGLRGSALAVQLVSPLTFDTDGNIKLTLDRGLHVTTGDAIESNISWAKGLKFEDGAIATNIGNGLEFGSSSTETGVDDAYPIQVKLGSGLSFDSTGAIMAGNKEDDKLTLWTTPDPSPNCQILAENDAKLTLCLTKCGSQILATVSVLVVGSGNLNPITGTVSSAQVFLRFDANGVLLTEHSTLKKYWGYRQGDSIDGTPYTNAVGFMPNLKAYPKSQSSTTKNNIVGQVYMNGDVSKPMLLTITLNGTDDSNSTYSMSFSYTWTNGSYVGATFGANSYTFSYIAQE

SEQ ID NO: 10 - DNA, 1278 bp, Chimpanzee adenovirus type 63
atgtccaaaaagcgcgtccgggtggatgatgacttcgaccccgtctacccctacgatgcagacaacgcaccgaccgtgcccttcatcaacccccccttcgtctcttcagatggattccaagagaagcccctgggggtgctgtccctgcgactggccgaccccgtcaccaccaagaacggggaaatcaccctcaagctgggagagggggtggacctcgactcctcgggaaaactcatctccaacacggccaccaaggccgccgcccctctcagtttttccaacaacaccatttcccttaacatggatcaccccttttacactaaagatggaaaattatccttacaagtttctccaccattaaatatactgagaacaagcattctaaacacactagctttaggttttggatcaggtttaggactccgtggctctgccttggcagtacagttagtctctccacttacatttgatactgatggaaacataaagcttaccttagacagaggtttgcatgttacaacaggagatgcaattgaaagcaacataagctgggctaaaggtttaaaatttgaagatggagccatagcaaccaacattggaaatgggttagagtttggaagcagtagtacagaaacaggtgttgatgatgcttacccaatccaagttaaacttggatctggccttagctttgacagtacaggagccataatggctggtaacaaagaagacgataaactcactttgtggacaacacctgatccatcgccaaactgtcaaatactcgcagaaaatgatgcaaaactaacactttgcttgactaaatgtggtagtcaaatactggccactgtgtcagtcttagttgtaggaagtggaaacctaaaccccattactggcaccgtaagcagtgctcaggtgtttctacgttttgatgcaaacggtgttcttttaacagaacattctacactaaaaaaatactgggggtataggcagggagatagcatagatggcactccatataccaatgctgtaggattcatgcccaatttaaaagcttatccaaagtcacaaagttctactactaaaaataatatagtagggcaagtatacatgaatggagatgtttcaaaacctatgcttctcactataaccctcaatggtactgatgacagcaacagtacatattcaatgtcattttcatacacctggactaatggaagctatgttggagcaacatttggggctaactcttataccttctcatacatcgcccaagaatga

SEQ ID NO: 11 - protein, 941 aa, Chimpanzee adenovirus type 63
MATPSMLPQWAYMHIAGQDASEYLSPGLVQFARATDTYFSLGNKFRNPTVAPTHDVTTDRSQRLTLRFVPVDREDNTYSYKVRYTLAVGDNRVLDMASTYFDIRGVLDRGPSFKPYSGTAYNSLAPKGAPNTSQWKDSDSKMHTFGVAAMPGVVGKKIEADGLPIGIDSSSGTDTIIYADKTFQPEPQVGSDSWVDTNGAEEKYGGRALKDTTNMKPCYGSFARPTNKEGGQANIKDSETASTTPNYDIDLAFFDSKNIAANYDPDIVMYTENVELQTPDTHIVFKPGTSDESSEANLGQQAMPNRPNYIGFRDNFIGLMYYNSTGNMGVLAGQASQLNAVVDLQDRNTELSYQLLLDSLGDRTRYFSMWNQAVDSYDPDVRIIENHGVEDELPNYCFPLNGVGFTDTYQGVKVKTDTAATGTNGTQWDKDDTTVSTANEIHSGNPFAMEINIQANLWRNFLYANVALYLPDSYKYTPANITLPTNTNTYDYMNGRVVAPSLVDAYINIGARWSLDPMDNVNPFNHHRNAGLRYRSMLLGNGRYVPFHIQVPQKFFAIKSLLLLPGSYTYEWNFRKDVNMILQSSLGNDLRTDGASIAFTSINLYATFFPMAHNTASTLEAMLRNDTNDQSFNDYLSAANMLYPIPANATNVPISIPSRNWAAFRGWSFTRLKTRETPSLGSGFDPYFVYSGSIPYLDGTFYLNHTFKKVSITFDSSVSWPGNDRLLTPNEFEIKRTVDGEGYNVAQCNMTKDWFLVQMLAHYNIGYQGFYVPEGYKDRMYSFFRNFQPMSRQVVDEVNYKDYQAVTLAYQHNNSGFVGYLAPTMRQGQPYPANYPYPLIGKSAVASVTQKKFLCDRVMWRIPFSSNFMSMGALTDLGQNMLYANSAHALDMNFEVDPMDESTLLYVVFEVFDVVRVHQPHRGVIEAVYLRTPFSAGNATT

SEQ ID NO: 12 - DNA, 2877 bp, Chimpanzee adenovirus type 63
atgtatgtccgccgaccagaaggaggaagaggcgcgtcgccgagttgcaagatggccaccccatcgatgctgccccagtgggcgtacatgcacatcgccggacaggacgcttcggagtacctgagtccgggtctggtgcagttcgcccgcgccacagacacctacttcagtctggggaacaagtttaggaaccccacggtggcgcccacgcacgatgtgaccaccgaccgcagccagcggctgacgctgcgcttcgtgcccgtggaccgcgaggacaacacctactcgtacaaagtgcgctacacgctggccgtgggcgacaaccgcgtgctggacatggccagcacctactttgacatccgcggcgtgctggatcggggccccagcttcaaaccctactccggcaccgcctacaacagcctagctcccaagggagcgcccaacacctcacagtggaaggattccgacagcaaaatgcatacttttggagttgctgccatgcccggtgttgttggtaaaaaaatagaagccgatggtctgcctattggaatagattcatcctctggaactgacaccataatttatgctgataaaactttccaaccagagccacaggttggaagtgacagttgggtcgacaccaatggtgcagaggaaaaatatggaggtagagctcttaaggacactacaaacatgaagccctgctacggttcttttgccaggcctaccaacaaagaaggtggacaggctaacataaaagattctgaaactgccagcactactcctaactatgatatagatttggcattctttgacagcaaaaatattgcagctaactacgatccagatattgtaatgtacacagaaaatgttgagttgcaaactccagatactcatattgtgtttaagccaggaacttcagatgaaagttcagaagccaatttgggccagcaggccatgcccaacagacccaactacatcgggttcagagacaactttatcgggctcatgtactacaacagcactggcaatatgggtgtactggctggtcaggcctcccagctaaatgctgtggtggacttgcaggacagaaacaccgaactgtcctaccagctcttgcttgactctctgggtgacagaaccaggtatttcagtatgtggaatcaggcggtggacagctatgaccccgatgtgcgcattattgaaaatcacggtgtggaggatgaactccccaattattgcttccctttgaatggtgtaggctttacagatacttaccagggtgttaaagttaagacagatacagccgctactggtaccaatggaacgcagtgggacaaagatgataccacagtcagcactgccaatgagatccactcaggcaatcctttcgccatggagatcaacatccaggccaacctgtggcggaacttcctctacgcgaacgtggcgctgtacctgcccgactcctacaagtacacgccggccaacatcacgctgccgaccaacaccaacacctacgattacatgaacggccgcgtggtggcgccctcgctggtggacgcctacatcaacatcggggcgcgctggtcgctggaccccatggacaacgtcaaccccttcaaccaccaccgcaacgcgggcctgcgctaccgctccatgctcctgggcaacgggcgctacgtgcccttccacatccaggtgccccaaaagtttttcgccatcaagagcctcctgctcctgcccgggtcctacacctacgagtggaacttccgcaaggacgtcaacatgatcctgcagagctccctcggcaacgacctgcgcacggacggggcctccatcgccttcaccagcatcaacctctacgccaccttcttccccatggcgcacaacaccgcctccacgctcgaggccatgctgcgcaacgacaccaacgaccagtccttcaacgactacctctcggcggccaacatgctctaccccatcccggccaacgccaccaacgtgcccatctccatcccctcgcgcaactgggccgccttccgcggatggtccttcacgcgcctcaagacccgcgagacgccctcgctcggctccgggttcgacccctacttcgtctactcgggctccatcccctacctcgacggcaccttctacctcaaccacaccttcaagaaggtctccatcaccttcgactcctccgtcagctggcccggcaacgaccgcctcctgacgcccaacgagttcgaaatcaagcgcaccgtcgacggagagggatacaacgtggcccagtgcaacatgaccaaggactggttcctggtccagatgctggcccactacaacatcggctaccagggcttctacgtgcccgagggctacaaggaccgcatgtactccttcttccgcaacttccagcccatgagccgccaggtcgtggacgaggtcaactacaaggactaccaggccgtcaccctggcctaccagcacaacaactcgggcttcgtcggctacctcgcgcccaccatgcgccagggccagccctaccccgccaactacccctacccgctcatcggcaagagcgccgtcgccagcgtcacccagaaaaagttcctctgcgaccgggtcatgtggcgcatccccttctccagcaacttcatgtccatgggcgcgctcaccgacctcggccagaacatgctctacgccaactccgcccacgcgctagacatgaatttcgaagtcgaccccatggatgagtccacccttctctatgttgtcttcgaagtcttcgacgtcgtccgagtgcaccagccccaccgcggcgtcatcgaggccgtctacctgcgcacgcccttctcggccggcaacgccaccacctaa

SEQ ID NO: 13 - DNA, 35890 bp, Artificial Sequence
  ChAd3 delta E1,3,4, Ad5 E4orf6, NSmut
catcatcaataatataccttattttggattgaagccaatatgataatgagatgggcggcgcgaggcggggcgcggggcgggaggcgggtttgggggcgggccggcgggcggggcggtgtggcggaagtggactttgtaagtgtggcggatgtgacttgctagtgccgggcgcggtaaaagtgacgttttccgtgcgcgacaacgcccccgggaagtgacatttttcccgcggtttttaccggatgttgtagtgaatttgggcgtaaccaagtaagatttggccattttcgcgggaaaactgaaacggggaagtgaaatctgattaattttgcgttagtcataccgcgtaatatttgtctagggccgagggactttggccgattacgtggaggactcgcccaggtgttttttgaggtgaatttccgcgttccgggtcaaagtctccgttttattattataggatatcccattgcatacgttgtatccatatcataatatgtacatttatattggctcatgtccaacattaccgccatgttgacattgattattgactagttattaatagtaatcaattacggggtcattagttcatagcccatatatggagttccgcgttacataacttacggtaaatggcccgcctggctgaccgcccaacgacccccgcccattgacgtcaataatgacgtatgttcccatagtaacgccaatagggactttccattgacgtcaatgggtggagtatttacggtaaactgcccacttggcagtacatcaagtgtatcatatgccaagtacgccccctattgacgtcaatgacggtaaatggcccgcctggcattatgcccagtacatgaccttatgggactttcctacttggcagtacatctacgtattagtcatcgctattaccatggtgatgcggttttggcagtacatcaatgggcgtggatagcggtttgactcacggggatttccaagtctccaccccattgacgtcaatgggagtttgttttggcaccaaaatcaacgggactttccaaaatgtcgtaacaactccgccccattgacgcaaatgggcggtaggcgtgtacggtgggaggtctatataagcagagctcgtttagtgaaccgtcagatcgcctggagacgccatccacgctgttttgacctccatagaagacaccgggaccgatccagcctccgcggccgggaacggtgcattggaacgcggattccccgtgccaagagtgagatctgccaccatggcgcccatcacggcctactcccaacagacgcggggcctacttggttgcatcatcactagccttacaggccgggacaagaaccaggtcgagggagaggttcaggtggtttccaccgcaacacaatccttcctggcgacctgcgtcaacggcgtgtgttggaccgtttaccatggtgctggctcaaagaccttagccggcccaaaggggccaatcacccagatgtacactaatgtggaccaggacctcgtcggctggcaggcgccccccggggcgcgttccttgacaccatgcacctgtggcagctcagacctttacttggtcacgagacatgctgacgtcattccggtgcgccggcggggcgacagtagggggagcctgctctcccccaggcctgtctcctacttgaagggctcttcgggtggtccactgctctgcccttcggggcacgctgtgggcatcttccgggctgccgtatgcacccggggggttgcgaaggcggtggactttgtgcccgtagagtccatggaaactactatgcggtctccggtcttcacggacaactcatcccccccggccgtaccgcagtcatttcaagtggcccacctacacgctcccactggcagcggcaagagtactaaagtgccggctgcatatgcagcccaagggtacaaggtgctcgtcctcaatccgtccgttgccgctaccttagggtttggggcgtatatgtctaaggcacacggtattgaccccaacatcagaactggggtaaggaccattaccacaggcgcccccgtcacatactctacctatggcaagtttcttgccgatggtggttgctctgggggcgcttatgacatcataatatgtgatgagtgccattcaactgactcgactacaatcttgggcatcggcacagtcctggaccaagcggagacggctggagcgcggcttgtcgtgctcgccaccgctacgcctccgggatcggtcaccgtgccacacccaaacatcgaggaggtggccttgtctaatactggagagatccccttctatggcaaagccatccccattgaagccatcagggggggaaggcatctcattttctgtcattccaagaagaagtgcgacgagctcgccgcaaagctgtcaggcctcggaatcaacgctgtggcgtattaccgggggctcgatgtgtccgtcataccaactatcggagacgtcgttgtcgtggcaacagacgctctgatgacgggctatacgggcgactttgactcagtgatcgactgtaacacatgtgtcacccagacagtcgacttcagcttggatcccaccttcaccattgagacgacgaccgtgcctcaagacgcagtgtcgcgctcgcagcggcggggtaggactggcaggggtaggagaggcatctacaggtttgtgactccgggagaacggccctcgggcatgttcgattcctcggtcctgtgtgagtgctatgacgcgggctgtgcttggtacgagctcacccccgccgagacctcggttaggttgcgggcctacctgaacacaccagggttgcccgtttgccaggaccacctggagttctgggagagtgtcttcacaggcctcacccacatagatgcacacttcttgtcccagaccaagcaggcaggagacaacttcccctacctggtagcataccaagccacggtgtgcgccagggctcaggccccacctccatcatgggatcaaatgtggaagtgtctcatacggctgaaacctacgctgcacgggccaacacccttgctgtacaggctgggagccgtccaaaatgaggtcaccctcacccaccccataaccaaatacatcatggcatgcatgtcggctgacctggaggtcgtcactagcacctgggtgctggtgggcggagtccttgcagctctggccgcgtattgcctgacaacaggcagtgtggtcattgtgggtaggattatcttgtccgggaggccggctattgttcccgacagggagtttctctaccaggagttcgatgaaatggaagagtgcgcctcgcacctcccttacatcgagcagggaatgcagctcgccgagcaattcaagcagaaagcgctcgggttactgcaaacagccaccaaacaagcggaggctgctgctcccgtggtggagtccaagtggcgagcccttgagacattctgggcgaagcacatgtggaatttcatcagcgggatacagtacttagcaggcttatccactctgcctgggaaccccgcaatagcatcattgatggcattcacagcctctatcaccagcccgctcaccacccaaagtaccctcctgtttaacatcttgggggggtgggtggctgcccaactcgccccccccagcgccgcttcggctttcgtgggcgccggcatcgccggtgcggctgttggcagcataggccttgggaaggtgcttgtggacattctggcgggttatggagcaggagtggccggcgcgctcgtggccttcaaggtcatgagcggcgagatgccctccaccgaggacctggtcaatctacttcctgccatcctctctcctggcgccctggtcgtcggggtcgtgtgtgcagcaatactgcgtcgacacgtgggtccgggagagggggctgtgcagtggatgaaccggctgatagcgttcgcctcgcggggtaatcatgtttcccccacgcactatgtgcctgagagcgacgccgcagcgcgtgttactcagatcctctccagccttaccatcactcagctgctgaaaaggctccaccagtggattaatgaagactgctccacaccgtgttccggctcgtggctaagggatgtttgggactggatatgcacggtgttgactgacttcaagacctggctccagtccaagctcctgccgcagctaccgggagtcccttttttctcgtgccaacgcgggtacaagggagtctggcggggagacggcatcatgcaaaccacctgcccatgtggagcacagatcaccggacatgtcaaaaacggttccatgaggatcgtcgggcctaagacctgcagcaacacgtggcatggaacattccccatcaacgcatacaccacgggcccctgcacaccctctccagcgccaaactattctagggcgctgtggcgggtggccgctgaggagtacgtggaggtcacgcgggtgggggatttccactacgtgacgggcatgaccactgacaacgtaaagtgcccatgccaggttccggctcctgaattcttcacggaggtggacggagtgcggttgcacaggtacgctccggcgtgcaggcctctcctacgggaggaggttacattccaggtcgggctcaaccaatacctggttgggtcacagctaccatgcgagcccgaaccggatgtagcagtgctcacttccatgctcaccgacccctcccacatcacagcagaaacggctaagcgtaggttggccagggggtctcccccctccttggccagctcttcagctagccagttgtctgcgccttccttgaaggcgacatgcactacccaccatgtctctccggacgctgacctcatcgaggccaacctcctgtggcggcaggagatgggcgggaacatcacccgcgtggagtcggagaacaaggtggtagtcctggactctttcgacccgcttcgagcggaggaggatgagagggaagtatccgttccggcggagatcctgcggaaatccaagaagttccccgcagcgatgcccatctgggcgcgcccggattacaaccctccactgttagagtcctggaaggacccggactacgtccctccggtggtgcacgggtgcccgttgccacctatcaaggcccctccaataccacctccacggagaaagaggacggttgtcctaacagagtcctccgtgtcttctgccttagcggagctcgctactaagaccttcggcagctccgaatcatcggccgtcgacagcggcacggcgaccgcccttcctgaccaggcctccgacgacggtgacaaaggatccgacgttgagtcgtactcctccatgcccccccttgagggggaaccgggggaccccgatctcagtgacgggtcttggtctaccgtgagcgaggaagctagtgaggatgtcgtctgctgctcaatgtcctacacatggacaggcgccttgatcacgccatgcgctgcggaggaaagcaagctgcccatcaacgcgttgagcaactctttgctgcgccaccataacatggtttatgccacaacatctcgcagcgcaggcctgcggcagaagaaggtcacctttgacagactgcaagtcctggacgaccactaccgggacgtgctcaaggagatgaaggcgaaggcgtccacagttaaggctaaactcctatccgtagaggaagcctgcaagctgacgcccccacattcggccaaatccaagtttggctatggggcaaaggacgtccggaacctatccagcaaggccgttaaccacatccactccgtgtggaaggacttgctggaagacactgtgacaccaattgacaccaccatcatggcaaaaaatgaggttttctgtgtccaaccagagaaaggaggccgtaagccagcccgccttatcgtattcccagatctgggagtccgtgtatgcgagaagatggccctctatgatgtggtctccacccttcctcaggtcgtgatgggctcctcatacggattccagtactctcctgggcagcgagtcgagttcctggtgaatacctggaaatcaaagaaaaaccccatgggcttttcatatgacactcgctgtttcgactcaacggtcaccgagaacgacatccgtgttgaggagtcaatttaccaatgttgtgacttggcccccgaagccagacaggccataaaatcgctcacagagcggctttatatcgggggtcctctgactaattcaaaagggcagaactgcggttatcgccggtgccgcgcgagcggcgtgctgacgactagctgcggtaacaccctcacatgttacttgaaggcctctgcagcctgtcgagctgcgaagctccaggactgcacgatgctcgtgaacgccgccggccttgtcgttatctgtgaaagcgcgggaacccaagaggacgcggcgagcctacgagtcttcacggaggctatgactaggtactctgccccccccggggacccgccccaaccagaatacgacttggagctgataacatcatgttcctccaatgtgtcggtcgcccacgatgcatcaggcaaaagggtgtactacctcacccgtgatcccaccacccccctcgcacgggctgcgtgggaaacagctagacacactccagttaactcctggctaggcaacattatcatgtatgcgcccactttgtgggcaaggatgattctgatgactcacttcttctccatccttctagcacaggagcaacttgaaaaagccctggactgccagatctacggggcctgttactccattgagccacttgacctacctcagatcattgaacgactccatggccttagcgcattttcactccatagttactctccaggtgagatcaatagggtggcttcatgcctcaggaaacttggggtaccacccttgcgagtctggagacatcgggccaggagcgtccgcgctaggctactgtcccagggggggagggccgccacttgtggcaagtacctcttcaactgggcagtgaagaccaaactcaaactcactccaatcccggctgcgtcccagctggacttgtccggctggttcgttgctggttacagcgggggagacatatatcacagcctgtctcgtgcccgaccccgctggttcatgctgtgcctactcctactttctgtaggggtaggcatctacctgctccccaaccgataaatctagagctgtgccttctagttgccagccatctgttgtttgcccctcccccgtgccttccttgaccctggaaggtgccactcccactgtcctttcctaataaaatgaggaaattgcatcgcattgtctgagtaggtgtcattctattctggggggtggggtggggcagcacagcaagggggaggattgggaagacaatagcaggcatgctggggatgcggtgggcgatatcagcgatcgctgaggtgggtgagtgggcgtggcctggggtggtcatgaaaatatataagttgggggtcttagggtctctttatttgtgttgcagagaccgccggagccatgagcgggagcagcagcagcagcagtagcagcagcgccttggatggcagcatcgtgagcccttatttgacgacgcggatgccccactgggccggggtgcgtcagaatgtgatgggctccagcatcgacggccgacccgtcctgcccgcaaattccgccacgctgacctatgcgaccgtcgcggggacgccgttggacgccaccgccgccgccgccgccaccgcagccgcctcggccgtgcgcagcctggccacggactttgcattcctgggaccactggcgacaggggctacttctcgggccgctgctgccgccgttcgcgatgacaagctgaccgccctgctggcgcagttggatgcgcttactcgggaactgggtgacctttctcagcaggtcatggccctgcgccagcaggtctcctccctgcaagctggcgggaatgcttctcccacaaatgccgtttaagataaataaaaccagactctgtttggattaaagaaaagtagcaagtgcattgctctctttatttcataattttccgcgcgcgataggccctagaccagcgttctcggtcgttgagggtgcggtgtatcttctccaggacgtggtagaggtggctctggacgttgagatacatgggcatgagcccgtcccgggggtggaggtagcaccactgcagagcttcatgctccggggtggtgttgtagatgatccagtcgtagcaggagcgctgggcatggtgcctaaaaatgtccttcagcagcaggccgatggccagggggaggcccttggtgtaagtgtttacaaaacggttaagttgggaagggtgcattcggggagagatgatgtgcatcttggactgtatttttagattggcgatgtttccgcccagatcccttctgggattcatgttgtgcaggaccaccagtacagtgtatccggtgcacttggggaatttgtcatgcagcttagagggaaaagcgtggaagaacttggagacgcccttgtggcctcccagattttccatgcattcgtccatgatgatggcaatgggcccgcgggaggcagcttgggcaaagatatttctggggtcgctgacgtcgtagttgtgttccagggtgaggtcgtcataggccatttttacaaagcgcgggcggagggtgcccgactgggggatgatggtcccctctggccctggggcgtagttgccctcgcagatctgcatttcccaggccttaatctcggaggggggaatcatatccacctgcggggcgatgaagaaaacggtttccggagccggggagattaactgggatgagagcaggtttctaagcagctgtgattttccacaaccggtgggcccataaataacacctataaccggttgcagctggtagtttagagagctgcagctgccgtcgtcccggaggaggggggccacctcgttgagcatgtccctgacgcgcatgttctccccgaccagatccgccagaaggcgctcgccgcccagggacagcagctcttgcaaggaagcaaagtttttcagcggcttgaggccgtccgccgtgggcatgtttttcagggtctggctcagcagctccaggcggtcccagagctcggtgacgtgctctacggcatctctatccagcatatctcctcgtttcgcgggttggggcgactttcgctgtagggcaccaagcggtggtcgtccagcggggccaaagtcatgtccttccatgggcgcagggtcctcgtcagggtggtctgggtcacggtgaaggggtgcgctccgggctgagcgcttgccaaggtgcgcttgaggctggttctgctggtgctgaagcgctgccggtcttcgccctgcgcgtcggccaggtagcatttgaccatggtgtcatagtccagcccctccgcggcgtgtcccttggcgcgcagcttgcccttggaggtggcgccgcacgaggggcagagcaggctcttgagcgcgtagagcttgggggcgaggaagaccgattcgggggagtaggcgtccgcgccgcagaccccgcacacggtctcgcactccaccagccaggtgagctcggggcgcgccgggtcaaaaaccaggtttcccccatgctttttgatgcgtttcttacctcgggtctccatgaggtggtgtccccgctcggtgacgaagaggctgtccgtgtctccgtagaccgacttgaggggtcttttctccaggggggtccctcggtcttcctcgtagaggaactcggaccactctgagacgaaggcccgcgtccaggccaggacgaaggaggctatgtgggaggggtagcggtcgttgtccactagggggtccaccttctccaaggtgtgaagacacatgtcgccttcctcggcgtccaggaaggtgattggcttgtaggtgtaggccacgtgaccgggggttcctgacgggggggtataaaagggggtgggggcgcgctcgtcgtcactctcttccgcatcgctgtctgcgagggccagctgctggggtgagtattccctctcgaaggcgggcatgacctccgcgctgaggttgtcagtttccaaaaacgaggaggatttgatgttcacctgtcccgaggtgatacctttgagggtacccgcgtccatctggtcagaaaacacgatctttttattgtccagcttggtggcgaacgacccgtagagggcgttggagagcagcttggcgatggagcgcagggtctggttcttgtccctgtcggcgcgctccttggccgcgatgttgagctgcacgtactcgcgcgcgacgcagcgccactcggggaagacggtggtgcgctcgtcgggcaccaggcgcacgcgccagccgcggttgtgcagggtgaccaggtccacgctggtggcgacctcgccgcgcaggcgctcgttggtccagcagagacggccgcccttgcgcgagcagaaggggggcagggggtcgagctgggtctcgtccggggggtccgcgtccacggtgaaaaccccggggcgcaggcgcgcgtcgaagtagtctatcttgcaaccttgcatgtccagcgcctgctgccagtcgcgggcggcgagcgcgcgctcgtaggggttgagcggcgggccccagggcatggggtgggtgagtgcggaggcgtacatgccgcagatgtcatagacgtagaggggctcccgcaggaccccgatgtaggtggggtagcagcggccgccgcggatgctggcgcgcacgtagtcatacagctcgtgcgagggggcgaggaggtcggggcccaggttggtgcgggcggggcgctccgcgcggaagacgatctgcctgaagatggcatgcgagttggaagagatggtggggcgctggaagacgttgaagctggcgtcctgcaggccgacggcgtcgcgcacgaaggaggcgtaggagtcgcgcagcttgtgtaccagctcggcggtgacctgcacgtcgagcgcgcagtagtcgagggtctcgcggatgatgtcatatttagcctgccccttctttttccacagctcgcggttgaggacaaactcttcgcggtctttccagtactcttggatcgggaaaccgtccggttccgaacggtaagagcctagcatgtagaactggttgacggcctggtaggcgcagcagcccttctccacggggagggcgtaggcctgcgcggccttgcggagcgaggtgtgggtcagggcgaaggtgtccctgaccatgactttgaggtactggtgcttgaagtcggagtcgtcgcagccgccccgctcccagagcgagaagtcggtgcgcttcttggagcgggggttgggcagagcgaaggtgacatcgttgaagaggattttgcccgcgcggggcatgaagttgcgggtgatgcggaagggccccggcacttcagagcggttgttgatgacctgggcggcgagcacgatctcgtcgaagccgttgatgttgtggcccacgatgtagagttccaggaagcggggccggccctttacggtgggcagcttctttagctcttcgtaggtgagctcctcgggcgaggcgaggccgtgctcggccagggcccagtccgcgaggtgcgggttgtctctgaggaaggactcccagaggtcgcgggccaggagggtctgcaggcggtccctgaaggtcctgaactggcggcccacggccattttttcgggggtgatgcagtagaaggtgagggggtcttgctgccagcggtcccagtcgagctgcagggcgaggtcgcgcgcggcggtgaccaggcgctcgtcgcccccgaatttcatgaccagcatgaagggcacgagctgctttccgaaggcccccatccaagtgtaggtctctacatcgtaggtgacaaagaggcgctccgtgcgaggatgcgagccgatcgggaagaactggatctcccgccaccagttggaggagtggctgttgatgtggtggaagtagaagtcccgtcgccgggccgaacactcgtgctggcttttgtaaaagcgagcgcagtactggcagcgctgcacgggctgtacctcctgcacgagatgcacctttcgcccgcgcacgaggaagccgaggggaaatctgagccccccgcctggctcgcggcatggctggtgctcttctactttggatgcgtgtccgtctccgtctggctcctcgaggggtgttacggtggagcggaccaccacgccgcgcgagccgcaggtccagatatcggcgcgcggcggtcggagtttgatgacgacatcgcgcagctgggagctgtccatggtctggagctcccgcggcggcggcaggtcagccgggagttcttgcaggttcacctcgcagagtcgggccagggcgcggggcaggtctaggtggtacctgatctctaggggcgtgttggtggcggcgtcgatggcttgcaggagcccgcatccccggggggcgacgacggtgccccgcggggtggtggtggtggtggtggtggtggtggtggcggtgcagctcagaagcggtgccgcgggcgggcccccggaggtagggggggctccggtcccgccggcaggggcggcagcggcacgtcggcgtggagcgcgggcaggagttggtgctgtgcccggaggttgctggcgaaggcgacgacgcggcggttgatctcctggatctggcgcctctgcgtgaagacgacgggcccggtgagcttgaacctgaaagagagttcgacagaatcaatctcggtgtcattgaccgcggcctggcgcaggatctcctgcacgtctcccgagttgtcttggtaggcgatctcggccatgaactgctcgatctcttcctcctggaggtctccgcgtccggcgcgttccacggtggccgccaggtcgttggagatgcgccccatgagctgcgagaaggcgttgagtccgccctcgttccagactcggctgtagaccacgcccccctggtcatcgcgggcgcgcatgaccacctgcgcgaggttgagctccacgtgccgcgcgaagacggcgtagttgcgcagacgctggaagaggtagttgagggtggtggcggtgtgctcggccacgaagaagttcatgacccagcggcgcaacgtggattcgttgatgtcccccaaggcctccagccgttccatggcctcgtagaagtccacggcgaagttgaaaaactgggagttgcgcgccgacacggtcaactcctcctccagaagacggatgagctcggcgacggtgtcgcgcacctcgcgctcgaaggctatggggatctcttcctccgctagcatcaccacctcctcctcttcctcctcttctggcacttccatgatggcttcctcctcttcggggggcggcggcggcggcggtgggggagggggcgctctgcgccggcggcggcgcaccgggaggcggtccacgaagcgcgcgatcatctccccgcggcggcggcgcatggtctcggtgacggcgcggccgttctcccgggggcgcagttggaagacgccgccggacatctggtgctggggcgggtggccgtgaggcagcgaaacggcgctgacgatgcatctcaacaattgctgcgtaggtacgccgccgagggacctgagggagtccatatccaccggatccgaaaacctttcgaggaaggcgtctaaccagtcgcagtcgcaaggtaggctgagcaccgtggcgggcggcggggggtggggggagtgtctggcggaggtgctgctgatgatgtaattgaagtaggcggacttgacacggcggatggtcgacaggagcaccatgtccttgggtccggcctgctggatgcggaggcggtcggctatgccccaggcttcgttctggcatcggcgcaggtccttgtagtagtcttgcatgagcctttccaccggcacctcttctccttcctcttctgcttcttccatgtctgcttcggccctggggcggcgccgcgcccccctgccccccatgcgcgtgaccccgaaccccctgagcggttggagcagggccaggtcggcgacgacgcgctcggccaggatggcctgctgcacctgcgtgagggtggtttggaagtcatccaagtccacgaagcggtggtaggcgcccgtgttgatggtgtaggtgcagttggccatgacggaccagttgacggtctggtggcccggttgcgacatctcggtgtacctgagtcgcgagtaggcgcgggagtcgaagacgtagtcgttgcaagtccgcaccaggtactggtagcccaccaggaagtgcggcggcggctggcggtagaggggccagcgcagggtggcgggggctccgggggccaggtcttccagcatgaggcggtggtaggcgtagatgtacctggacatccaggtgatacccgcggcggtggtggaggcgcgcgggaagtcgcgcacccggttccagatgttgcgcaggggcagaaagtgctccatggtaggcgtgctctgtccagtcagacgcgcgcagtcgttgatactctagaccagggaaaacgaaagccggtcagcgggcactcttccgtggtctggtgaatagatcgcaagggtatcatggcggagggcctcggttcgagccccgggtccgggccggacggtccgccatgatccacgcggttaccgcccgcgtgtcgaacccaggtgtgcgacgtcagacaacggtggagtgttccttttggcgtttttctggccgggcgccggcgtcgcgtaagagactaagccgcgaaagcgaaagcagtaagtggctcgctccccgtagccggagggatccttgctaagggttgcgttgcggcgaaccccggttcgaatcccgtactcgggccggccggacccgcggctaaggtgttggattggcctccccctcgtataaagaccccgcttgcggattgactccggacacggggacgagccccttttatttttgctttccccagatgcatccggtgctgcggcagatgcgccccccgccccagcagcagcaacaacaccagcaagagcggcagcaacagcagcgggagtcatgcagggccccctcacccaccctcggcgggccggccacctcggcgtccgcggccgtgtctggcgcctgcggcggcggcggggggccggctgacgaccccgaggagcccccgcggcgcagggccagacactacctggacctggaggagggcgagggcctggcgcggctgggggcgccgtctcccgagcgccacccgcgggtgcagctgaagcgcgactcgcgcgaggcgtacgtgcctcggcagaacctgttcagggaccgcgcgggcgaggagcccgaggagatgcgggacaggaggttcagcgcagggcgggagctgcggcaggggctgaaccgcgagcggctgctgcgcgaggaggactttgagcccgacgcgcggacggggatcagccccgcgcgcgcgcacgtggcggccgccgacctggtgacggcgtacgagcagacggtgaaccaggagatcaacttccaaaagagtttcaacaaccacgtgcgcacgctggtggcgcgcgaggaggtgaccatcgggctgatgcacctgtgggactttgtaagcgcgctggtgcagaaccccaacagcaagcctctgacggcgcagctgttcctgatagtgcagcacagcagggacaacgaggcgtttagggacgcgctgctgaacatcaccgagcccgagggtcggtggctgctggacctgattaacatcctgcagagcatagtggtgcaggagcgcagcctgagcctggccgacaaggtggcggccatcaactactcgatgctgagcctgggcaagttttacgcgcgcaagatctaccagacgccgtacgtgcccatagacaaggaggtgaagatcgacggtttttacatgcgcatggcgctgaaggtgctcaccctgagcgacgacctgggcgtgtaccgcaacgagcgcatccacaaggccgtgagcgtgagccggcggcgcgagctgagcgaccgcgagctgatgcacagcctgcagcgggcgctggcgggcgccggcagcggcgacagggaggcggagtcctacttcgatgcgggggcggacctgcgctgggcgcccagccggcgggccctggaggccgcgggggtccgcgaggactatgacgaggacggcgaggaggatgaggagtacgagctagaggagggcgagtacctggactaaaccgcgggtggtgtttccggtagatgcaagacccgaacgtggtggacccggcgctgcgggcggctctgcagagccagccgtccggccttaactcctcagacgactggcgacaggtcatggaccgcatcatgtcgctgacggcgcgtaacccggacgcgttccggcagcagccgcaggccaacaggctctccgccatcctggaggcggtggtgcctgcgcgctcgaaccccacgcacgagaaggtgctggccatagtgaacgcgctggccgagaacagggccatccgcccggacgaggccgggctggtgtacgacgcgctgctgcagcgcgtggcccgctacaacagcggcaacgtgcagaccaacctggaccggctggtgggggacgtgcgcgaggcggtggcgcagcgcgagcgcgcggatcggcagggcaacctgggctccatggtggcgctgaatgccttcctgagcacgcagccggccaacgtgccgcgggggcaggaagactacaccaactttgtgagcgcgctgcggctgatggtgaccgagaccccccagagcgaggtgtaccagtcgggcccggactacttcttccagaccagcagacagggcctgcagacggtgaacctgagccaggctttcaagaacctgcgggggctgtggggcgtgaaggcgcccaccggcgaccgggcgacggtgtccagcctgctgacgcccaactcgcgcctgctgctgctgctgatcgcgccgttcacggacagcggcagcgtgtcccgggacacctacctggggcacctgctgaccctgtaccgcgaggccatcgggcaggcgcaggtggacgagcacaccttccaggagatcaccagcgtgagccgcgcgctggggcaggaggacacgagcagcctggaggcgactctgaactacctgctgaccaaccggcggcagaagattccctcgctgcacagcctgacctccgaggaggagcgcatcttgcgctacgtgcagcagagcgtgagcctgaacctgatgcgcgacggggtgacgcccagcgtggcgctggacatgaccgcgcgcaacatggaaccgggcatgtacgccgcgcaccggccttacatcaaccgcctgatggactacctgcatcgcgcggcggccgtgaaccccgagtactttaccaacgccatcctgaacccgcactggctcccgccgcccgggttctacagcgggggcttcgaggtcccggaggccaacgatggcttcctgtgggacgacatggacgacagcgtgttctccccgcggccgcaggcgctggcggaagcgtccctgctgcgtcccaagaaggaggaggaggaggcgagtcgccgccgcggcagcagcggcgtggcttctctgtccgagctgggggcggcagccgccgcgcgccccgggtccctgggcggcagcccctttccgagcctggtggggtctctgcacagcgagcgcaccacccgccctcggctgctgggcgaggacgagtacctgaataactccctgctgcagccggtgcgggagaaaaacctgccccccgccttccccaacaacgggatagagagcctggtggacaagatgagcagatggaagacctatgcgcaggagcacagggacgcgcccgcgctccggccgcccacgcggcgccagcgccacgaccggcagcgggggctggtgtgggatgacgaggactccgcggacgatagcagcgtgctggacctgggagggagcggcaacccgttcgcgcacctgcgcccccgcctggggaggatgttttaaaaaaaaaaaaagcaagaagcatgatgcaaaattaaataaaactcaccaaggccatggcgaccgagcgttggtttcttgtgttcccttcagtatgcggcgcgcggcgatgtaccaggagggacctcctccctcttacgagagcgtggtgggcgcggcggcggcggcgccctcttctccctttgcgtcgcagctgctggagccgccgtacgtgcctccgcgctacctgcggcctacgggggggagaaacagcatccgttactcggagctggcgcccctgttcgacaccacccgggtgtacctggtggacaacaagtcggcggacgtggcctccctgaactaccagaacgaccacagcaattttttgaccacggtcatccagaacaatgactacagcccgagcgaggccagcacccagaccatcaatctggatgaccggtcgcactggggcggcgacctgaaaaccatcctgcacaccaacatgcccaacgtgaacgagttcatgttcaccaataagttcaaggcgcgggtgatggtgtcgcgctcgcacaccaaggaagaccgggtggagctgaagtacgagtgggtggagttcgagctgccagagggcaactactccgagaccatgaccattgacctgatgaacaacgcgatcgtggagcactatctgaaagtgggcaggcaaaacggggtcctggagagcgacatcggggtcaagttcgacaccaggaacttccgcctggggctggaccccgtgaccgggctggttatgcccggggtgtacaccaacgaggccttccatcccgacatcatcctgctgcccggctgcggggtggacttcacttacagccgcctgagcaacctcctgggcatccgcaagcggcagcccttccaggagggcttcaggatcacctacgaggacctggaggggggcaacatccccgcgctcctcgatgtggaggcctaccaggatagcttgaaggaaaatgaggcgggacaggaggataccacccccgccgcctccgccgccgccgagcagggcgaggatgctgctgacaccgcggccgcggacggggcagaggccgaccccgctatggtggtggaggctcccgagcaggaggaggatatgaatgacagtgcggtgcgcggagacaccttcgtcacccggggggaggaaaagcaagcggaggccgaggccgcggccgaggaaaagcaactggcggcagcagcggcggcggcggcgttggccgcggcggaggctgagtctgaggggaccaagcccgccaaggagcccgtgattaagcccctgaccgaagatagcaagaagcgcagttacaacctgctcaaggacagcaccaacaccgcgtaccgcagctggtacctggcctacaactacggcgacccgtcgacgggggtgcgctcctggaccctgctgtgcacgccggacgtgacctgcggctcggagcaggtgtactggtcgctgcccgacatgatgcaagaccccgtgaccttccgctccacgcggcaggtcagcaacttcccggtggtgggcgccgagctgctgcccgtgcactccaagagcttctacaacgaccaggccgtctactcccagctcatccgccagttcacctctctgacccacgtgttcaatcgctttcctgagaaccagattctggcgcgcccgcccgcccccaccatcaccaccgtcagtgaaaacgttcctgctctcacagatcacgggacgctaccgctgcgcaacagcatcggaggagtccagcgagtgaccgttactgacgccagacgccgcacctgcccctacgtttacaaggccttgggcatagtctcgccgcgcgtcctttccagccgcactttttgagcaacaccaccatcatgtccatcctgatctcacccagcaataactccggctggggactgctgcgcgcgcccagcaagatgttcggaggggcgaggaagcgttccgagcagcaccccgtgcgcgtgcgcgggcacttccgcgccccctggggagcgcacaaacgcggccgcgcggggcgcaccaccgtggacgacgccatcgactcggtggtggagcaggcgcgcaactacaggcccgcggtctctaccgtggacgcggccatccagaccgtggtgcggggcgcgcggcggtacgccaagctgaagagccgccggaagcgcgtggcccgccgccaccgccgccgacccggggccgccgccaaacgcgccgccgcggccctgcttcgccgggccaagcgcacgggccgccgcgccgccatgagggccgcgcgccgcttggccgccggcatcaccgccgccaccatggccccccgtacccgaagacgcgcggccgccgccgccgccgccgccatcagtgacatggccagcaggcgccggggcaacgtgtactgggtgcgcgactcggtgaccggcacgcgcgtgcccgtgcgcttccgccccccgcggacttgagatgatgtgaaaaaacaacactgagtctcctgctgttgtgtgtatcccagcggcggcggcgcgcgcagcgtcatgtccaagcgcaaaatcaaagaagagatgctccaggtcgtcgcgccggagatctatgggcccccgaagaaggaagagcaggattcgaagccccgcaagataaagcgggtcaaaaagaaaaagaaagatgatgacgatgccgatggggaggtggagttcctgcgcgccacggcgcccaggcgcccggtgcagtggaagggccggcgcgtaaagcgcgtcctgcgccccggcaccgcggtggtcttcacgcccggcgagcgctccacccggactttcaagcgcgtctatgacgaggtgtacggcgacgaagacctgctggagcaggccaacgagcgcttcggagagtttgcttacgggaagcgtcagcgggcgctggggaaggaggacctgctggcgctgccgctggaccagggcaaccccacccccagtctgaagcccgtgaccctgcagcaggtgctgccgagcagcgcaccctccgaggcgaagcggggtctgaagcgcgagggcggcgacctggcgcccaccgtgcagctcatggtgcccaagcggcagaggctggaggatgtgctggagaaaatgaaagtagaccccggtctgcagccggacatcagggtccgtcccatcaagcaggtggcgccgggcctcggcgtgcagaccgtggacgtggtcatccccaccggcaactcccccgccgccaccaccactaccgctgcctccacggacatggagacacagaccgatcccgccgcagccgcagccgccgccgcagccgcgacctcctcggcggaggtgcagacggacccctggctgccgccggcgatgtcagctccccgcgcgcgccgcggacgcagaaagtacggcgccgccaacgcgctcctgcccgagtacgccttgcatccttccatcgcgcccacccccggctaccgaggctatacctaccgcccgcgaagagccaagggttccacccgccgtccccgccgacgcgccgccgccaccacccgccgccgccgccgcagacgccagcccgcactggctccagtctccgtgaggagagtggcgcgcgacggacacaccctggtgctgcccagggcgcgctaccaccccagcatcgtttaaaagcctgttgtggttcttgcagatatggccctcacttgccgcctccgtttcccggtgccgggataccgaggaggaagatcgcgccgcaggaggggtctggccggccgcggcctgagcggaggcagccgccgcgcgcaccggcggcgacgcgccaccagccgacgcatgcgcggcggggtgctgcccctgttaatccccctgatcgccgcggcgatcggcgccgtgcccgggatcgcctccgtggccttgcaagcgtcccagaggcattgacagacttgcaaacttgcaaatatggaaaaaaaaaaaaaaccccaataaaaagtctagactctcacgctcgcttggtcctgtgactattttgtagaatggaagacatcaactttgcgtcgctggccccgcgtcacggctcgcgcccgttcctgggacactggaacgatatcggcaccagcaacatgagcggtggcgccttcagttggggctctctgtggagcggcattaaaagtatcgggtctgccgttaaaaattacggctcccgggcctggaacagcagcacgggccagatgttgagagacaagttgaaagagcagaacttccagcagaaggtggtggagggcctggcctccggcatcaacggggtggtggacctggccaaccaggccgtgcagaataaaatcaacagcagactggacccccggccgccggtggaggaggtgccgccggcgctggagacggtgtcccccgatgggcgtggcgagaagcgcccgcggcccgatagggaagagaccactctggtcacgcagaccgatgagccgcccccgtatgaggaggccctaaagcaaggtctgcccaccacgcggcccatcgcgcccatggccaccggggtggtgggccgccacacccccgccacgctggacttgcctccgcccgccgatgtgccgcagcagcagaaggcggcacagccgggcccgcccgcgaccgcctcccgttcctccgccggtcctctgcgccgcgcggccagcggcccccgcgggggggtcgcgaggcacggcaactggcagagcacgctgaacagcatcgtgggtctgggggtgcggtccgtgaagcgccgccgatgctactgaatagcttagctaacgtgttgtatgtgtgtatgcgccctatgtcgccgccagaggagctgctgagtcgccgccgttcgcgcgcccaccaccaccgccactccgcccctcaagatggcgaccccatcgatgatgccgcagtggtcgtacatgcacatctcgggccaggacgcctcggagtacctgagccccgggctggtgcagttcgcccgcgccaccgagagctacttcagcctgagtaacaagtttaggaaccccacggtggcgcccacgcacgatgtgaccaccgaccggtctcagcgcctgacgctgcggttcattcccgtggaccgcgaggacaccgcgtactcgtacaaggcgcggttcaccctggccgtgggcgacaaccgcgtgctggacatggcctccacctactttgacatccgcggggtgctggaccggggtcccactttcaagccctactctggcaccgcctacaactccctggcccccaagggcgctcccaactcctgcgagtgggagcaagaggaaactcaggcagttgaagaagcagcagaagaggaagaagaagatgctgacggtcaagctgaggaagagcaagcagctaccaaaaagactcatgtatatgctcaggctcccctttctggcgaaaaaattagtaaagatggtctgcaaataggaacggacgctacagctacagaacaaaaacctatttatgcagaccctacattccagcccgaaccccaaatcggggagtcccagtggaatgaggcagatgctacagtcgccggcggtagagtgctaaagaaatctactcccatgaaaccatgctatggttcctatgcaagacccacaaatgctaatggaggtcagggtgtactaacggcaaatgcccagggacagctagaatctcaggttgaaatgcaattcttttcaacttctgaaaacgcccgtaacgaggctaacaacattcagcccaaattggtgctgtatagtgaggatgtgcacatggagaccccggatacgcacctttcttacaagcccgcaaaaagcgatgacaattcaaaaatcatgctgggtcagcagtccatgcccaacagacctaattacatcggcttcagagacaactttatcggcctcatgtattacaatagcactggcaacatgggagtgcttgcaggtcaggcctctcagttgaatgcagtggtggacttgcaagacagaaacacagaactgtcctaccagctcttgcttgattccatgggtgacagaaccagatacttttccatgtggaatcaggcagtggacagttatgacccagatgttagaattattgaaaatcatggaactgaagacgagctccccaactattgtttccctctgggtggcataggggtaactgacacttaccaggctgttaaaaccaacaatggcaataacgggggccaggtgacttggacaaaagatgaaacttttgcagatcgcaatgaaataggggtgggaaacaatttcgctatggagatcaacctcagtgccaacctgtggagaaacttcctgtactccaacgtggcgctgtacctaccagacaagcttaagtacaacccctccaatgtggacatctctgacaaccccaacacctacgattacatgaacaagcgagtggtggccccggggctggtggactgctacatcaacctgggcgcgcgctggtcgctggactacatggacaacgtcaaccccttcaaccaccaccgcaatgcgggcctgcgctaccgctccatgctcctgggcaacgggcgctacgtgcccttccacatccaggtgccccagaagttctttgccatcaagaacctcctcctcctgccgggctcctacacctacgagtggaacttcaggaaggatgtcaacatggtcctccagagctctctgggtaacgatctcagggtggacggggccagcatcaagttcgagagcatctgcctctacgccaccttcttccccatggcccacaacacggcctccacgctcgaggccatgctcaggaacgacaccaacgaccagtccttcaatgactacctttccgccgccaacatgctctaccccatacccgccaacgccaccaacgtccccatctccatcccctcgcgcaactgggcggccttccgcggctgggccttcacccgcctcaagaccaaggagaccccctccctgggctcgggattcgacccctactacacctactcgggctctattccctacctggacggcaccttctacctcaaccacactttcaagaaggtctcggtcaccttcgactcctcggtcagctggccgggcaacgaccgtctgctcacccccaacgagttcgagatcaagcgctcggtcgacggggaaggctacaacgtggcccagtgcaacatgaccaaggactggttcctggtccagatgctggccaactacaacatcggctaccagggcttctacatcccagagagctacaaggacaggatgtactccttcttcaggaacttccagcccatgagccggcaggtggtggaccagaccaagtacaaggactaccaggaggtgggcatcatccaccagcacaacaactcgggcttcgtgggctacctcgcccccaccatgcgcgagggacaggcctaccccgccaacttcccctacccgctcataggcaagaccgcggtcgacagcatcacccagaaaaagttcctctgcgaccgcaccctctggcgcatccccttctccagcaacttcatgtccatgggtgcgctctcggacctgggccagaacttgctctacgccaactccgcccacgccctcgacatgaccttcgaggtcgaccccatggacgagcccacccttctctatgttctgttcgaagtctttgacgtggtccgggtccaccagccgcaccgcggcgtcatcgagaccgtgtacctgcgtacgcccttctcggccggcaacgccaccacctaaagaagcaagccgcagtcatcgccgcctgcatgccgtcgggttccaccgagcaagagctcagggccatcgtcagagacctgggatgcgggccctattttttgggcaccttcgacaagcgcttccctggctttgtctccccacacaagctggcctgcgccatcgtcaacacggccggccgcgagaccgggggcgtgcactggctggcctttgcctggaacccgcgctccaaaacatgcttcctctttgaccccttcggcttttcggaccagcggctcaagcaaatctacgagttcgagtacgagggcttgctgcgtcgcagcgccatcgcctcctcgcccgaccgctgcgtcaccctcgaaaagtccacccagaccgtgcaggggcccgactcggccgcctgcggtctcttctgctgcatgtttctgcacgcctttgtgcactggcctcagagtcccatggaccgcaaccccaccatgaacttgctgacgggggtgcccaactccatgctccaaagcccccaggtcgagcccaccctgcgccgcaaccaggagcagctctacagcttcctggagcgccactcgccctacttccgccgccacagcgcacagatcaggagggccacctccttctgccacttgcaagagatgcaagaagggtaataacgatgtacacacttttttctcaataaatggcattttttttttatttatacaagctctctggggtattcatttcccaccaccaccacccgccgttgtcgccatctggctctatttagaaatcgaaagggttctgccgggagtcgccgtgcgccacgggcagggacacgttgcgatactggtagcgggtgccccacttgaactcgggcaccaccaggcgaggcagctcggggaagttttcgctccacaggctgcgggtcagcaccagcgcgttcatcaggtcgggcgccgagatcttgaagtcgcagttggggccgccgccctgcgcgcgcgagttgcggtacaccgggttgcagcactggaacaccaacagcgccgggtgcttcacgctggccagcacgctgcggtcggagatcagctcggcgtccaggtcctccgcgttgctcagcgcgaacggggtcatcttgggcacttgccgccccaggaagggcgcgtgccccggtttcgagttgcagtcgcagcgcagcgggatcagcaggtgcccgtgcccggactcggcgttggggtacagcgcgcgcatgaaggcctgcatctggcggaaggccatctgggccttggcgccctccgagaagaacatgccgcaggacttgcccgagaactggtttgcggggcagctggcgtcgtgcaggcagcagcgcgcgtcggtgttggcgatctgcaccacgttgcgcccccaccggttcttcacgatcttggccttggacgattgctccttcagcgcgcgctgcccgttctcgctggtcacatccatctcgatcacatgttccttgttcaccatgctgctgccgtgcagacacttcagctcgccctccgtctcggtgcagcggtgctgccacagcgcgcagcccgtgggctcgaaagacttgtaggtcacctccgcgaaggactgcaggtacccctgcaaaaagcggcccatcatggtcacgaaggtcttgttgctgctgaaggtcagctgcagcccgcggtgctcctcgttcagccaggtcttgcacacggccgccagcgcctccacctggtcgggcagcatcttgaagttcaccttcagctcattctccacgtggtacttgtccatcagcgtgcgcgccgcctccatgcccttctcccaggccgacaccagcggcaggctcacggggttcttcaccatcaccgtggccgccgcctccgccgcgctttcgctttccgccccgctgttctcttcctcttcctcctcttcctcgccgccgcccactcgcagcccccgcaccacggggtcgtcttcctgcaggcgctgcaccttgcgcttgccgttgcgcccctgcttgatgcgcacgggcgggttgctgaagcccaccatcaccagcgcggcctcttcttgctcgtcctcgctgtccagaatgacctccggggagggggggttggtcatcctcagtaccgaggcacgcttctttttcttcctgggggcgttcgccagctccgcggctgcggccgctgccgaggtcgaaggccgagggctgggcgtgcgcggcaccagcgcgtcttgcgagccgtcctcgtcctcctcggactcgagacggaggcgggcccgcttcttcgggggcgcgcggggcggcggaggcggcggcggcgacggagacggggacgagacatcgtccagggtgggtggacggcgggccgcgccgcgtccgcgctcgggggtggtttcgcgctggtcctcttcccgactggccatctcccactgctccttctcctataggcagaaagagatcatggagtctctcatgcgagtcgagaaggaggaggacagcctaaccgccccctctgagccctccaccaccgccgccaccaccgccaatgccgccgcggacgacgcgcccaccgagaccaccgccagtaccaccctccccagcgacgcacccccgctcgagaatgaagtgctgatcgagcaggacccgggttttgtgagcggagaggaggatgaggtggatgagaaggagaaggaggaggtcgccgcctcagtgccaaaagaggataaaaagcaagaccaggacgacgcagataaggatgagacagcagtcgggcgggggaacggaagccatgatgctgatgacggctacctagacgtgggagacgacgtgctgcttaagcacctgcaccgccagtgcgtcatcgtctgcgacgcgctgcaggagcgctgcgaagtgcccctggacgtggcggaggtcagccgcgcctacgagcggcacctcttcgcgccgcacgtgccccccaagcgccgggagaacggcacctgcgagcccaacccgcgtctcaacttctacccggtcttcgcggtacccgaggtgctggccacctaccacatcttcttccaaaactgcaagatccccctctcctgccgcgctaaccgcacccgcgccgacaaaaccctgaccctgcggcagggcgcccacatacctgatattgcctctctggaggaagtgcccaagatcttcgagggtctcggtcgcgacgagaaacgggcggcgaacgctctgcacggagacagcgaaaacgagagtcactcgggggtgctggtggagctcgagggcgacaacgcgcgcctggccgtactcaagcgcagcatagaggtcacccactttgcctacccggcgctcaacctgccccccaaggtcatgagtgtggtcatgggcgagctcatcatgcgccgcgctcagcccctggccgcggatgcaaacttgcaagagtcctccgaggaaggcctgcccgcggtcagcgacgagcagctagcgcgctggctggagacccgcgaccccgcgcagctggaggagcggcgcaagctcatgatggccgcggtgctggtcaccgtggagctcgagtgtctgcagcgcttcttcgcggaccccgagatgcagcgcaagctcgaggagaccctgcactacaccttccgccagggctacgtgcgccaggcctgcaagatctccaacgtggagctctgcaacctggtctcctacctgggcatcctgcacgagaaccgcctcgggcagaacgtcctgcactccaccctcaaaggggaggcgcgccgcgactacatccgcgactgcgcctacctcttcctctgctacacctggcagacggccatgggggtctggcagcagtgcctggaggagcgcaacctcaaggagctggaaaagctactcaagcgcaccctcagggacctctggacgggcttcaacgagcgctcggtggccgccgcgctggcggacatcatcttccccgagcgcctgctcaagaccctgcagcagggcctgcccgacttcaccagccagagcatgctgcagaactttaggactttcatcctggagcgctcgggcatcctgcctgccacttgctgcgcgctgcccagcgacttcgtgcccatcaagtacagggagtgcccgccgccgctctggggccactgctacctcttccagctggccaactacctcgcctaccactcggacctcatggaagacgtgagcggcgagggcctgctcgagtgccactgccgctgcaacctctgcacgccccaccgctctctagtctgcaacccgcagctgctcagcgagagtcagattatcggtaccttcgagctgcagggtccctcgcctgacgagaagtccgcggctccggggctgaaactcactccggggctgtggacttccgcctacctacgcaaatttgtacctgaggactaccacgcccacgagatcaggttctacgaagaccaatcccgcccgcccaaggcggagctcaccgcctgcgtcatcacccaggggcacatcctgggccaattgcaagccatcaacaaagcccgccgagagttcttgctgaaaaagggtcggggggtgtacctggacccccagtccggcgaggagctaaacccgctacccccgccgccgccccagcagcgggaccttgcttcccaggatggcacccagaaagaagcagcagccgccgccgccgcagccatacatgcttctggaggaagaggaggaggactgggacagtcaggcagaggaggtttcggacgaggagcaggaggagatgatggaagactgggaggaggacagcagcctagacgaggaagcttcagaggccgaagaggtggcagacgcaacaccatcaccctcggtcgcagccccctcgccggggcccctgaaatcctccgaacccagcaccagcgctataacctccgctcctccggcgccggcgccacccgcccgcagacccaaccgtagatgggacaccacaggaaccggggtcggtaagtccaagtgcccgccgccgccaccgcagcagcagcagcagcgccagggctaccgctcgtggcgcgggcacaagaacgccatagtcgcctgcttgcaagactgcgggggcaacatctctttcgcccggcgcttcctgctattccaccacggggtcgcctttccccgcaatgtcctgcattactaccgtcatctctacagcccctactgcagcggcgacccagaggcggcagcggcagccacagcggcgaccaccacctaggaagatatcctccgcgggcaagacagcggcagcagcggccaggagacccgcggcagcagcggcgggagcggtgggcgcactgcgcctctcgcccaacgaacccctctcgacccgggagctcagacacaggatcttccccactttgtatgccatcttccaacagagcagaggccaggagcaggagctgaaaataaaaaacagatctctgcgctccctcacccgcagctgtctgtatcacaaaagcgaagatcagcttcggcgcacgctggaggacgcggaggcactcttcagcaaatactgcgcgctcactcttaaagactagctccgcgcccttctcgaatttaggcgggagaaaactacgtcatcgccggccgccgcccagcccgcccagccgagatgagcaaagagattcccacgccatacatgtggagctaccagccgcagatgggactcgcggcgggagcggcccaggactactccacccgcatgaactacatgagcgcgggaccccacatgatctcacaggtcaacgggatccgcgcccagcgaaaccaaatactgctggaacaggcggccatcaccgccacgccccgccataatctcaacccccgaaattggcccgccgccctcgtgtaccaggaaaccccctccgccaccaccgtactacttccgcgtgacgcccaggccgaagtccagatgactaactcaggggcgcagctcgcgggcggctttcgtcacggggcgcggccgctccgaccaggtataagacacctgatgatcagaggccgaggtatccagctcaacgacgagtcggtgagctcttcgctcggtctccgtccggacggaactttccagctcgccggatccggccgctcttcgttcacgccccgccaggcgtacctgactctgcagacctcgtcctcggagccccgctccggaggcatcggaaccctccagttcgtggaggagttcgtgccctcggtctacttcaaccccttctcgggacctcccggacgctaccccgaccagttcattccgaactttgacgcggtgaaggactcggcggacggctacgactgaatgtcaggtgccgaggcagagcagcttcgcctgagacacctcgagcactgccgccgccacaagtgcttcgcccgcggttccggtgagttctgctactttcagctacccgaggagcataccgaggggccggcgcacggcgtccgcctgaccacccagggcgaggttacctgttccctcatccgggagttcaccctccgtcccctgctagtggagcgggagcggggtccctgtgtcctaactatcgcctgcaactgccctaaccctggattacatcaagatctttgctgtcatctctgtgctgagtttaataaacgctgagatcagaatctactgggaattcgatttagtcccctttaactaatcaaacactggaatcaataaaaagaatcacttacttaaaatcagacagcaggtctctgtccagtttattcagcagcacctccttcccctcctcccaactctggtactccaaacgccttctggcggcaaacttcctccacaccctgaagggaatgtcagattcttgctcctgtccctccgcacccactatcttcatgttgttgcagatgaagcgcaccaaaacgtctgacgagagcttcaaccccgtgtacccctatgacacggaaagcggccctccctccgtccctttcctcacccctcccttcgtgtctcccgatggattccaagaaagcccccccggggtcctgtctctgaacctggccgagcccctggtcacttcccacggcatgctcgccctgaaaatgggaagtggcctctccctggacgacgctggcaacctcacctctcaagatatcaccaccgctagccctcccctcaaaaaaaccaagaccaacctcagcctagaaacctcatcccccctaactgtaagcacctcaggcgccctcaccgtagcagccgccgctcccctggcagtggccggcacctccctcaccatgcaatcagaggcccccctgacagtacaggatgcaaaactcaccctggccaccaaaggccccctgaccgtgtctgaaggcaaactggccttgcaaacatcggccccgctgacggccgctgacagcagcaccctcaccgttagcgccacaccaccaattaatgtaagcagtggaagtttaggcttagacatggaagaccctatgtatactcacgatggaaaactgggaataagaattgggggtccactaagagtagtagacagcttgcacacactcactgtagttaccggaaatggactaactgtagataacaatgccctccaaactagagttacgggcgccctaggttatgacacatcaggaaatctacaattgagagctgcaggaggtatgcgaattgatgcaaatggccaacttatccttaatgtggcatacccatttgatgctcagaacaatctcagccttagacttggtcagggacccctgtatataaacacagaccacaacctggatttgaattgcaacagaggtctaaccacaactaccaccaacaacacaaaaaaacttgagactaaaattagctcaggcttagactatgacaccaatggtgctgtcattattaaacttggcactggtctaagcttcgacaacacaggcgccctaactgtgggaaacactggtgatgataaactgactctgtggacgaccccagacccatctccaaattgcagaattcactcagacaaagactgcaagtttactctagtcctaactaagtgtggaagccaaatcctggcctctgtcgccgccctagcggtatcaggaaatctggcttcgataacaggcaccgttgccagcgttaccatctttctcagatttgatcagaatggagtgcttatggaaaactcctcgctagacaggcagtactggaacttcagaaatggcaactcaactaacgctgccccctacaccaatgcagttgggttcatgccaaacctcgcagcataccccaaaacgcaaagccagactgctaaaaacaacattgtaagtcaggtttacttgaatggagacaaatccaaacccatgacccttaccatcaccctcaatggaactaatgaatccagtgaaactagccaggtgagtcactactccatgtcatttacatgggcttgggaaagtgggcaatatgccactgaaacctttgccaccaactccttcaccttttcttacattgctgaacaataaaaagcatgacactgatgttcatttctgattcttattttattattttcaaacacaacaaaatcattcaagtcattcttccatcttagcttaatagacacagtagcttaatagacccagtagtgcaaagccccattctagcttataactagtggagaagtactcgcctacatgggggtagagtcataatcgtgcatcaggatagggcggtggtgctgcagcagcgcgcgaataaactgctgccgccgccgctccgtcctgcaggaatacaacatggcagtggtctcctcagcgatgattcgcaccgcccgcagcataaggcgccttgtcctccgggcacagcagcgcaccctgatctcacttaaatcagcacagtaactgcagcacagcaccacaatattgttcaaaatcccacagtgcaaggcgctgtatccaaagctcatggcggggaccacagaacccacgtggccatcataccacaagcgcaggtagattaagtggcgacccctcataaacacgctggacataaacattacctcttttggcatgttgtaattcaccacctcccggtaccatataaacctctgattaaacatggcgccatccaccaccatcctaaaccagctggccaaaacctgcccgccggctatacactgcagggaaccgggactggaacaatgacagtggagagcccaggactcgtaaccatggatcatcatgctcgtcatgatatcaatgttggcacaacacaggcacacgtgcatacacttcctcaggattacaagctcctcccgcgttagaaccatatcccagggaacaacccattcctgaatcagcgtaaatcccacactgcagggaagacctcgcacgtaactcacgttgtgcattgtcaaagtgttacattcgggcagcagcggatgatcctccagtatggtagcgcgggtttctgtctcaaaaggaggtagacgatccctactgtacggagtgcgccgagacaaccgagatcgtgttggtcgtagtgtcatgccaaatggaacgccggacgtagtcatatttcctgaagtcttagatctctcaacgcagcaccagcaccaacacttcgcagtgtaaaaggccaagtgccgagagagtatatataggaataaaaagtgacgtaaacgggcaaagtccaaaaaacgcccagaaaaaccgcacgcgaacctacgccccgaaacgaaagccaaaaaacactagacactcccttccggcgtcaacttccgctttcccacgctacgtcacttgccccagtcaaacaaactacatatcccgaacttccaagtcgccacgcccaaaacaccgcctacacctccccgcccgccggcccgcccccaaacccgcctcccgccccgcgccccgccccgcgccgcccatctcattatcatattggcttcaatccaaaataaggtatattattgatgatg

SEQ ID NO: 14 - DNA, 37741 bp, Chimpanzee adenovirus type 3
catcatcaataatataccttattttggattgaagccaatatgataatgagatgggcggcgcgaggcggggcgcggggcgggaggcgggtttgggggcgggccggcgggcggggcggtgtggcggaagtggactttgtaagtgtggcggatgtgacttgctagtgccgggcgcggtaaaagtgacgttttccgtgcgcgacaacgcccccgggaagtgacatttttcccgcggtttttaccggatgttgtagtgaatttgggcgtaaccaagtaagatttggccattttcgcgggaaaactgaaacggggaagtgaaatctgattaattttgcgttagtcataccgcgtaatatttgtctagggccgagggactttggccgattacgtggaggactcgcccaggtgttttttgaggtgaatttccgcgttccgggtcaaagtctccgttttattattatagtcagctgacgcggagtgtatttataccctctgatctcgtcaagaggccactcttgagtgccagcgagtagagttttctcctctgccgctctccgctccgctccgctcggctctgacaccggggaaaaaatgagacatttcacctacgatggcggtgtgctcaccggccagctggctgctgaggtcctggacaccctgatcgaggaggtattggccgataattatcctccctcgactccttttgagccacctacacttcacgaactatacgatctggatgtggtggggcccagcgatccgaacgagcaggcggtttccagtttttttccagagtccatgttgttggccagccaggagggggtcgaacttgagacccctcctccgatcgtggattcccccgatccgccgcagctgactaggcagcccgagcgctgtgcgggacctgagactatgccccagctgctacctgaggtgatcgatctcacctgtaatgagtctggttttccacccagcgaggatgaggacgaagagggtgagcagtttgtgttagattctgtggaacaacccgggcgaggatgcaggtcttgtcaatatcaccggaaaaacacaggagactcccagattatgtgttctctgtgttatatgaagatgacctgtatgtttatttacagtaagtttatcatcggtgggcaggtgggctatagtgtgggtggtggtctttggggggttttttaatatatgtcaggggttatgctgaagacttttttattgtgatttttaaaggtccagtgtctgagcccgagcaagaacctgaaccggagcctgagccttctcgccccaggagaaagcctgtaatcttaactagacccagcgcaccggtagcgagaggcctcagcagcgcggagaccaccgactccggtgcttcctcatcacccccggagattcaccccctggtgcccctatgtcccgttaagcccgttgccgtgagagtcagtgggcggcggtctgctgtggagtgcattgaggacttgctttttgattcacaggaacctttggacttgagcttgaaacgccccaggcattaaacctggtcacctggactgaatgagttgacgcctatgtttgcttttgaatgacttaatgtgtatagataataaagagtgagataatgttttaattgcatggtgtgtttaacttgggcggagtctgctgggtatataagcttccctgggctaaacttggttacacttgacctcatggaggcctgggagtgtttggagaactttgccggagttcgtgccttgctggacgagagctctaacaatacctcttggtggtggaggtatttgtggggctctccccagggcaagttagtttgtagaatcaaggaggattacaagtgggaatttgaagagcttttgaaatcctgtggtgagctattggattctttgaatctaggccaccaggctctcttccaggagaaggtcatcaggactttggatttttccacaccggggcgcattgcagccgcggttgcttttctagcttttttgaaggatagatggagcgaagagacccacttgagttcgggctacgtcctggattttctggccatgcaactgtggagagcatggatcagacacaagaacaggctgcaactgttgtcttccgtccgcccgttgctgattccggcggaggagcaacaggccgggtcagaggaccgggcccgtcgggatccggaggagagggcaccgaggccgggcgagaggagcgcgctgaacctgggaaccgggctgagcggccatccacatcgggagtgaatgtcgggcaggtggtggatctttttccagaactgcggcggattttgactattagggaggatgggcaatttgttaagggtcttaagagggagaggggggcttctgagcataacgaggaggccagtaatttagcttttagcttgatgaccagacaccgtccagagtgcatcacttttcagcagattaaggacaattgtgccaatgagttggatctgttgggtcagaagtatagcatagagcagctgaccacttactggctgcagccgggtgatgatctggaggaagctattagggtgtatgctaaggtggccctgcggcccgattgcaagtacaagctcaaggggctggtgaatatcaggaattgttgctacatttctggcaacggggcggaggtggagatagagaccgaagacagggtggctttcagatgcagcatgatgaatatgtggccgggggtgctgggcatggacggggtggtgattatgaatgtgaggttcacggggcccaactttaacggcacggtgtttttggggaacaccaacctggtcctgcacggggtgagcttctatgggtttaacaacacctgtgtggaggcctggaccgatgtgaaggtccgcggttgcgccttttatggatgttggaaggccatagtgagccgccctaagagcaggagttccattaagaaatgcttgtttgagaggtgcaccttggggatcctggccgagggcaactgcagggtgcgccacaatgtggcctccgagtgcggttgcttcatgctagtcaagagcgtggcggtaatcaagcataatatggtgtgcggcaacagcgaggacaaggcctcacagatgctgacctgcacggatggcaactgccacttgctgaagaccatccatgtaaccagccacagccggaaggcctggcccgtgttcgagcacaacttgctgacccgctgctccttgcatctgggcaacaggcggggggtgttcctgccctatcaatgcaactttagtcacaccaagatcttgctagagcccgagagcatgtccaaggtgaacttgaacggggtgtttgacatgaccatgaagatctggaaggtgctgaggtacgacgagaccaggtcccggtgcagaccctgcgagtgcgggggcaagcatatgaggaaccagcccgtgatgctggatgtgaccgaggagctgaggacagaccacttggttctggcctgcaccagggccgagtttggttctagcgatgaagacacagattgaggtgggtgagtgggcgtggcctggggtggtcatgaaaatatataagttgggggtcttagggtctctttatttgtgttgcagagaccgccggagccatgagcgggagcagcagcagcagcagtagcagcagcgccttggatggcagcatcgtgagcccttatttgacgacgcggatgccccactgggccggggtgcgtcagaatgtgatgggctccagcatcgacggccgacccgtcctgcccgcaaattccgccacgctgacctatgcgaccgtcgcggggacgccgttggacgccaccgccgccgccgccgccaccgcagccgcctcggccgtgcgcagcctggccacggactttgcattcctgggaccactggcgacaggggctacttctcgggccgctgctgccgccgttcgcgatgacaagctgaccgccctgctggcgcagttggatgcgcttactcgggaactgggtgacctttctcagcaggtcatggccctgcgccagcaggtctcctccctgcaagctggcgggaatgcttctcccacaaatgccgtttaagataaataaaaccagactctgtttggattaaagaaaagtagcaagtgcattgctctctttatttcataattttccgcgcgcgataggccctagaccagcgttctcggtcgttgagggtgcggtgtatcttctccaggacgtggtagaggtggctctggacgttgagatacatgggcatgagcccgtcccgggggtggaggtagcaccactgcagagcttcatgctccggggtggtgttgtagatgatccagtcgtagcaggagcgctgggcatggtgcctaaaaatgtccttcagcagcaggccgatggccagggggaggcccttggtgtaagtgtttacaaaacggttaagttgggaagggtgcattcggggagagatgatgtgcatcttggactgtatttttagattggcgatgtttccgcccagatcccttctgggattcatgttgtgcaggaccaccagtacagtgtatccggtgcacttggggaatttgtcatgcagcttagagggaaaagcgtggaagaacttggagacgcccttgtggcctcccagattttccatgcattcgtccatgatgatggcaatgggcccgcgggaggcagcttgggcaaagatatttctggggtcgctgacgtcgtagttgtgttccagggtgaggtcgtcataggccatttttacaaagcgcgggcggagggtgcccgactgggggatgatggtcccctctggccctggggcgtagttgccctcgcagatctgcatttcccaggccttaatctcggaggggggaatcatatccacctgcggggcgatgaagaaaacggtttccggagccggggagattaactgggatgagagcaggtttctaagcagctgtgattttccacaaccggtgggcccataaataacacctataaccggttgcagctggtagtttagagagctgcagctgccgtcgtcccggaggaggggggccacctcgttgagcatgtccctgacgcgcatgttctccccgaccagatccgccagaaggcgctcgccgcccagggacagcagctcttgcaaggaagcaaagtttttcagcggcttgaggccgtccgccgtgggcatgtttttcagggtctggctcagcagctccaggcggtcccagagctcggtgacgtgctctacggcatctctatccagcatatctcctcgtttcgcgggttggggcgactttcgctgtagggcaccaagcggtggtcgtccagcggggccaaagtcatgtccttccatgggcgcagggtcctcgtcagggtggtctgggtcacggtgaaggggtgcgctccgggctgagcgcttgccaaggtgcgcttgaggctggttctgctggtgctgaagcgctgccggtcttcgccctgcgcgtcggccaggtagcatttgaccatggtgtcatagtccagcccctccgcggcgtgtcccttggcgcgcagcttgcccttggaggtggcgccgcacgaggggcagagcaggctcttgagcgcgtagagcttgggggcgaggaagaccgattcgggggagtaggcgtccgcgccgcagaccccgcacacggtctcgcactccaccagccaggtgagctcggggcgcgccgggtcaaaaaccaggtttcccccatgctttttgatgcgtttcttacctcgggtctccatgaggtggtgtccccgctcggtgacgaagaggctgtccgtgtctccgtagaccgacttgaggggtcttttctccaggggggtccctcggtcttcctcgtagaggaactcggaccactctgagacgaaggcccgcgtccaggccaggacgaaggaggctatgtgggaggggtagcggtcgttgtccactagggggtccaccttctccaaggtgtgaagacacatgtcgccttcctcggcgtccaggaaggtgattggcttgtaggtgtaggccacgtgaccgggggttcctgacgggggggtataaaagggggtgggggcgcgctcgtcgtcactctcttccgcatcgctgtctgcgagggccagctgctggggtgagtattccctctcgaaggcgggcatgacctccgcgctgaggttgtcagtttccaaaaacgaggaggatttgatgttcacctgtcccgaggtgatacctttgagggtacccgcgtccatctggtcagaaaacacgatctttttattgtccagcttggtggcgaacgacccgtagagggcgttggagagcagcttggcgatggagcgcagggtctggttcttgtccctgtcggcgcgctccttggccgcgatgttgagctgcacgtactcgcgcgcgacgcagcgccactcggggaagacggtggtgcgctcgtcgggcaccaggcgcacgcgccagccgcggttgtgcagggtgaccaggtccacgctggtggcgacctcgccgcgcaggcgctcgttggtccagcagagacggccgcccttgcgcgagcagaaggggggcagggggtcgagctgggtctcgtccggggggtccgcgtccacggtgaaaaccccggggcgcaggcgcgcgtcgaagtagtctatcttgcaaccttgcatgtccagcgcctgctgccagtcgcgggcggcgagcgcgcgctcgtaggggttgagcggcgggccccagggcatggggtgggtgagtgcggaggcgtacatgccgcagatgtcatagacgtagaggggctcccgcaggaccccgatgtaggtggggtagcagcggccgccgcggatgctggcgcgcacgtagtcatacagctcgtgcgagggggcgaggaggtcggggcccaggttggtgcgggcggggcgctccgcgcggaagacgatctgcctgaagatggcatgcgagttggaagagatggtggggcgctggaagacgttgaagctggcgtcctgcaggccgacggcgtcgcgcacgaaggaggcgtaggagtcgcgcagcttgtgtaccagctcggcggtgacctgcacgtcgagcgcgcagtagtcgagggtctcgcggatgatgtcatatttagcctgccccttctttttccacagctcgcggttgaggacaaactcttcgcggtctttccagtactcttggatcgggaaaccgtccggttccgaacggtaagagcctagcatgtagaactggttgacggcctggtaggcgcagcagcccttctccacggggagggcgtaggcctgcgcggccttgcggagcgaggtgtgggtcagggcgaaggtgtccctgaccatgactttgaggtactggtgcttgaagtcggagtcgtcgcagccgccccgctcccagagcgagaagtcggtgcgcttcttggagcgggggttgggcagagcgaaggtgacatcgttgaagaggattttgcccgcgcggggcatgaagttgcgggtgatgcggaagggccccggcacttcagagcggttgttgatgacctgggcggcgagcacgatctcgtcgaagccgttgatgttgtggcccacgatgtagagttccaggaagcggggccggccctttacggtgggcagcttctttagctcttcgtaggtgagctcctcgggcgaggcgaggccgtgctcggccagggcccagtccgcgaggtgcgggttgtctctgaggaaggactcccagaggtcgcgggccaggagggtctgcaggcggtccctgaaggtcctgaactggcggcccacggccattttttcgggggtgatgcagtagaaggtgagggggtcttgctgccagcggtcccagtcgagctgcagggcgaggtcgcgcgcggcggtgaccaggcgctcgtcgcccccgaatttcatgaccagcatgaagggcacgagctgctttccgaaggcccccatccaagtgtaggtctctacatcgtaggtgacaaagaggcgctccgtgcgaggatgcgagccgatcgggaagaactggatctcccgccaccagttggaggagtggctgttgatgtggtggaagtagaagtcccgtcgccgggccgaacactcgtgctggcttttgtaaaagcgagcgcagtactggcagcgctgcacgggctgtacctcctgcacgagatgcacctttcgcccgcgcacgaggaagccgaggggaaatctgagccccccgcctggctcgcggcatggctggtgctcttctactttggatgcgtgtccgtctccgtctggctcctcgaggggtgttacggtggagcggaccaccacgccgcgcgagccgcaggtccagatatcggcgcgcggcggtcggagtttgatgacgacatcgcgcagctgggagctgtccatggtctggagctcccgcggcggcggcaggtcagccgggagttcttgcaggttcacctcgcagagtcgggccagggcgcggggcaggtctaggtggtacctgatctctaggggcgtgttggtggcggcgtcgatggcttgcaggagcccgcatccccggggggcgacgacggtgccccgcggggtggtggtggtggtggtggtggtggtggtggcggtgcagctcagaagcggtgccgcgggcgggcccccggaggtagggggggctccggtcccgccggcaggggcggcagcggcacgtcggcgtggagcgcgggcaggagttggtgctgtgcccggaggttgctggcgaaggcgacgacgcggcggttgatctcctggatctggcgcctctgcgtgaagacgacgggcccggtgagcttgaacctgaaagagagttcgacagaatcaatctcggtgtcattgaccgcggcctggcgcaggatctcctgcacgtctcccgagttgtcttggtaggcgatctcggccatgaactgctcgatctcttcctcctggaggtctccgcgtccggcgcgttccacggtggccgccaggtcgttggagatgcgccccatgagctgcgagaaggcgttgagtccgccctcgttccagactcggctgtagaccacgcccccctggtcatcgcgggcgcgcatgaccacctgcgcgaggttgagctccacgtgccgcgcgaagacggcgtagttgcgcagacgctggaagaggtagttgagggtggtggcggtgtgctcggccacgaagaagttcatgacccagcggcgcaacgtggattcgttgatgtcccccaaggcctccagccgttccatggcctcgtagaagtccacggcgaagttgaaaaactgggagttgcgcgccgacacggtcaactcctcctccagaagacggatgagctcggcgacggtgtcgcgcacctcgcgctcgaaggctatggggatctcttcctccgctagcatcaccacctcctcctcttcctcctcttctggcacttccatgatggcttcctcctcttcggggggcggcggcggcggcggtgggggagggggcgctctgcgccggcggcggcgcaccgggaggcggtccacgaagcgcgcgatcatctccccgcggcggcggcgcatggtctcggtgacggcgcggccgttctcccgggggcgcagttggaagacgccgccggacatctggtgctggggcgggtggccgtgaggcagcgaaacggcgctgacgatgcatctcaacaattgctgcgtaggtacgccgccgagggacctgagggagtccatatccaccggatccgaaaacctttcgaggaaggcgtctaaccagtcgcagtcgcaaggtaggctgagcaccgtggcgggcggcggggggtggggggagtgtctggcggaggtgctgctgatgatgtaattgaagtaggcggacttgacacggcggatggtcgacaggagcaccatgtccttgggtccggcctgctggatgcggaggcggtcggctatgccccaggcttcgttctggcatcggcgcaggtccttgtagtagtcttgcatgagcctttccaccggcacctcttctccttcctcttctgcttcttccatgtctgcttcggccctggggcggcgccgcgcccccctgccccccatgcgcgtgaccccgaaccccctgagcggttggagcagggccaggtcggcgacgacgcgctcggccaggatggcctgctgcacctgcgtgagggtggtttggaagtcatccaagtccacgaagcggtggtaggcgcccgtgttgatggtgtaggtgcagttggccatgacggaccagttgacggtctggtggcccggttgcgacatctcggtgtacctgagtcgcgagtaggcgcgggagtcgaagacgtagtcgttgcaagtccgcaccaggtactggtagcccaccaggaagtgcggcggcggctggcggtagaggggccagcgcagggtggcgggggctccgggggccaggtcttccagcatgaggcggtggtaggcgtagatgtacctggacatccaggtgatacccgcggcggtggtggaggcgcgcgggaagtcgcgcacccggttccagatgttgcgcaggggcagaaagtgctccatggtaggcgtgctctgtccagtcagacgcgcgcagtcgttgatactctagaccagggaaaacgaaagccggtcagcgggcactcttccgtggtctggtgaatagatcgcaagggtatcatggcggagggcctcggttcgagccccgggtccgggccggacggtccgccatgatccacgcggttaccgcccgcgtgtcgaacccaggtgtgcgacgtcagacaacggtggagtgttccttttggcgtttttctggccgggcgccggcgtcgcgtaagagactaagccgcgaaagcgaaagcagtaagtggctcgctccccgtagccggagggatccttgctaagggttgcgttgcggcgaaccccggttcgaatcccgtactcgggccggccggacccgcggctaaggtgttggattggcctccccctcgtataaagaccccgcttgcggattgactccggacacggggacgagccccttttatttttgctttccccagatgcatccggtgctgcggcagatgcgccccccgccccagcagcagcaacaacaccagcaagagcggcagcaacagcagcgggagtcatgcagggccccctcacccaccctcggcgggccggccacctcggcgtccgcggccgtgtctggcgcctgcggcggcggcggggggccggctgacgaccccgaggagcccccgcggcgcagggccagacactacctggacctggaggagggcgagggcctggcgcggctgggggcgccgtctcccgagcgccacccgcgggtgcagctgaagcgcgactcgcgcgaggcgtacgtgcctcggcagaacctgttcagggaccgcgcgggcgaggagcccgaggagatgcgggacaggaggttcagcgcagggcgggagctgcggcaggggctgaaccgcgagcggctgctgcgcgaggaggactttgagcccgacgcgcggacggggatcagccccgcgcgcgcgcacgtggcggccgccgacctggtgacggcgtacgagcagacggtgaaccaggagatcaacttccaaaagagtttcaacaaccacgtgcgcacgctggtggcgcgcgaggaggtgaccatcgggctgatgcacctgtgggactttgtaagcgcgctggtgcagaaccccaacagcaagcctctgacggcgcagctgttcctgatagtgcagcacagcagggacaacgaggcgtttagggacgcgctgctgaacatcaccgagcccgagggtcggtggctgctggacctgattaacatcctgcagagcatagtggtgcaggagcgcagcctgagcctggccgacaaggtggcggccatcaactactcgatgctgagcctgggcaagttttacgcgcgcaagatctaccagacgccgtacgtgcccatagacaaggaggtgaagatcgacggtttttacatgcgcatggcgctgaaggtgctcaccctgagcgacgacctgggcgtgtaccgcaacgagcgcatccacaaggccgtgagcgtgagccggcggcgcgagctgagcgaccgcgagctgatgcacagcctgcagcgggcgctggcgggcgccggcagcggcgacagggaggcggagtcctacttcgatgcgggggcggacctgcgctgggcgcccagccggcgggccctggaggccgcgggggtccgcgaggactatgacgaggacggcgaggaggatgaggagtacgagctagaggagggcgagtacctggactaaaccgcgggtggtgtttccggtagatgcaagacccgaacgtggtggacccggcgctgcgggcggctctgcagagccagccgtccggccttaactcctcagacgactggcgacaggtcatggaccgcatcatgtcgctgacggcgcgtaacccggacgcgttccggcagcagccgcaggccaacaggctctccgccatcctggaggcggtggtgcctgcgcgctcgaaccccacgcacgagaaggtgctggccatagtgaacgcgctggccgagaacagggccatccgcccggacgaggccgggctggtgtacgacgcgctgctgcagcgcgtggcccgctacaacagcggcaacgtgcagaccaacctggaccggctggtgggggacgtgcgcgaggcggtggcgcagcgcgagcgcgcggatcggcagggcaacctgggctccatggtggcgctgaatgccttcctgagcacgcagccggccaacgtgccgcgggggcaggaagactacaccaactttgtgagcgcgctgcggctgatggtgaccgagaccccccagagcgaggtgtaccagtcgggcccggactacttcttccagaccagcagacagggcctgcagacggtgaacctgagccaggctttcaagaacctgcgggggctgtggggcgtgaaggcgcccaccggcgaccgggcgacggtgtccagcctgctgacgcccaactcgcgcctgctgctgctgctgatcgcgccgttcacggacagcggcagcgtgtcccgggacacctacctggggcacctgctgaccctgtaccgcgaggccatcgggcaggcgcaggtggacgagcacaccttccaggagatcaccagcgtgagccgcgcgctggggcaggaggacacgagcagcctggaggcgactctgaactacctgctgaccaaccggcggcagaagattccctcgctgcacagcctgacctccgaggaggagcgcatcttgcgctacgtgcagcagagcgtgagcctgaacctgatgcgcgacggggtgacgcccagcgtggcgctggacatgaccgcgcgcaacatggaaccgggcatgtacgccgcgcaccggccttacatcaaccgcctgatggactacctgcatcgcgcggcggccgtgaaccccgagtactttaccaacgccatcctgaacccgcactggctcccgccgcccgggttctacagcgggggcttcgaggtcccggaggccaacgatggcttcctgtgggacgacatggacgacagcgtgttctccccgcggccgcaggcgctggcggaagcgtccctgctgcgtcccaagaaggaggaggaggaggcgagtcgccgccgcggcagcagcggcgtggcttctctgtccgagctgggggcggcagccgccgcgcgccccgggtccctgggcggcagcccctttccgagcctggtggggtctctgcacagcgagcgcaccacccgccctcggctgctgggcgaggacgagtacctgaataactccctgctgcagccggtgcgggagaaaaacctgccccccgccttccccaacaacgggatagagagcctggtggacaagatgagcagatggaagacctatgcgcaggagcacagggacgcgcccgcgctccggccgcccacgcggcgccagcgccacgaccggcagcgggggctggtgtgggatgacgaggactccgcggacgatagcagcgtgctggacctgggagggagcggcaacccgttcgcgcacctgcgcccccgcctggggaggatgttttaaaaaaaaaaaaagcaagaagcatgatgcaaaattaaataaaactcaccaaggccatggcgaccgagcgttggtttcttgtgttcccttcagtatgcggcgcgcggcgatgtaccaggagggacctcctccctcttacgagagcgtggtgggcgcggcggcggcggcgccctcttctccctttgcgtcgcagctgctggagccgccgtacgtgcctccgcgctacctgcggcctacgggggggagaaacagcatccgttactcggagctggcgcccctgttcgacaccacccgggtgtacctggtggacaacaagtcggcggacgtggcctccctgaactaccagaacgaccacagcaattttttgaccacggtcatccagaacaatgactacagcccgagcgaggccagcacccagaccatcaatctggatgaccggtcgcactggggcggcgacctgaaaaccatcctgcacaccaacatgcccaacgtgaacgagttcatgttcaccaataagttcaaggcgcgggtgatggtgtcgcgctcgcacaccaaggaagaccgggtggagctgaagtacgagtgggtggagttcgagctgccagagggcaactactccgagaccatgaccattgacctgatgaacaacgcgatcgtggagcactatctgaaagtgggcaggcaaaacggggtcctggagagcgacatcggggtcaagttcgacaccaggaacttccgcctggggctggaccccgtgaccgggctggttatgcccggggtgtacaccaacgaggccttccatcccgacatcatcctgctgcccggctgcggggtggacttcacttacagccgcctgagcaacctcctgggcatccgcaagcggcagcccttccaggagggcttcaggatcacctacgaggacctggaggggggcaacatccccgcgctcctcgatgtggaggcctaccaggatagcttgaaggaaaatgaggcgggacaggaggataccacccccgccgcctccgccgccgccgagcagggcgaggatgctgctgacaccgcggccgcggacggggcagaggccgaccccgctatggtggtggaggctcccgagcaggaggaggatatgaatgacagtgcggtgcgcggagacaccttcgtcacccggggggaggaaaagcaagcggaggccgaggccgcggccgaggaaaagcaactggcggcagcagcggcggcggcggcgttggccgcggcggaggctgagtctgaggggaccaagcccgccaaggagcccgtgattaagcccctgaccgaagatagcaagaagcgcagttacaacctgctcaaggacagcaccaacaccgcgtaccgcagctggtacctggcctacaactacggcgacccgtcgacgggggtgcgctcctggaccctgctgtgcacgccggacgtgacctgcggctcggagcaggtgtactggtcgctgcccgacatgatgcaagaccccgtgaccttccgctccacgcggcaggtcagcaacttcccggtggtgggcgccgagctgctgcccgtgcactccaagagcttctacaacgaccaggccgtctactcccagctcatccgccagttcacctctctgacccacgtgttcaatcgctttcctgagaaccagattctggcgcgcccgcccgcccccaccatcaccaccgtcagtgaaaacgttcctgctctcacagatcacgggacgctaccgctgcgcaacagcatcggaggagtccagcgagtgaccgttactgacgccagacgccgcacctgcccctacgtttacaaggccttgggcatagtctcgccgcgcgtcctttccagccgcactttttgagcaacaccaccatcatgtccatcctgatctcacccagcaataactccggctggggactgctgcgcgcgcccagcaagatgttcggaggggcgaggaagcgttccgagcagcaccccgtgcgcgtgcgcgggcacttccgcgccccctggggagcgcacaaacgcggccgcgcggggcgcaccaccgtggacgacgccatcgactcggtggtggagcaggcgcgcaactacaggcccgcggtctctaccgtggacgcggccatccagaccgtggtgcggggcgcgcggcggtacgccaagctgaagagccgccggaagcgcgtggcccgccgccaccgccgccgacccggggccgccgccaaacgcgccgccgcggccctgcttcgccgggccaagcgcacgggccgccgcgccgccatgagggccgcgcgccgcttggccgccggcatcaccgccgccaccatggccccccgtacccgaagacgcgcggccgccgccgccgccgccgccatcagtgacatggccagcaggcgccggggcaacgtgtactgggtgcgcgactcggtgaccggcacgcgcgtgcccgtgcgcttccgccccccgcggacttgagatgatgtgaaaaaacaacactgagtctcctgctgttgtgtgtatcccagcggcggcggcgcgcgcagcgtcatgtccaagcgcaaaatcaaagaagagatgctccaggtcgtcgcgccggagatctatgggcccccgaagaaggaagagcaggattcgaagccccgcaagataaagcgggtcaaaaagaaaaagaaagatgatgacgatgccgatggggaggtggagttcctgcgcgccacggcgcccaggcgcccggtgcagtggaagggccggcgcgtaaagcgcgtcctgcgccccggcaccgcggtggtcttcacgcccggcgagcgctccacccggactttcaagcgcgtctatgacgaggtgtacggcgacgaagacctgctggagcaggccaacgagcgcttcggagagtttgcttacgggaagcgtcagcgggcgctggggaaggaggacctgctggcgctgccgctggaccagggcaaccccacccccagtctgaagcccgtgaccctgcagcaggtgctgccgagcagcgcaccctccgaggcgaagcggggtctgaagcgcgagggcggcgacctggcgcccaccgtgcagctcatggtgcccaagcggcagaggctggaggatgtgctggagaaaatgaaagtagaccccggtctgcagccggacatcagggtccgtcccatcaagcaggtggcgccgggcctcggcgtgcagaccgtggacgtggtcatccccaccggcaactcccccgccgccaccaccactaccgctgcctccacggacatggagacacagaccgatcccgccgcagccgcagccgccgccgcagccgcgacctcctcggcggaggtgcagacggacccctggctgccgccggcgatgtcagctccccgcgcgcgccgcggacgcagaaagtacggcgccgccaacgcgctcctgcccgagtacgccttgcatccttccatcgcgcccacccccggctaccgaggctatacctaccgcccgcgaagagccaagggttccacccgccgtccccgccgacgcgccgccgccaccacccgccgccgccgccgcagacgccagcccgcactggctccagtctccgtgaggagagtggcgcgcgacggacacaccctggtgctgcccagggcgcgctaccaccccagcatcgtttaaaagcctgttgtggttcttgcagatatggccctcacttgccgcctccgtttcccggtgccgggataccgaggaggaagatcgcgccgcaggaggggtctggccggccgcggcctgagcggaggcagccgccgcgcgcaccggcggcgacgcgccaccagccgacgcatgcgcggcggggtgctgcccctgttaatccccctgatcgccgcggcgatcggcgccgtgcccgggatcgcctccgtggccttgcaagcgtcccagaggcattgacagacttgcaaacttgcaaatatggaaaaaaaaaaaaaaccccaataaaaagtctagactctcacgctcgcttggtcctgtgactattttgtagaatggaagacatcaactttgcgtcgctggccccgcgtcacggctcgcgcccgttcctgggacactggaacgatatcggcaccagcaacatgagcggtggcgccttcagttggggctctctgtggagcggcattaaaagtatcgggtctgccgttaaaaattacggctcccgggcctggaacagcagcacgggccagatgttgagagacaagttgaaagagcagaacttccagcagaaggtggtggagggcctggcctccggcatcaacggggtggtggacctggccaaccaggccgtgcagaataaaatcaacagcagactggacccccggccgccggtggaggaggtgccgccggcgctggagacggtgtcccccgatgggcgtggcgagaagcgcccgcggcccgatagggaagagaccactctggtcacgcagaccgatgagccgcccccgtatgaggaggccctaaagcaaggtctgcccaccacgcggcccatcgcgcccatggccaccggggtggtgggccgccacacccccgccacgctggacttgcctccgcccgccgatgtgccgcagcagcagaaggcggcacagccgggcccgcccgcgaccgcctcccgttcctccgccggtcctctgcgccgcgcggccagcggcccccgcgggggggtcgcgaggcacggcaactggcagagcacgctgaacagcatcgtgggtctgggggtgcggtccgtgaagcgccgccgatgctactgaatagcttagctaacgtgttgtatgtgtgtatgcgccctatgtcgccgccagaggagctgctgagtcgccgccgttcgcgcgcccaccaccaccgccactccgcccctcaagatggcgaccccatcgatgatgccgcagtggtcgtacatgcacatctcgggccaggacgcctcggagtacctgagccccgggctggtgcagttcgcccgcgccaccgagagctacttcagcctgagtaacaagtttaggaaccccacggtggcgcccacgcacgatgtgaccaccgaccggtctcagcgcctgacgctgcggttcattcccgtggaccgcgaggacaccgcgtactcgtacaaggcgcggttcaccctggccgtgggcgacaaccgcgtgctggacatggcctccacctactttgacatccgcggggtgctggaccggggtcccactttcaagccctactctggcaccgcctacaactccctggcccccaagggcgctcccaactcctgcgagtgggagcaagaggaaactcaggcagttgaagaagcagcagaagaggaagaagaagatgctgacggtcaagctgaggaagagcaagcagctaccaaaaagactcatgtatatgctcaggctcccctttctggcgaaaaaattagtaaagatggtctgcaaataggaacggacgctacagctacagaacaaaaacctatttatgcagaccctacattccagcccgaaccccaaatcggggagtcccagtggaatgaggcagatgctacagtcgccggcggtagagtgctaaagaaatctactcccatgaaaccatgctatggttcctatgcaagacccacaaatgctaatggaggtcagggtgtactaacggcaaatgcccagggacagctagaatctcaggttgaaatgcaattcttttcaacttctgaaaacgcccgtaacgaggctaacaacattcagcccaaattggtgctgtatagtgaggatgtgcacatggagaccccggatacgcacctttcttacaagcccgcaaaaagcgatgacaattcaaaaatcatgctgggtcagcagtccatgcccaacagacctaattacatcggcttcagagacaactttatcggcctcatgtattacaatagcactggcaacatgggagtgcttgcaggtcaggcctctcagttgaatgcagtggtggacttgcaagacagaaacacagaactgtcctaccagctcttgcttgattccatgggtgacagaaccagatacttttccatgtggaatcaggcagtggacagttatgacccagatgttagaattattgaaaatcatggaactgaagacgagctccccaactattgtttccctctgggtggcataggggtaactgacacttaccaggctgttaaaaccaacaatggcaataacgggggccaggtgacttggacaaaagatgaaacttttgcagatcgcaatgaaataggggtgggaaacaatttcgctatggagatcaacctcagtgccaacctgtggagaaacttcctgtactccaacgtggcgctgtacctaccagacaagcttaagtacaacccctccaatgtggacatctctgacaaccccaacacctacgattacatgaacaagcgagtggtggccccggggctggtggactgctacatcaacctgggcgcgcgctggtcgctggactacatggacaacgtcaaccccttcaaccaccaccgcaatgcgggcctgcgctaccgctccatgctcctgggcaacgggcgctacgtgcccttccacatccaggtgccccagaagttctttgccatcaagaacctcctcctcctgccgggctcctacacctacgagtggaacttcaggaaggatgtcaacatggtcctccagagctctctgggtaacgatctcagggtggacggggccagcatcaagttcgagagcatctgcctctacgccaccttcttccccatggcccacaacacggcctccacgctcgaggccatgctcaggaacgacaccaacgaccagtccttcaatgactacctttccgccgccaacatgctctaccccatacccgccaacgccaccaacgtccccatctccatcccctcgcgcaactgggcggccttccgcggctgggccttcacccgcctcaagaccaaggagaccccctccctgggctcgggattcgacccctactacacctactcgggctctattccctacctggacggcaccttctacctcaaccacactttcaagaaggtctcggtcaccttcgactcctcggtcagctggccgggcaacgaccgtctgctcacccccaacgagttcgagatcaagcgctcggtcgacggggaaggctacaacgtggcccagtgcaacatgaccaaggactggttcctggtccagatgctggccaactacaacatcggctaccagggcttctacatcccagagagctacaaggacaggatgtactccttcttcaggaacttccagcccatgagccggcaggtggtggaccagaccaagtacaaggactaccaggaggtgggcatcatccaccagcacaacaactcgggcttcgtgggctacctcgcccccaccatgcgcgagggacaggcctaccccgccaacttcccctacccgctcataggcaagaccgcggtcgacagcatcacccagaaaaagttcctctgcgaccgcaccctctggcgcatccccttctccagcaacttcatgtccatgggtgcgctctcggacctgggccagaacttgctctacgccaactccgcccacgccctcgacatgaccttcgaggtcgaccccatggacgagcccacccttctctatgttctgttcgaagtctttgacgtggtccgggtccaccagccgcaccgcggcgtcatcgagaccgtgtacctgcgtacgcccttctcggccggcaacgccaccacctaaagaagcaagccgcagtcatcgccgcctgcatgccgtcgggttccaccgagcaagagctcagggccatcgtcagagacctgggatgcgggccctattttttgggcaccttcgacaagcgcttccctggctttgtctccccacacaagctggcctgcgccatcgtcaacacggccggccgcgagaccgggggcgtgcactggctggcctttgcctggaacccgcgctccaaaacatgcttcctctttgaccccttcggcttttcggaccagcggctcaagcaaatctacgagttcgagtacgagggcttgctgcgtcgcagcgccatcgcctcctcgcccgaccgctgcgtcaccctcgaaaagtccacccagaccgtgcaggggcccgactcggccgcctgcggtctcttctgctgcatgtttctgcacgcctttgtgcactggcctcagagtcccatggaccgcaaccccaccatgaacttgctgacgggggtgcccaactccatgctccaaagcccccaggtcgagcccaccctgcgccgcaaccaggagcagctctacagcttcctggagcgccactcgccctacttccgccgccacagcgcacagatcaggagggccacctccttctgccacttgcaagagatgcaagaagggtaataacgatgtacacacttttttctcaataaatggcattttttttttatttatacaagctctctggggtattcatttcccaccaccaccacccgccgttgtcgccatctggctctatttagaaatcgaaagggttctgccgggagtcgccgtgcgccacgggcagggacacgttgcgatactggtagcgggtgccccacttgaactcgggcaccaccaggcgaggcagctcggggaagttttcgctccacaggctgcgggtcagcaccagcgcgttcatcaggtcgggcgccgagatcttgaagtcgcagttggggccgccgccctgcgcgcgcgagttgcggtacaccgggttgcagcactggaacaccaacagcgccgggtgcttcacgctggccagcacgctgcggtcggagatcagctcggcgtccaggtcctccgcgttgctcagcgcgaacggggtcatcttgggcacttgccgccccaggaagggcgcgtgccccggtttcgagttgcagtcgcagcgcagcgggatcagcaggtgcccgtgcccggactcggcgttggggtacagcgcgcgcatgaaggcctgcatctggcggaaggccatctgggccttggcgccctccgagaagaacatgccgcaggacttgcccgagaactggtttgcggggcagctggcgtcgtgcaggcagcagcgcgcgtcggtgttggcgatctgcaccacgttgcgcccccaccggttcttcacgatcttggccttggacgattgctccttcagcgcgcgctgcccgttctcgctggtcacatccatctcgatcacatgttccttgttcaccatgctgctgccgtgcagacacttcagctcgccctccgtctcggtgcagcggtgctgccacagcgcgcagcccgtgggctcgaaagacttgtaggtcacctccgcgaaggactgcaggtacccctgcaaaaagcggcccatcatggtcacgaaggtcttgttgctgctgaaggtcagctgcagcccgcggtgctcctcgttcagccaggtcttgcacacggccgccagcgcctccacctggtcgggcagcatcttgaagttcaccttcagctcattctccacgtggtacttgtccatcagcgtgcgcgccgcctccatgcccttctcccaggccgacaccagcggcaggctcacggggttcttcaccatcaccgtggccgccgcctccgccgcgctttcgctttccgccccgctgttctcttcctcttcctcctcttcctcgccgccgcccactcgcagcccccgcaccacggggtcgtcttcctgcaggcgctgcaccttgcgcttgccgttgcgcccctgcttgatgcgcacgggcgggttgctgaagcccaccatcaccagcgcggcctcttcttgctcgtcctcgctgtccagaatgacctccggggagggggggttggtcatcctcagtaccgaggcacgcttctttttcttcctgggggcgttcgccagctccgcggctgcggccgctgccgaggtcgaaggccgagggctgggcgtgcgcggcaccagcgcgtcttgcgagccgtcctcgtcctcctcggactcgagacggaggcgggcccgcttcttcgggggcgcgcggggcggcggaggcggcggcggcgacggagacggggacgagacatcgtccagggtgggtggacggcgggccgcgccgcgtccgcgctcgggggtggtttcgcgctggtcctcttcccgactggccatctcccactgctccttctcctataggcagaaagagatcatggagtctctcatgcgagtcgagaaggaggaggacagcctaaccgccccctctgagccctccaccaccgccgccaccaccgccaatgccgccgcggacgacgcgcccaccgagaccaccgccagtaccaccctccccagcgacgcacccccgctcgagaatgaagtgctgatcgagcaggacccgggttttgtgagcggagaggaggatgaggtggatgagaaggagaaggaggaggtcgccgcctcagtgccaaaagaggataaaaagcaagaccaggacgacgcagataaggatgagacagcagtcgggcgggggaacggaagccatgatgctgatgacggctacctagacgtgggagacgacgtgctgcttaagcacctgcaccgccagtgcgtcatcgtctgcgacgcgctgcaggagcgctgcgaagtgcccctggacgtggcggaggtcagccgcgcctacgagcggcacctcttcgcgccgcacgtgccccccaagcgccgggagaacggcacctgcgagcccaacccgcgtctcaacttctacccggtcttcgcggtacccgaggtgctggccacctaccacatcttcttccaaaactgcaagatccccctctcctgccgcgctaaccgcacccgcgccgacaaaaccctgaccctgcggcagggcgcccacatacctgatattgcctctctggaggaagtgcccaagatcttcgagggtctcggtcgcgacgagaaacgggcggcgaacgctctgcacggagacagcgaaaacgagagtcactcgggggtgctggtggagctcgagggcgacaacgcgcgcctggccgtactcaagcgcagcatagaggtcacccactttgcctacccggcgctcaacctgccccccaaggtcatgagtgtggtcatgggcgagctcatcatgcgccgcgctcagcccctggccgcggatgcaaacttgcaagagtcctccgaggaaggcctgcccgcggtcagcgacgagcagctagcgcgctggctggagacccgcgaccccgcgcagctggaggagcggcgcaagctcatgatggccgcggtgctggtcaccgtggagctcgagtgtctgcagcgcttcttcgcggaccccgagatgcagcgcaagctcgaggagaccctgcactacaccttccgccagggctacgtgcgccaggcctgcaagatctccaacgtggagctctgcaacctggtctcctacctgggcatcctgcacgagaaccgcctcgggcagaacgtcctgcactccaccctcaaaggggaggcgcgccgcgactacatccgcgactgcgcctacctcttcctctgctacacctggcagacggccatgggggtctggcagcagtgcctggaggagcgcaacctcaaggagctggaaaagctactcaagcgcaccctcagggacctctggacgggcttcaacgagcgctcggtggccgccgcgctggcggacatcatcttccccgagcgcctgctcaagaccctgcagcagggcctgcccgacttcaccagccagagcatgctgcagaactttaggactttcatcctggagcgctcgggcatcctgcctgccacttgctgcgcgctgcccagcgacttcgtgcccatcaagtacagggagtgcccgccgccgctctggggccactgctacctcttccagctggccaactacctcgcctaccactcggacctcatggaagacgtgagcggcgagggcctgctcgagtgccactgccgctgcaacctctgcacgccccaccgctctctagtctgcaacccgcagctgctcagcgagagtcagattatcggtaccttcgagctgcagggtccctcgcctgacgagaagtccgcggctccggggctgaaactcactccggggctgtggacttccgcctacctacgcaaatttgtacctgaggactaccacgcccacgagatcaggttctacgaagaccaatcccgcccgcccaaggcggagctcaccgcctgcgtcatcacccaggggcacatcctgggccaattgcaagccatcaacaaagcccgccgagagttcttgctgaaaaagggtcggggggtgtacctggacccccagtccggcgaggagctaaacccgctacccccgccgccgccccagcagcgggaccttgcttcccaggatggcacccagaaagaagcagcagccgccgccgccgcagccatacatgcttctggaggaagaggaggaggactgggacagtcaggcagaggaggtttcggacgaggagcaggaggagatgatggaagactgggaggaggacagcagcctagacgaggaagcttcagaggccgaagaggtggcagacgcaacaccatcaccctcggtcgcagccccctcgccggggcccctgaaatcctccgaacccagcaccagcgctataacctccgctcctccggcgccggcgccacccgcccgcagacccaaccgtagatgggacaccacaggaaccggggtcggtaagtccaagtgcccgccgccgccaccgcagcagcagcagcagcgccagggctaccgctcgtggcgcgggcacaagaacgccatagtcgcctgcttgcaagactgcgggggcaacatctctttcgcccggcgcttcctgctattccaccacggggtcgcctttccccgcaatgtcctgcattactaccgtcatctctacagcccctactgcagcggcgacccagaggcggcagcggcagccacagcggcgaccaccacctaggaagatatcctccgcgggcaagacagcggcagcagcggccaggagacccgcggcagcagcggcgggagcggtgggcgcactgcgcctctcgcccaacgaacccctctcgacccgggagctcagacacaggatcttccccactttgtatgccatcttccaacagagcagaggccaggagcaggagctgaaaataaaaaacagatctctgcgctccctcacccgcagctgtctgtatcacaaaagcgaagatcagcttcggcgcacgctggaggacgcggaggcactcttcagcaaatactgcgcgctcactcttaaagactagctccgcgcccttctcgaatttaggcgggagaaaactacgtcatcgccggccgccgcccagcccgcccagccgagatgagcaaagagattcccacgccatacatgtggagctaccagccgcagatgggactcgcggcgggagcggcccaggactactccacccgcatgaactacatgagcgcgggaccccacatgatctcacaggtcaacgggatccgcgcccagcgaaaccaaatactgctggaacaggcggccatcaccgccacgccccgccataatctcaacccccgaaattggcccgccgccctcgtgtaccaggaaaccccctccgccaccaccgtactacttccgcgtgacgcccaggccgaagtccagatgactaactcaggggcgcagctcgcgggcggctttcgtcacggggcgcggccgctccgaccaggtataagacacctgatgatcagaggccgaggtatccagctcaacgacgagtcggtgagctcttcgctcggtctccgtccggacggaactttccagctcgccggatccggccgctcttcgttcacgccccgccaggcgtacctgactctgcagacctcgtcctcggagccccgctccggaggcatcggaaccctccagttcgtggaggagttcgtgccctcggtctacttcaaccccttctcgggacctcccggacgctaccccgaccagttcattccgaactttgacgcggtgaaggactcggcggacggctacgactgaatgtcaggtgccgaggcagagcagcttcgcctgagacacctcgagcactgccgccgccacaagtgcttcgcccgcggttccggtgagttctgctactttcagctacccgaggagcataccgaggggccggcgcacggcgtccgcctgaccacccagggcgaggttacctgttccctcatccgggagttcaccctccgtcccctgctagtggagcgggagcggggtccctgtgtcctaactatcgcctgcaactgccctaaccctggattacatcaagatctttgctgtcatctctgtgctgagtttaataaacgctgagatcagaatctactggggctcctgtcgccatcctgtgaacgccaccgtcttcacccaccccgaccaggcccaggcgaacctcacctgcggtctgcatcggagggccaagaagtacctcacctggtacttcaacggcaccccctttgtggtttacaacagcttcgacggggacggagtctccctgaaagaccagctctccggtctcagctactccatccacaagaacaccaccctccaactcttccctccctacctgccgggaacctacgagtgcgtcaccggccgctgcacccacctcacccgcctgatcgtaaaccagagctttccgggaacagataactccctcttccccagaacaggaggtgagctcaggaaactccccggggaccagggcggagacgtaccttcgacccttgtggggttaggattttttattaccgggttgctggctcttttaatcaaagcttccttgagatttgttctttccttctacgtgtatgaacacctcagcctccaataactctaccctttcttcggaatcaggtgacttctctgaaatcgggcttggtgtgctgcttactctgttgatttttttccttatcatactcagccttctgtgcctcaggctcgccgcctgctgcgcacacatctatatctactgctggttgctcaagtgcaggggtcgccacccaagatgaacaggtacatggtcctatcgatcctaggcctgctggccctggcggcctgcagcgccgccaaaaaagagattacctttgaggagcccgcttgcaatgtaactttcaagcccgagggtgaccaatgcaccaccctcgtcaaatgcgttaccaatcatgagaggctgcgcatcgactacaaaaacaaaactggccagtttgcggtctatagtgtgtttacgcccggagacccctctaactactctgtcaccgtcttccagggcggacagtctaagatattcaattacactttccctttttatgagttatgcgatgcggtcatgtacatgtcaaaacagtacaacctgtggcctccctctccccaggcgtgtgtggaaaatactgggtcttactgctgtatggctttggcaatcactacgctcgctctaatctgcacggtgctatacataaaattcaggcagaggcgaatctttatcgatgaaaagaaaatgccttgatcgctaacaccggctttctatctgcagaatgaatgcaatcacctccctactaatcaccaccaccctccttgcgattgcccatgggttgacacgaatcgaagtgccagtggggtccaatgtcaccatggtgggccccgccggcaattccaccctcatgtgggaaaaatttgtccgcaatcaatgggttcatttctgctctaaccgaatcagtatcaagcccagagccatctgcgatgggcaaaatctaactctgatcaatgtgcaaatgatggatgctgggtactattacgggcagcggggagaaatcattaattactggcgaccccacaaggactacatgctgcatgtagtcgaggcacttcccactaccacccccactaccacctctcccaccaccactaccaccactactactactactactaccactaccgctgcccgccatacccgcaaaagcaccatgattagcacaaagccccctcgtgctcactcccacgccggcgggcccatcggtgcgacctcagaaaccaccgagctttgcttctgccaatgcactaacgccagcgctcatgaactgttcgacctggagaatgaggatgcccagcagagctccgcttgcctgacccaggaggctgtggagcccgttgccctgaagcagatcggtgattcaataattgactcttcttcttttgccactcccgaataccctcccgattctactttccacatcacgggtaccaaagaccctaacctctctttctacctgatgctgctgctctgtatctctgtggtctcttccgcgctgatgttactggggatgttctgctgcctgatctgccgcagaaagagaaaagctcgctctcagggccaaccactgatgcccttcccctaccccccggattttgcagataacaagatatgagctcgctgctgacactaaccgctttactagcctgcgctctaacccttgtcgcttgcgactcgagattccacaatgtcacagctgtggcaggagaaaatgttactttcaactccacggccgatacccagtggtcgtggagtggctcaggtagctacttaactatctgcaatagctccacttcccccagcatatccccaaccaagtaccaatgcaatgccagcctgttcaccctcatcaacgcttccaccctggacaatggactctatgtaggctatgtaccctttggtgggcaaggaaagacccacgcttacaacctggaagttcgccagcccagaaccactacccaagcttctcccaccaccaccaccaccaccaccaccaccatcaccagcagcagcagcagccacagcagcagcagcagattattgactttggttttggccagctcatctgccgctacccaggccatctacagctctgtgcccgaaaccactcagatccaccgcccagaaacgaccaccgccaccaccctacacacctccagcgatcagatgccgaccaacatcacccccttggctcttcaaatgggacttacaagccccactccaaaaccagtggatgcggccgaggtctccgccctcgtcaatgactgggcggggctgggaatgtggtggttcgccataggcatgatggcgctctgcctgcttctgctctggctcatctgctgcctccaccgcaggcgagccagaccccccatctatagacccatcattgtcctgaaccccgataatgatgggatccatagattggatggcctgaaaaacctacttttttcttttacagtatgataaattgagacatgcctcgcattttcttgtacatgttccttctcccaccttttctggggtgttctacgctggccgctgtgtctcacctggaggtagactgcctctcacccttcactgtctacctgctttacggattggtcaccctcactctcatctgcagcctaatcacagtaatcatcgccttcatccagtgcattgattacatctgtgtgcgcctcgcatacttcagacaccacccgcagtaccgagacaggaacattgcccaacttctaagactgctctaatcatgcataagactgtgatctgccttctgatcctctgcatcctgcccaccctcacctcctgccagtacaccacaaaatctccgcgcaaaagacatgcctcctgccgcttcacccaactgtggaatatacccaaatgctacaacgaaaagagcgagctctccgaagcttggctgtatggggtcatctgtgtcttagttttctgcagcactgtctttgccctcatgatctacccctactttgatttgggatggaacgcgatcgatgccatgaattaccccacctttcccgcacccgagataattccactgcgacaagttgtacccgttgtcgttaatcaacgccccccatcccctacgcccactgaaatcagctactttaacctaacaggcggagatgactgacgccctagatctagaaatggacggcatcagtaccgagcagcgtctcctagagaggcgcaggcaggcggctgagcaagagcgcctcaatcaggagctccgagatctcgttaacctgcaccagtgcaaaagaggcatcttttgtctggtaaagcaggccaaagtcacctacgagaagaccggcaacagccaccgcctcagttacaaattgcccacccagcgccagaagctggtgctcatggtgggtgagaatcccatcaccgtcacccagcactcggtagagaccgaggggtgtctgcactctccctgtcggggtccagaagacctctgcaccctggtaaagaccctgtgcggtctcagagatttagtcccctttaactaatcaaacactggaatcaataaaaagaatcacttacttaaaatcagacagcaggtctctgtccagtttattcagcagcacctccttcccctcctcccaactctggtactccaaacgccttctggcggcaaacttcctccacaccctgaagggaatgtcagattcttgctcctgtccctccgcacccactatcttcatgttgttgcagatgaagcgcaccaaaacgtctgacgagagcttcaaccccgtgtacccctatgacacggaaagcggccctccctccgtccctttcctcacccctcccttcgtgtctcccgatggattccaagaaagcccccccggggtcctgtctctgaacctggccgagcccctggtcacttcccacggcatgctcgccctgaaaatgggaagtggcctctccctggacgacgctggcaacctcacctctcaagatatcaccaccgctagccctcccctcaaaaaaaccaagaccaacctcagcctagaaacctcatcccccctaactgtaagcacctcaggcgccctcaccgtagcagccgccgctcccctggcagtggccggcacctccctcaccatgcaatcagaggcccccctgacagtacaggatgcaaaactcaccctggccaccaaaggccccctgaccgtgtctgaaggcaaactggccttgcaaacatcggccccgctgacggccgctgacagcagcaccctcaccgttagcgccacaccaccaattaatgtaagcagtggaagtttaggcttagacatggaagaccctatgtatactcacgatggaaaactgggaataagaattgggggtccactaagagtagtagacagcttgcacacactcactgtagttaccggaaatggactaactgtagataacaatgccctccaaactagagttacgggcgccctaggttatgacacatcaggaaatctacaattgagagctgcaggaggtatgcgaattgatgcaaatggccaacttatccttaatgtggcatacccatttgatgctcagaacaatctcagccttagacttggtcagggacccctgtatataaacacagaccacaacctggatttgaattgcaacagaggtctaaccacaactaccaccaacaacacaaaaaaacttgagactaaaattagctcaggcttagactatgacaccaatggtgctgtcattattaaacttggcactggtctaagcttcgacaacacaggcgccctaactgtgggaaacactggtgatgataaactgactctgtggacgaccccagacccatctccaaattgcagaattcactcagacaaagactgcaagtttactctagtcctaactaagtgtggaagccaaatcctggcctctgtcgccgccctagcggtatcaggaaatctggcttcgataacaggcaccgttgccagcgttaccatctttctcagatttgatcagaatggagtgcttatggaaaactcctcgctagacaggcagtactggaacttcagaaatggcaactcaactaacgctgccccctacaccaatgcagttgggttcatgccaaacctcgcagcataccccaaaacgcaaagccagactgctaaaaacaacattgtaagtcaggtttacttgaatggagacaaatccaaacccatgacccttaccatcaccctcaatggaactaatgaatccagtgaaactagccaggtgagtcactactccatgtcatttacatgggcttgggaaagtgggcaatatgccactgaaacctttgccaccaactccttcaccttttcttacattgctgaacaataaaaagcatgacactgatgttcatttctgattcttattttattattttcaaacacaacaaaatcattcaagtcattcttccatcttagcttaatagacacagtagcttaatagacccagtagtgcaaagccccattctagcttatagatcagacagtgataattaaccaccaccaccaccataccttttgattcaggaaatcatgatcatcacaggatcctagtcttcaggccgccccctccctcccaagacacagaatacacagtcctctccccccgactggctttaaataacaccatctggttggtcacagacatgttcttaggggttatattccacacggtctcctgccgcgccaggcgctcgtcggtgatgttgataaactctcccggcagctcgctcaagttcacgtcgctgtccagcggctgaacctccggctgacgcgataactgtgcgaccggctgctggacaaacggaggccgcgcctacaagggggtagagtcataatcctcggtcaggatagggcggtgatgcagcagcagcgagcgaaacatctgctgccgccgccgctccgtccggcaggaaaacaacaagccggtggtctcctccgcgataatccgcaccgcccgcagcatcagcttcctcgttctccgcgcgcagcacctcaccctgatctcgctcaagtcggcgcagtaggtacagcacagcaccacgatgttattcatgatcccacagtgcagggcgctgtatccaaagctcatgccgggaaccaccgcccccacgtggccatcgtaccacaagcgcacgtaaattaagtgtcgacccctcatgaacgtgctggacacaaacattacttccttgggcatgttgtaattcaccacctcccggtaccagataaacctctggttaaacagggcaccttccaccaccatcctgaaccaagaggccagaacctgcccaccggctatgcactgcagggaacccgggttggaacaatgacaatgcagactccaaggctcgtaaccgtggatcatccggctgctgaaggcatcgatgttggcacaacacagacacacgtgcatgcactttctcatgattagcagctcttccctcgtcaggatcatatcccaaggaataacccattcttgaatcaacgtaaaacccacacagcagggaaggcctcgcacataactcacgttgtgcatggtcagcgtgttgcattctggaaacagcggatgatcctccagtatcgaggcgcgggtctccttctcacagggaggtaaagggtccctgctgtacggactgcgccgggacgaccgagatcgtgttgagcgtagtgtcatggaaaagggaacgccggacgtggtcatacttcttgaagcagaaccaggttcgcgcgtggcaggcctccttgcgtctgcggtctcgccgtctagctcgctccgtgtgatagttgtagtacagccactcccgcagagcgtcgaggcgcaccctggcttccggatctatgtagactccgtcttgcaccgcggccctgataatatccaccaccgtagaataagcaacacccagccaagcaatacactcgctctgcgagcggcagacaggaggagcgggcagagatgggagaaccatgataaaaaactttttttaaagaatattttccaattcttcgaaagtaagatctatcaagtggcagcgctcccctccactggcgcggtcaaactctacggccaaagcacagacaacggcatttctaagatgttccttaatggcgtccaaaagacacaccgctctcaagttgcagtaaactatgaatgaaaacccatccggctgattttccaatatagacgcgccggcggcgtccaccaaacccagataattttcttctctccagcggtttagaatctgtctaagcaaatcccttatatcaagtccggccatgccaaaaatctgctcaagagcgccctccaccttcatgaccaagcagcgcatcatgattgcaaaaattcaggttcttcagagacctgtataagattcaaaatgggaacattaacaaaaattcctctgtcgcgcagatcccttcgcagggcaagctgaacataatcagacaggtctgaacggaccagtgaggccaaatccccaccaggaaccagatccagagaccctatactgattatgacgcgcatactcggggctatgctgaccagcgtagcgccgatgtaggcgtgctgcatgggcggcgagataaaatgcaaagtgctggttaaaaaatcaggcaaagcctcgcgcaaaaaagctaacacatcataatcatgctcatgcaggtagttgcaggtaagctcaggaaccaaaacggaataacacacgattttcctctcaaacatgacttcgcggatactgcgtaaaacaaaaattataaataaaaaattaattaacttaaacattggaagcctgtctcacaacaggaaaaaccactttaatcaacataagacgggccacgggcatgccggcatagccgtaaaaaaattggtccccgtgattaacaagtaccacagacagctccccggtcatgtcgggggtcatcatgtgagactctgtatacacgtctggattgtgaacatcagacaaacaaagaaatcgagccacgtagcccggaggtataatcacccgcaggcggaggtacagcaaaacgacccccataggaggaatcacaaaattagtaggagaaaaaaatacataaacaccagaaaaaccctgttgctgaggcaaaatagcgccctcccgatccaaaacaacataaagcgcttccacaggagcagccataacaaagacccgagtcttaccagtaaaagaaaaaagatctctcaacgcagcaccagcaccaacacttcgcagtgtaaaaggccaagtgccgagagagtatatataggaataaaaagtgacgtaaacgggcaaagtccaaaaaacgcccagaaaaaccgcacgcgaacctacgccccgaaacgaaagccaaaaaacactagacactcccttccggcgtcaacttccgctttcccacgctacgtcacttgccccagtcaaacaaactacatatcccgaacttccaagtcgccacgcccaaaacaccgcctacacctccccgcccgccggcccgcccccaaacccgcctcccgccccgcgccccgcctcgcgccgcccatctcattatcatattggcttcaatccaaaataaggtatattattgatgatg

SEQ ID NO: 15 - DNA, 36643 bp, Chimpanzee adenovirus type 63
catcatcaataatatacctcaaacttttggtgcgcgttaatatgcaaatgaggtgtttgaatttggggatgcggggcgctgattggctgagagacgggcgaccgttaggggcggggcgggtgacgttttgatgacgtggccgtgaggcggagccggtttgcaagttctcgtgggaaaagtgacgtcaaacgaggtgtggtttgaacacggaaatactcaattttcccgcgctctctgacaggaaatgaggtgtttctgggcggatgcaagtgaaaacgggccattttcgcgcgaaaactgaatgaggaagtgaaaatctgagtaattccgcgtttatggcagggaggagtatttgccgagggccgagtagactttgaccgattacgtgggggtttcgattaccgtatttttcacctaaatttccgcgtacggtgtcaaagtccggtgtttttacgtaggcgtcagctgatcgccagggtatttaaacctgcgctctctagtcaagaggccactcttgagtgccagcgagtagagttttctcctccgcgccgcgagtcagatctacactttgaaagatgaggcacctgagagacctgcccggtaatgttttcctggctactgggaacgagattctggaactggtggtggacgccatgatgggtgacgaccctcccgagccccctaccccatttgaggcgccttcgctgtacgatttgtatgatctggaggtggatgtgcccgagaacgaccccaacgaggaggcggtgaatgatttgtttagcgatgccgcgctgctggctgccgagcaggctaatacggactctggctcagacagcgattcctctcttcataccccgagacccggcagaggtgagaaaaagatccccgagcttaaaggggaagagctcgacctgcgctgctatgaggaatgcttgcctccgagcgatgatgaggaggacgaggaggcgattcgagctgcagcgagcgagggagtgaaagttgcgggcgagagctttagcctggactgtcctactctgcccggacacggctgtaagtcttgtgaatttcatcgcatgaatactggagataagaatgtgatgtgtgccctgtgctatatgagagcttacaaccattgtgtttacagtaagtgtgattaactttagttgggaaggcagagggtgactgggtgctgactggtttatttatgtatatgtttttttatgtgtaggtcccgtctctgacgtagatgagacccccacttcagagtgcatttcatcacccccagaaattggcgaggaaccgcccgaagatattattcatagaccagttgcagtgagagtcaccgggcggagagcagctgtggagagtttggatgacttgctacagggtggggatgaacctttggacttgtgtacccggaaacgccccaggcactaagtgccacacatgtgtgtttacttaaggtgatgtcagtatttatagggtgtggagtgcaataaaaatatgtgttgactttaagtgcgtggtttatgactcaggggtggggactgtgggtatataagcaggtgcagacctgtgtggtcagttcagagcaggactcatggagatctggacggtcttggaagactttcaccagactagacagctgctagagaactcatcggcggaagtctcttacctgtggagattctgcttcggtgggcctctagctaagctagtctatagggccaagcaggattataaggatcaatttgaggatattttgagagagtgtcctggtatttttgactctctcaacttgggccatcagtctcactttaaccagagtattctgagagcccttgacttttccactcctggcagaactaccgccgcggtagccttttttgcctttatccttgacaaatggagtcaagaaacccatttcagcagggattaccgtctggactgcttagcagtagctttgtggagaacatggaggtgccagcgcctgaatgcaatctccggctacttgccagtacagccggtagacacgctgaggatcctgagtctccagtcaccccaggaacaccaacgccgccagcagccgcagcaggagcagcagcaagaggaggaggaggaccgagaagagaacctgagagccggtctggaccctccggtggcggaggaggaggagtagctgacttgtttcccgagctgcgccgggtgctgactaggtcttccagtggacgggagagggggattaagcgggagaggcatgaggagactagccacagaactgaactgactgtcagtctgatgagccgcaggcgcccagaatcggtgtggtggcatgaggtgcagtcgcaggggatagatgaggtctcagtgatgcatgagaaatattccctagaacaagtcaagacttgttggttggagcctgaggatgattgggaggtagccatcaggaattatgccaagctggctctgaagccagacaagaagtacaagattaccaaactgattaatatcagaaattcctgctacatttcagggaatggggccgaggtggagatcagtacccaggagagggcggccttcagatgttgtatgatgaatatgtacccgggggtggtgggcatggagggagtcacctttatgaacacgaggttcaggggtgatgggtataatggggtggtctttatggccaacaccaagttgacagtgcacggatgctccttctttggcttcaataacatgtgcatcgaggcctggggcagtgtttcagtgaggggatgcagcttttcagccaactggatgggggtcgtgggcagaaccaagagcgtggtttcagtgaagaaatgcctgtttgagaggtgccacctgggggtgatgagcgagggcgaagccaaagtcaaacactgcgcctctaccgagacgggctgctttgtgctgatcaagggcaatgccaaagtcaagcataacatgatctgtggggcctcggatgagcgcggctaccagatgctgacctgcgccggtgggaacagccatatgctggccaccgtgcatgtggcctcgcacccccgcaagacatggcccgagttcgagcacaacgtcatgacccgctgcaatgtgcacctggggtcccgccgaggcatgttcatgccctaccagtgcaacatgcaatttgtgaaggtgctgctggagcccgatgccatgtccagagtgagcctgacgggggtgtttgacatgaatgtggagctgtggaaaattctgagatatgatgaatccaagaccaggtgccgggcctgcgaatgcggaggcaagcacgccaggcttcagcccgtgtgtgtggaggtgacggaggacctgcgacccgatcatttggtgttgtcctgcaacgggacggagttcggctccagcggggaagaatctgactagagtgagtagtgtttgggggtgggtgggagcctgcatgatgggcagaatgactaaaatctgtgtttttctgtgtgttgcagcagcatgagcggaagcgcctcctttgagggaggggtattcagcccttatctgacggggcgtctcccctcctgggcgggagtgcgtcagaatgtgatgggatccacggtggacggccggcccgtgcagcccgcgaactcttcaaccctgacctacgcgaccctgagctcctcgtccgtggacgcagctgccgccgcagctgctgcttccgccgccagcgccgtgcgcggaatggccctgggcgccggctactacagctctctggtggccaactcgagttccaccaataatcccgccagcctgaacgaggagaagctgttgctgctgatggcccagctcgaggccctgacccagcgcctgggcgagctgacccagcaggtggctcagctgcaggcggagacgcgggccgcggttgccacggtgaaaaccaaataaaaaatgaatcaataaataaacggagacggttgttgattttaacacagagtcttgaatctttatttgatttttcgcgcgcggtaggccctggaccaccggtctcgatcattgagcacccggtggatcttttccaggacccggtagaggtgggcttggatgttgaggtacatgggcatgagcccgtcccgggggtggaggtagctccattgcagggcctcgtgctcgggggtggtgttgtaaatcacccagtcatagcaggggcgcagggcgtggtgctgcacgatgtctttgaggaggagactgatggccacgggcagccccttggtgtaggtgttgacgaacctattgagctgggagggatgcatgcggggggagatgagatgcatcttggcctggatcttgagattggcgatgttcccgcccagatcccgccgggggttcatgttgtgcaggaccaccagcacggtgtatccggtgcacttggggaatttgtcatgcaacttggaagggaaggcgtgaaagaatttggagacgcccttgtgaccgcccaggttttccatgcactcatccatgatgatggcgatgggcccgtgggcggcggcctgggcaaagacgtttcgggggtcggacacatcgtagttgtggtcctgggtgagctcgtcataggccattttaatgaatttggggcggagggtacccgactgggggacaaaggtgccctcgatcccgggggcgtagttcccctcgcagatctgcatctcccaggccttgagctcggagggggggatcatgtccacctgcggggcgatgaaaaaaacggtttccggggcgggggagatgagctgcgccgaaagcaggttccggagcagctgggacttgccgcagccggtggggccgtagatgaccccgatgaccggctgcaggtggtagttgagggagagacagctgccgtcctcgcggaggaggggggccacctcgttcatcatctcgcgcacatgcatgttctcgcgcacgagttccgccaggaggcgctcgccccccagcgagaggagctcttgcagcgaggcgaagtttttcagcggcttgagcccgtcggccatgggcattttggagagggtctgttgcaagagttccagacggtcccagagctcggtgatgtgctctagggcatctcgatccagcagacctcctcgtttcgcgggttggggcgactgcgggagtagggcaccaggcgatgggcgtccagcgaggccagggtccggtccttccagggtcgcagggtccgcgtcagcgtggtctccgtcacggtgaaggggtgcgcgccgggctgggcgcttgcgagggtgcgcttcaggctcatccggctggtcgagaaccgctcccggtcggcgccctgcgcgtcggccaggtagcaattgagcatgagttcgtagttgagcgcctcggccgcgtggcccttggcgcggagcttacctttggaagtgtgtccgcagacgggacagaggagggacttgagggcgtagagcttgggggcgaggaagacggactcgggggcgtaggcgtccgcgccgcagctggcgcagacggtctcgcactccacgagccaggtgaggtcggggcggtcggggtcaaaaacgaggtttcctccgtgctttttgatgcgtttcttacctctggtctccatgagctcgtgtccccgctgggtgacaaagaggctgtccgtgtccccgtagaccgactttatgggccggtcctcgagcggggtgccgcggtcctcgtcgtagaggaaccccgcccactccgagacgaaggcccgggtccaggccagcacgaaggaggccacgtgggaggggtagcggtcgttgtccaccagcgggtccaccttctccagggtatgcaagcacatgtccccctcgtccacatccaggaaggtgattggcttgtaagtgtaggccacgtgaccgggggtcccggccgggggggtataaaagggggcgggcccctgctcgtcctcactgtcttccggatcgctgtccaggagcgccagctgttggggtaggtattccctctcgaaggcgggcatgacctcggcactcaggttgtcagtttctagaaacgaggaggatttgatattgacggtgccgttggagacgcctttcatgagcccctcgtccatctggtcagaaaagacgatctttttgttgtcgagcttggtggcgaaggagccgtagagggcgttggagagcagcttggcgatggagcgcatggtctggttcttttccttgtcggcgcgctccttggcggcgatgttgagctgcacgtactcgcgcgccacgcacttccattcggggaagacggtggtgagctcgtcgggcacgattctgacccgccagccgcggttgtgcagggtgatgaggtccacgctggtggccacctcgccgcgcaggggctcgttggtccagcagaggcgcccgcccttgcgcgagcagaaggggggcagcgggtccagcatgagctcgtcgggggggtcggcgtccacggtgaagatgccgggcaggagctcggggtcgaagtagctgatgcaggtgcccagatcgtccagacttgcttgccagtcgcgcacggccagcgcgcgctcgtaggggctgaggggcgtgccccagggcatggggtgcgtgagcgcggaggcgtacatgccgcagatgtcgtagacgtagaggggctcctggaggacgccgatgtaggtggggtagcagcgccccccgcggatgctggcgcgcacgtagtcgtacagctcgtgcgagggcgcgaggagccccgtgccgagattggagcgctgcggcttttcggcgcggtagacgatctggcggaagatggcgtgggagttggaggagatggtgggcctctggaagatgttgaagtgggcatggggcagtccgaccgagtccctgatgaagtgggcgtaggagtcctgcagcttggcgacgagctcggcggtgacgaggacgtccagggcgcagtagtcgagggtctcttggatgatgtcgtacttgagctggcccttctgcttccacagctcgcggttgagaaggaactcttcgcggtccttccagtactcttcgagggggaacccgtcctgatcggcacggtaagagcccaccatgtagaactggttgacggccttgtaggcgcagcagcccttctccacggggagggcgtaagcttgcgcggccttgcgcagggaggtgtgggtgagggcgaaggtgtcgcgcaccatgactttgaggaactggtgcttgaagtcgaggtcgtcgcagccgccctgctcccagagctggaagtccgtgcgcttcttgtaggcggggttgggcaaagcgaaagtaacatcgttgaagaggatcttgcccgcgcggggcatgaagttgcgagtgatgcggaaaggctggggcacctcggcccggttgttgatgacctgggcggcgaggacgatctcgtcgaagccgttgatgttgtgcccgacgatgtagagttccacgaatcgcgggcggcccttgacgtggggcagcttcttgagctcgtcgtaggtgagctcggcggggtcgctgagcccgtgctgctcgagggcccagtcggcgacgtgggggttggcgctgaggaaggaagtccagagatccacggccagggcggtctgcaagcggtcccggtactgacggaactgctggcccacggccattttttcgggggtgacgcagtagaaggtgcgggggtcgccgtgccagcggtcccacttgagctggagggcgaggtcgtgggcgagctcgacgagcggcgggtccccggagagtttcatgaccagcatgaaggggacgagctgcttgccgaaggaccccatccaggtgtaggtttccacatcgtaggtgaggaagagcctttcggtgcgaggatgcgagccgatggggaagaactggatctcctgccaccagttggaggaatggctgttgatgtgatggaagtagaaatgccgacggcgcgccgagcactcgtgcttgtgtttatacaagcgtccgcagtgctcgcaacgctgcacgggatgcacgtgctgcacgagctgtacctgggttcctttgacgaggaatttcagtgggcagtggagcgctggcggctgcatctggtgctgtactacgtcctggccatcggcgtggccatcgtctgcctcgatggtggtcatgctgacgagcccgcgcgggaggcaggtccagacctcggctcggacgggtcggagagcgaggacgagggcgcgcaggccggagctgtccagggtcctgagacgctgcggagtcaggtcagtgggcagcggcggcgcgcggttgacttgcaggagcttttccagggcgcgcgggaggtccagatggtacttgatctccacggcgccgttggtggcgacgtccacggcttgcagggtcccgtgcccctggggcgccaccaccgtgccccgtttcttcttgggcggcggcggctccatgcttagaagcggcggcgaggacgcgcgccgggcggcaggggcggctcggggcccggaggcaggggcggcaggggcacgtcggcgccgcgcgcgggcaggttctggtactgcgcccggagaagactggcgtgagcgacgacgcgacggttgacgtcctggatctgacgcctctgggtgaaggccacgggacccgtgagtttgaacctgaaagagagttcgacagaatcaatctcggtatcgttgacggcggcctgccgcaggatctcttgcacgtcgcccgagttgtcctggtaggcgatctcggtcatgaactgctcgatctcctcctcctgaaggtctccgcggccggcgcgctcgacggtggccgcgaggtcgttggagatgcggcccatgagctgcgagaaggcgttcatgccggcctcgttccagacgcggctgtagaccacggctccgtcggggtcgcgcgcgcgcatgaccacctgggcgaggttgagctcgacgtggcgcgtgaagaccgcgtagttgcagaggcgctggtagaggtagttgagcgtggtggcgatgtgctcggtgacgaagaagtacatgatccagcggcggagcggcatctcgctgacgtcgcccagggcttccaagcgctccatggcctcgtagaagtccacggcgaagttgaaaaactgggagttgcgcgccgagacggtcaactcctcctccagaagacggatgagctcggcgatggtggcgcgcacctcgcgctcgaaggccccggggggctcctcttccatttcctcctcttcctcctccactaacatctcttctacttcctcctcaggaggcggcggcgggggaggggccctgcgtcgccggcggcgcacgggcagacggtcgatgaagcgctcgatggtctccccgcgccggcgacgcatggtctcggtgacggcgcgcccgtcctcgcggggccgcagcgtgaagacgccgccgcgcatctccaggtggccgccgggggggtctccgttgggcagggagagggcgctgacgatgcatcttatcaattgacccgtagggactccgcgcaaggacctgagcgtctcgagatccacgggatccgaaaaccgctgaacgaaggcttcgagccagtcgcagtcgcaaggtaggctgagcccggtttcttgttcttcgggtatttggtcgggaggcgggcgggcgatgctgctggtgatgaagttgaagtaggcggtcctgagacggcggatggtggcgaggagcaccaggtccttgggcccggcttgctggatgcgcagacggtcggccatgccccaggcgtggtcctgacacctggcgaggtccttgtagtagtcctgcatgagccgctccacgggcacctcctcctcgcccgcgcggccgtgcatgcgcgtgagcccgaacccgcgctgcggctggacgagcgccaggtcggcgacgacgcgctcggcgaggatggcctgctggatctgggtgagggtggtctggaagtcgtcgaagtcgacgaagcggtggtaggctccggtgttgatggtgtaggagcagttggccatgacggaccagttgacggtctggtggccggggcgcacgagctcgtggtacttgaggcgcgagtaggcgcgcgtgtcgaagatgtagtcgttgcaggtgcgcacgaggtactggtatccgacgaggaagtgcggcggcggctggcggtagagcggccatcgctcggtggcgggggcgccgggcgcgaggtcctcgagcatgaggcggtggtagccgtagatgtacctggacatccaggtgatgccggcggcggtggtggaggcgcgcgggaactcgcggacgcggttccagatgttgcgcagcggcaggaagtagttcatggtggccgcggtctggcccgtgaggcgcgcgcagtcgtggatgctctagacatacgggcaaaaacgaaagcggtcagcggctcgactccgtggcctggaggctaagcgaacgggttgggctgcgcgtgtaccccggttcgaatctcgaatcaggctggagccgcagctaacgtggtactggcactcccgtctcgacccaagcctgctaacgaaacctccaggatacggaggcgggtcgttttttggccttggtcgctggtcatgaaaaactagtaagcgcggaaagcggccgcccgcgatggctcgctgccgtagtctggagaaagaatcgccagggttgcgttgcggtgtgccccggttcgagcctcagcgctcggcgccggccggattccgcggctaacgtgggcgtggctgccccgtcgtttccaagaccccttagccagccgacttctccagttacggagcgagcccctctttttttcttgtgtttttgccagatgcatcccgtactgcggcagatgcgcccccaccctccaccacaaccgcccctaccgcagcagcagcaacagccggcgcttctgcccccgccccagcagcagcagccagccactaccgcggcggccgccgtgagcggagccggcgttcagtatgacctggccttggaagagggcgaggggctggcgcggctgggggcgtcgtcgccggagcggcacccgcgcgtgcagatgaaaagggacgctcgcgaggcctacgtgcccaagcagaacctgttcagagacaggagcggcgaggagcccgaggagatgcgcgcctcccgcttccacgcggggcgggagctgcggcgcggcctggaccgaaagcgggtgctgagggacgaggatttcgaggcggacgagctgacggggatcagccccgcgcgcgcgcacgtggccgcggccaacctggtcacggcgtacgagcagaccgtgaaggaggagagcaacttccaaaaatccttcaacaaccacgtgcgcacgctgatcgcgcgcgaggaggtgaccctgggcctgatgcacctgtgggacctgctggaggccatcgtgcagaaccccacgagcaagccgctgacggcgcagctgtttctggtggtgcagcacagtcgggacaacgagacgttcagggaggcgctgctgaatatcaccgagcccgagggccgctggctcctggacctggtgaacattctgcagagcatcgtggtgcaggagcgcgggctgccgctgtccgagaagctggcggccatcaacttctcggtgctgagcctgggcaagtactacgctaggaagatctacaagaccccgtacgtgcccatagacaaggaggtgaagatcgatgggttttacatgcgcatgaccctgaaagtgctgaccctgagcgacgatctgggggtgtaccgcaacgacaggatgcaccgcgcggtgagcgccagccgccggcgcgagctgagcgaccaggagctgatgcacagcctgcagcgggccctgaccggggccgggaccgagggggagagctactttgacatgggcgcggacctgcgctggcagcccagccgccgggccttggaagctgccggcggcgtgccctacgtggaggaggtggacgatgaggaggaggagggcgagtacctggaagactgatggcgcgaccgtatttttgctagatgcagcaacagccaccgccgccgcctcctgatcccgcgatgcgggcggcgctgcagagccagccgtccggcattaactcctcggacgattggacccaggccatgcaacgcatcatggcgctgacgacccgcaatcccgaagcctttagacagcagcctcaggccaaccggctctcggccatcctggaggccgtggtgccctcgcgctcgaaccccacgcacgagaaggtgctggccatcgtgaacgcgctggtggagaacaaggccatccgcggcgacgaggccgggctggtgtacaacgcgctgctggagcgcgtggcccgctacaacagcaccaacgtgcagacgaacctggaccgcatggtgaccgacgtgcgcgaggcggtgtcgcagcgcgagcggttccaccgcgagtcgaacctgggctccatggtggcgctgaacgccttcctgagcacgcagcccgccaacgtgccccggggccaggaggactacaccaacttcatcagcgcgctgcggctgatggtggccgaggtgccccagagcgaggtgtaccagtcggggccggactacttcttccagaccagtcgccagggcttgcagaccgtgaacctgagccaggctttcaagaacttgcagggactgtggggcgtgcaggccccggtcggggaccgcgcgacggtgtcgagcctgctgacgccgaactcgcgcctgctgctgctgctggtggcgcccttcacggacagcggcagcgtgagccgcgactcgtacctgggctacctgcttaacctgtaccgcgaggccatcgggcaggcgcacgtggacgagcagacctaccaggagatcacccacgtgagccgcgcgctgggccaggaggacccgggcaacctggaggccaccctgaacttcctgctgaccaaccggtcgcagaagatcccgccccagtacgcgctgagcaccgaggaggagcgcatcctgcgctacgtgcagcagagcgtggggctgttcttgatgcaggagggggccacgcccagcgccgcgctcgacatgaccgcgcgcaacatggagcccagcatgtacgcccgcaaccgcccgttcatcaataagctgatggactacttgcatcgggcggccgccatgaactcggactactttaccaacgccatcttgaacccgcactggctcccgccgcccgggttctacacgggcgagtacgacatgcccgaccccaacgacgggttcctgtgggacgacgtggacagcagcgtgttctcgccgcggcccaccaccaccaccgtgtggaagaaagagggcggggaccggcggccgtcctcggcgctgtccggtcgcgcgggtgctgccgcggcggtgcccgaggctgccagccccttcccgagcctgcccttttcgctgaacagcgtgcgcagcagcgagctgggtcggctgacgcggccgcgcctgctgggcgaggaggagtacctgaacgactccttgttgaagcccgagcgcgagaagaacttccccaataacgggatagagagcctggtggacaagatgagccgctggaagacgtacgcgcacgagcacagggacgagccccgagctagcagcgcaggcacccgtagacgccagcggcacgacaggcagcggggactggtgtgggacgatgaggattccgccgacgacagcagcgtgttggacttgggtgggagtggtggtggtaacccgttcgctcacctgcgcccccgtatcgggcgcctgatgtaagaatctgaaaaaataaaagacggtactcaccaaggccatggcgaccagcgtgcgttcttctctgttgtttgtagtagtatgatgaggcgcgtgtacccggagggtcctcctccctcgtacgagagcgtgatgcagcaggcggtggcggcggcgatgcagcccccgctggaggcgccttacgtgcccccgcggtacctggcgcctacggaggggcggaacagcattcgttactcggagctggcacccttgtacgataccacccggttgtacctggtggacaacaagtcggcggacatcgcctcgctgaactaccagaacgaccacagcaacttcctgaccaccgtggtgcagaacaacgatttcacccccacggaggccagcacccagaccatcaactttgacgagcgctcgcggtggggcggccagctgaaaaccatcatgcacaccaacatgcccaacgtgaacgagttcatgtacagcaacaagttcaaggcgcgggtgatggtctcgcgcaagacccccaacggggtcacggtaggggatgattatgatggtagtcaggacgagctgacctacgagtgggtggagtttgagctgcccgagggcaacttctcggtgaccatgaccatcgatctgatgaacaacgccatcatcgacaactacttggcggtggggcggcagaacggggtgctggagagcgacatcggcgtgaagttcgacacgcgcaacttccggctgggctgggaccccgtgaccgagctggtgatgccgggcgtgtacaccaacgaggccttccaccccgacatcgtcctgctgcccggctgcggcgtggacttcaccgagagccgcctcagcaacctgctgggcatccgcaagcggcagcccttccaggagggcttccagatcctgtacgaggacctggaggggggcaacatccccgcgctcttggatgtcgaagcctatgaagaaagtaaggaaaaagcagaggctgaggcaactacagccgtggctaccgccgcgactgtggcagatgccactgtcaccaggggcgatacattcgccacccaggcggaggaagcagccgccctagcggcgaccgatgatagtgaaagtaagatagtcatcaagccggtggagaaggacagcaagaacaggagctacaacgttctaccggatggaaagaacaccgcctaccgcagctggtacctggcctacaactacggcgaccccgagaagggcgtgcgctcctggacgctgctcaccacctcggacgtcacctgcggcgtggagcaagtctactggtcgctgcccgacatgatgcaagacccggtcaccttccgctccacgcgacaagttagcaactacccggtggtgggcgccgagctcctgcccgtctactccaagagcttcttcaacgagcaggccgtctactcgcagcagctgcgtgccttcacctcgctcacgcacgtcttcaaccgcttccccgagaaccagatcctcgtccgcccgcccgcgcccaccattaccaccgtcagtgaaaacgttcctgctctcacagatcacgggaccctgccgctgcgcagcagtatccggggagtccagcgcgtgaccgtcactgacgccagacgccgcacctgcccctacgtctacaaggccctgggcgtagtcgcgccgcgcgtcctctcgagccgcaccttctaaaaaatgtccattctcatctcgcccagtaataacaccggttggggcctgcgcgcgcccagcaagatgtacggaggcgctcgccaacgctccacgcaacaccccgtgcgcgtgcgcgggcacttccgcgctccctggggcgccctcaagggccgcgtgcgctcgcgcaccaccgtcgacgacgtgatcgaccaggtggtggccgacgcgcgcaactacacgcccgccgccgcgcccgcctccaccgtggacgccgtcatcgacagcgtggtggccgacgcgcgccggtacgcccgcgccaagagccggcggcggcgcatcgcccggcggcaccggagcacccccgccatgcgcgcggcgcgagccttgctgcgcagggccaggcgcacgggacgcagggccatgctcagggcggccagacgcgcggcctccggcagcagcagcgccggcaggacccgcagacgcgcggccacggcggcggcggcggccatcgccagcatgtcccgcccgcggcgcggcaacgtgtactgggtgcgcgacgccgccaccggtgtgcgcgtgcccgtgcgcacccgcccccctcgcacttgaagatgctgacttcgcgatgttgatgtgtcccagcggcgaggaggatgtccaagcgcaaatacaaggaagagatgctccaggtcatcgcgcctgagatctacggccccgcggcggcggtgaaggaggaaagaaagccccgcaaactgaagcgggtcaaaaaggacaaaaaggaggaggaagatgacggactggtggagtttgtgcgcgagttcgccccccggcggcgcgtgcagtggcgcgggcggaaagtgaaaccggtgctgcggcccggcaccacggtggtcttcacgcccggcgagcgttccggctccgcctccaagcgctcctacgacgaggtgtacggggacgaggacatcctcgagcaggcggtcgagcgtctgggcgagtttgcttacggcaagcgcagccgccccgcgcccttgaaagaggaggcggtgtccatcccgctggaccacggcaaccccacgccgagcctgaagccggtgaccctgcagcaggtgctgccgagcgcggcgccgcgccggggcttcaagcgcgagggcggcgaggatctgtacccgaccatgcagctgatggtgcccaagcgccagaagctggaggacgtgctggagcacatgaaggtggaccccgaggtgcagcccgaggtcaaggtgcggcccatcaagcaggtggccccgggcctgggcgtgcagaccgtggacatcaagatccccacggagcccatggaaacgcagaccgagcccgtgaagcccagcaccagcaccatggaggtgcagacggatccctggatgccagcggcttccaccaccaccactcgccgaagacgcaagtacggcgcggccagcctgctgatgcccaactacgcgctgcatccttccatcatccccacgccgggctaccgcggcacgcgcttctaccgcggctacaccagcagccgccgccgcaagaccaccacccgccgccgtcgtcgcagccgccgcagcagcaccgcgacttccgccttggtgcggagagtgtatcgcagcgggcgcgagcctctgaccctgccgcgcgcgcgctaccacccgagcatcgccatttaactaccgcctcctacttgcagatatggccctcacatgccgcctccgcgtccccattacgggctaccgaggaagaaagccgcgccgtagaaggctgacggggaacgggctgcgtcgccatcaccaccggcggcggcgcgccatcagcaagcggttggggggaggcttcctgcccgcgctgatccccatcatcgccgcggcgatcggggcgatccccggcatagcttccgtggcggtgcaggcctctcagcgccactgagacacaaaaaagcatggatttgtaataaaaaaatggactgacgctcctggtcctgtgatgtgtgtttttagatggaagacatcaatttttcgtccctggcaccgcgacacggcacgcggccgtttatgggcacctggagcgacatcggcaacagccaactgaacgggggcgccttcaattggagcagtctctggagcgggcttaagaatttcgggtccacgctcaaaacctatggcaacaaggcgtggaacagcagcacagggcaggcgctgagggaaaagctgaaagagcagaacttccagcagaaggtggtcgatggcctggcctcgggcatcaacggggtggtggacctggccaaccaggccgtgcagaaacagatcaacagccgcctggacgcggtcccgcccgcggggtccgtggagatgccccaggtggaggaggagctgcctcccctggacaagcgcggcgacaagcgaccgcgtcccgacgcggaggagacgctgctgacgcacacggacgagccgcccccgtacgaggaggcggtgaaactgggtctgcccaccacgcggcccgtggcgcctctggccaccggggtgctgaaacccagcagcagcagccagcccgcgaccctggacttgcctccgcctgcttcccgcccctccacagtggctaagcccctgccgccggtggccgtcgcgtcgcgcgccccccgaggccgcccccaggcgaactggcagagcactctgaacagcatcgtgggtctgggagtgcagagtgtgaagcgccgccgctgctattaaaagacactgtagcgcttaacttgcttgtctgtgtgtgtatatgtatgtccgccgaccagaaggaggaagaggcgcgtcgccgagttgcaagatggccaccccatcgatgctgccccagtgggcgtacatgcacatcgccggacaggacgcttcggagtacctgagtccgggtctggtgcagttcgcccgcgccacagacacctacttcagtctggggaacaagtttaggaaccccacggtggcgcccacgcacgatgtgaccaccgaccgcagccagcggctgacgctgcgcttcgtgcccgtggaccgcgaggacaacacctactcgtacaaagtgcgctacacgctggccgtgggcgacaaccgcgtgctggacatggccagcacctactttgacatccgcggcgtgctggatcggggccccagcttcaaaccctactccggcaccgcctacaacagcctagctcccaagggagcgcccaacacctcacagtggaaggattccgacagcaaaatgcatacttttggagttgctgccatgcccggtgttgttggtaaaaaaatagaagccgatggtctgcctattggaatagattcatcctctggaactgacaccataatttatgctgataaaactttccaaccagagccacaggttggaagtgacagttgggtcgacaccaatggtgcagaggaaaaatatggaggtagagctcttaaggacactacaaacatgaagccctgctacggttcttttgccaggcctaccaacaaagaaggtggacaggctaacataaaagattctgaaactgccagcactactcctaactatgatatagatttggcattctttgacagcaaaaatattgcagctaactacgatccagatattgtaatgtacacagaaaatgttgagttgcaaactccagatactcatattgtgtttaagccaggaacttcagatgaaagttcagaagccaatttgggccagcaggccatgcccaacagacccaactacatcgggttcagagacaactttatcgggctcatgtactacaacagcactggcaatatgggtgtactggctggtcaggcctcccagctaaatgctgtggtggacttgcaggacagaaacaccgaactgtcctaccagctcttgcttgactctctgggtgacagaaccaggtatttcagtatgtggaatcaggcggtggacagctatgaccccgatgtgcgcattattgaaaatcacggtgtggaggatgaactccccaattattgcttccctttgaatggtgtaggctttacagatacttaccagggtgttaaagttaagacagatacagccgctactggtaccaatggaacgcagtgggacaaagatgataccacagtcagcactgccaatgagatccactcaggcaatcctttcgccatggagatcaacatccaggccaacctgtggcggaacttcctctacgcgaacgtggcgctgtacctgcccgactcctacaagtacacgccggccaacatcacgctgccgaccaacaccaacacctacgattacatgaacggccgcgtggtggcgccctcgctggtggacgcctacatcaacatcggggcgcgctggtcgctggaccccatggacaacgtcaaccccttcaaccaccaccgcaacgcgggcctgcgctaccgctccatgctcctgggcaacgggcgctacgtgcccttccacatccaggtgccccaaaagtttttcgccatcaagagcctcctgctcctgcccgggtcctacacctacgagtggaacttccgcaaggacgtcaacatgatcctgcagagctccctcggcaacgacctgcgcacggacggggcctccatcgccttcaccagcatcaacctctacgccaccttcttccccatggcgcacaacaccgcctccacgctcgaggccatgctgcgcaacgacaccaacgaccagtccttcaacgactacctctcggcggccaacatgctctaccccatcccggccaacgccaccaacgtgcccatctccatcccctcgcgcaactgggccgccttccgcggatggtccttcacgcgcctcaagacccgcgagacgccctcgctcggctccgggttcgacccctacttcgtctactcgggctccatcccctacctcgacggcaccttctacctcaaccacaccttcaagaaggtctccatcaccttcgactcctccgtcagctggcccggcaacgaccgcctcctgacgcccaacgagttcgaaatcaagcgcaccgtcgacggagagggatacaacgtggcccagtgcaacatgaccaaggactggttcctggtccagatgctggcccactacaacatcggctaccagggcttctacgtgcccgagggctacaaggaccgcatgtactccttcttccgcaacttccagcccatgagccgccaggtcgtggacgaggtcaactacaaggactaccaggccgtcaccctggcctaccagcacaacaactcgggcttcgtcggctacctcgcgcccaccatgcgccagggccagccctaccccgccaactacccctacccgctcatcggcaagagcgccgtcgccagcgtcacccagaaaaagttcctctgcgaccgggtcatgtggcgcatccccttctccagcaacttcatgtccatgggcgcgctcaccgacctcggccagaacatgctctacgccaactccgcccacgcgctagacatgaatttcgaagtcgaccccatggatgagtccacccttctctatgttgtcttcgaagtcttcgacgtcgtccgagtgcaccagccccaccgcggcgtcatcgaggccgtctacctgcgcacgcccttctcggccggcaacgccaccacctaaagccccgctcttgcttcttgcaagatgacggcctgtggctccggcgagcaggagctcagggccatcctccgcgacctgggctgcgggccctgcttcctgggcaccttcgacaagcgcttcccgggattcatggccccgcacaagctggcctgcgccatcgtcaacacggccggccgcgagaccgggggcgagcactggctggccttcgcctggaacccgcgctcccacacctgctacctcttcgaccccttcgggttctcggacgagcgcctcaagcagatctaccagttcgagtacgagggcctgctgcgccgcagcgccctggccaccgaggaccgctgcatcaccctggaaaagtccacccagaccgtgcagggtccgcgctcggccgcctgcgggctcttctgctgcatgttcctgcacgccttcgtgcactggcccgaccgccccatggacaagaaccccaccatgaacttgctgacgggggtgcccaacggcatgctccagtcgccccaggtggaacccaccctgcgccgcaaccaggaggcgctctaccgcttcctcaacgcccactccgcctactttcgctcccaccgcgcgcgcatcgagaaggccaccgccttcgaccgcatgaatcaagacatgtaaactgtgtgtatgtgaatgctttattcatcataataaacagcacatgtttatgccaccttctctgaggctctgactttatttagaaatcgaaggggttctgccggctctcggcgtgccccgcgggcagggatacgttgcggaactggtacttgggcagccacttgaactcggggatcagcagcttcggcacggggaggtcggggaacgagtcgctccacagcttgcgcgtgagttgcagggcgcccagcaggtcgggcgcggagatcttgaaatcgcagttgggacccgcgttctgcgcgcgagagttgcggtacacggggttgcagcactggaacaccatcagggccgggtgcttcacgctcgccagcaccgtcgcgtcggtgatgccctccacgtccagatcctcggcgttggccatcccgaagggggtcatcttgcaggtctgccgccccatgctgggcacgcagccgggcttgtggttgcaatcgcagtgcagggggatcagcatcatctgagcctgctcggagctcatgcccgggtacatggccttcatgaaagcctccagctggcggaaggcctgctgcgccttgccgccctcggtgaagaagaccccacaggacttgctagagaactggttggtggcgcagcccgcgtcgtgcacgcagcagcgcgcgtcgttgttggccagctgcaccacgctgcgcccccagcggttctgggtgatcttggcccggtcggggttctccttcagcgcgcgctgcccgttctcgctcgccacatccatctcgatcgtgtgctccttctggatcatcacggtcccgtgcaggcaccgcagcttgccctcggcctcggtgcacccgtgcagccacagcgcgcagccggtgcactcccagttcttgtgggcgatctgggagtgcgagtgcacgaagccctgcaggaagcggcccatcatcgtggtcagggtcttgttgctggtgaaggtcagcgggatgccgcggtgctcctcgttcacatacaggtggcagatgcggcggtacacctcgccctgctcgggcatcagctggaaggcggacttcaggtcgctctccacgcggtaccgctccatcagcagcgtcatcacttccatgcccttctcccaggccgaaacgatcggcaggctcagggggttcttcaccgtcatcttagtcgccgccgccgaagtcagggggtcgttctcgtccagggtctcaaacactcgcttgccgtccttctcggtgatgcgcacggggggaaagctgaagcccacggccgccagctcctcctcggcctgcctttcgtcctcgctgtcctggctgatgtcttgcaaaggcacatgcttggtcttgcggggtttctttttgggcggcagaggcggcggcggagacgtgctgggcgagcgcgagttctcgctcaccacgactatttcttcttcttggccgtcgtccgagaccacgcggcggtaggcatgcctcttctggggcagaggcggaggcgacgggctctcgcggttcggcgggcggctggcagagccccttccgcgttcgggggtgcgctcctggcggcgctgctctgactgacttcctccgcggccggccattgtgttctcctagggagcaacaagcatggagactcagccatcgtcgccaacatcgccatctgcccccgccgccgacgagaaccagcagcagcagaatgaaagcttaaccgccccgccgcccagccccacctccgacgccgccgcggccccagacatgcaagagatggaggaatccatcgagattgacctgggctacgtgacgcccgcggagcacgaggaggagctggcagcgcgcttttcagccccggaagagaaccaccaagagcagccagagcaggaagcagagagcgagcagcagcaggctgggctcgagcatggcgactacctgagcggggcagaggacgtgctcatcaagcatctggcccgccaaagcatcatcgtcaaggacgcgctgctcgaccgcgccgaggtgcccctcagcgtggcggagctcagccgcgcctacgagcgcaacctcttctcgccgcgcgtgccccccaagcgccagcccaacggcacctgcgagcccaacccgcgcctcaacttctacccggtcttcgcggtgcccgaggccctggccacctaccacctctttttcaagaaccaaaggatccccgtctcctgccgcgccaaccgcacccgcgccgacgccctgctcaacctgggtcccggcgcccgcctacctgatatcacctccttggaagaggttcccaagatcttcgagggtctgggcagcgacgagactcgggccgcgaacgctctgcaaggaagcggagaggagcatgagcaccacagcgccctggtggagttggaaggcgacaacgcgcgcctggcggtgctcaagcgcacggtcgagctgacccacttcgcctacccggcgctcaacctgccccccaaggtcatgagcgccgtcatggaccaggtgctcatcaagcgcgcctcgcccctctcagaggaggagatgcaggaccccgagagctcggacgagggcaagcccgtggtcagcgacgagcagctggcgcgctggctgggagcgagcagcaccccccagagcctggaagagcggcgcaagctcatgatggccgtggtcctggtgaccgtggagctggagtgtctgcgccgcttcttcgccgacgcggagaccctgcgcaaggtcgaggagaacctgcactacctcttcaggcacgggttcgtgcgccaggcctgcaagatctccaacgtggagctgaccaacctggtctcctacatgggcatcctgcacgagaaccgcctggggcagaacgtgctgcacaccaccctgcgcggggaggcccgccgcgactacatccgcgactgcgtctacctgtacctctgccacacctggcagacgggcatgggcgtgtggcagcagtgcctggaggagcagaacctgaaagagctctgcaagctcctgcagaagaacctcaaggccctgtggaccgggttcgacgagcgcaccaccgcctcggacctggccgacctcatcttccccgagcgcctgcggctgacgctgcgcaacgggctgcccgactttatgagccaaagcatgttgcaaaactttcgctctttcatcctcgaacgctccgggatcctgcccgccacctgctccgcactgccctcggacttcgtgccgctgaccttccgcgagtgccccccgccgctctggagccactgctacttgctgcgcctggccaactacctggcctaccactcggacgtgatcgaggacgtcagcagcgagggtctgctcgagtgccactgccgctgcaacctctgcacgccgcaccgctccttggcctgcaacccccagctgctgagcgagacccagatcatcggcaccttcgagttgcaaggccccggcgagggcaaggggggtctcaaactcaccccggggctgtggacctcggcctacttgcgcaagttcgtgcccgaggactaccatcccttcgagatcaggttctacgaggaccaatcccagccgcccaaggccgagctgtcggcctgcgtcatcacccagggggccatcctggcccaattgcaagccatccagaaatcccgccaagaatttctgctgaaaaagggccacggggtctacttggacccccagaccggagaggagctcaaccccagcttcccccaggatgccccgaggaagcagcaagaagctgaaagtggagctgccgctgccgccggaggatttggaggaagactgggagagcagtcaggcagaggagatggaagactgggacagcactcaggcagaggaggacagcctgcaagacagtctggaggaggaagacgaggtggaggaggaggcagaggaagaagcagccgccgccagaccgtcgtcctcggcggaggagaaagcaagcagcacggataccatctccgctccgggtcggggtcgcggcggccgggcccacagtagatgggacgagaccgggcgcttcccgaaccccaccacccagaccggtaagaaggagcggcagggatacaagtcctggcgggggcacaaaaacgccatcgtctcctgcttgcaagcctgcgggggcaacatctccttcacccggcgctacctgctcttccaccgcggggtgaacttcccccgcaacatcttgcattactaccgtcacctccacagcccctactactgtttccaagaagaggcagaaacccagcagcagcagcagaaaaccagcggcagcagcagcagctagaaaatccacagcggcggcaggtggactgaggatcgcggcgaacgagccggcgcagacccgggagctgaggaaccggatctttcccaccctctatgccatcttccagcagagtcgggggcaggagcaggaactgaaagtcaagaaccgttctctgcgctcgctcacccgcagttgtctgtatcacaagagcgaagaccaacttcagcgcactctcgaggacgccgaggctctcttcaacaagtactgcgcgctcactcttaaagagtagcccgcgcccgcccacacacggaaaaaggcgggaattacgtcaccacctgcgcccttcgcccgaccatcatcatgagcaaagagattcccacgccttacatgtggagctaccagccccagatgggcctggccgccggcgccgcccaggactactccacccgcatgaactggctcagtgccgggcccgcgatgatctcacgggtgaatgacatccgcgcccaccgaaaccagatactcctagaacagtcagcgatcaccgccacgccccgccatcaccttaatccgcgtaattggcccgccgccctggtgtaccaggaaattccccagcccacgaccgtactacttccgcgagacgcccaggccgaagtccagctgactaactcaggtgtccagctggccggcggcgccgccctgtgtcgtcaccgccccgctcagggtataaagcggctggtgatccgaggcagaggcacacagctcaacgacgaggtggtgagctcttcgctgggtctgcgacctgacggagtcttccaactcgccggatcggggagatcttccttcacgcctcgtcaggccgtcctgactttggagagttcgtcctcgcagccccgctcgggcggcatcggcactctccagttcgtggaggagttcactccctcggtctacttcaaccccttctccggctcccccggccactacccggacgagttcatcccgaacttcgacgccatcagcgagtcggtggacggctacgattgaatgtcccatggtggcgcggctgacctagctcggcttcgacacctggaccactgccgccgcttccgctgcttcgctcgggatctcgccgagtttgcctactttgagctgcccgaggagcaccctcagggcccggcccacggagtgcggatcgtcgtcgaagggggcctcgactcccacctgcttcggattttcagccagcgtccgatcctggtcgagcgcgagcaaggacagacccttctgaccctgtactgcatctgcaaccaccccggcctgcatgaaagtctttgttgtctgctgtgtactgagtataataaaagctgagatcagcgactactccggactcgattgtggtgttcctgctatcaaccggtccctgttcttcaccgggaacgagaccgagctccagctccagtgtaagccccacaagaagtatctcacctggctgttccagggctctccgatcgccgttgtcaaccactgcgacaacgacggagtcctgctgagcggccctgccaaccttactttttccacccgcagaagcaagctccagctcttccaacccttcctccccgggacctatcagtgcgtctcgggaccctgccatcacaccttccacctgatcccgaataccacagcgccgctccccgctactaacaaccaaactacccaccaacgccaccgtcgcgacctttctgaatctaatactaccacccacaccggaggtgagctccgaggtcgaccaacctctgggatttactacggcccctgggaggtggtagggttaatagcgctaggcctagttgcgggtgggcttttggctctctgctacctatacctcccttgctgttcgtacttagtggtgctgtgttgctggtttaagaaatggggaagatcaccctagtgagctgcggtgtgctggtggcggtggtgctttcgattgtgggactgggcggcgcggctgtagtgaaggaggagaaggccgatccctgcttgcatttcaatcccgacaaatgccagctgagttttcagcccgatggcaatcggtgcacggtgctgatcaagtgcggatgggaatgcgagaacgtgagaatcgagtacaataacaagactcggaacaatactctcgcgtccgtgtggcagcccggggaccccgagtggtacaccgtctctgtccccggtgctgacggctccccgcgcaccgtgaacaatactttcatttttgcgcacatgtgcgacacggtcatgtggatgagcaagcagtacgatatgtggccccccacgaaggagaacatcgtggtcttctccatcgcttacagcctgtgcacggcgctaatcaccgctatcgtgtgcctgagcattcacatgctcatcgctattcgccccagaaataatgccgaaaaagagaaacagccataacacgttttttcacacacctttttcagaccatggcctctgttactgccctaactatttttttgggccttgtgggtactagcagcacttttcagcatataaacaaaactgtttatgctggttctaattctgtattacctgggcatcaatcacaccagaaagtttcatggtactggtatgataaaagtaacacgccagtcacactctgcaagggtcatcaaacacccataaaccgtagtggaattttttttaaatgtaatcataataatattacactactttcaattacaaagcactattctggtacttactatggaaccaattttaacataaaacaggacacttactatagtgtcacagtattggatccaactactcctagaacaactacaaaacccacaactactaagaggcacactaaacctaaaactaccaagaaaaccactgtcaaaactacaacaactaggaccaccacaactacagaggctaccaccagcacaacacttgctgccactacacacacacacactgagctaaccttacagaccactaatgatttgatcgccctgttgcaaaagggggataacagcaccacttccaatgaggagatacccagatccatgattggcattattgttgctgtagtggtgtgcatgttgatcatcgccttgtgcatggtgtactatgccttctgctacagaaagcacagactgaacgacaagctggaacacttactaagtgttgaattttaattttttagaaccatgaagatcctaggcctttttagtttttctatcattacctctactctttgtgaatcagtggataaagatgttactattaccactggttctaattatacactgaaagggccaccctcaggtatgctttcgtggtattgctattttggaactgacactgatcaaactgaattatgcaattttcaaaaaggcaaaacctcaaactctaaaatctctaattatcaatgcaatggcactgatctgatactactcaatgtcacgaaagcatatggtggcagttattcttgccctggacaaaacactgaggatatgattttttacaaagtggaagtggttgatcccactactccaccgcccaccaccacaactactcacaccacacacacagaacaaacaccagaggcagcagaagcagagttggccttccaggttcacggagattcctttgctgtcaatacccctacacccgatcagcggtgtccggggctgctcgtcagcggcattgtcggtgtgctttcgggattagcagtcataatcatctgcatgttcatttttgcttgctgctatagaaggctttaccgacaaaaatcagacccactgctgaacctctatgtttaattttttccagagccatgaaggcagttagcgctctagttttttgttctttgattggcattgtttttagtgctgggtttttgaaaaatcttaccatttatgaaggtgagaatgccactctagtgggcatcagtggtcaaaatgtcagctggctaaaataccatctagatgggtggaaagacatttgcgattggaatgtcactgtgtatacatgtaatggagttaacctcaccattactaatgccacccaagatcagaatggtaggtttaagggccagagtttcactagaaataatgggtatgaatcccataacatgtttatctatgacgtcactgtcatcagaaatgagactgccaccaccacacagatgcccactacacacagttctaccactactaccatgcaaaccacacagacaaccactttttatacatcaactcagcatatgaccaccactacagcagcaaagccaagtagtgcagcgcctcagccccaggctttggctttgatagctgcacaacctagtacaactactaggaccaatgagcagactactgattttttgtccactgtcgagagccacaccacagctacctccagtgccttctctagcaccgccaatctctcctcgctttcctctacaccaatcagtcccgctactactactcctagccccgctcctcttcccactcccctgaagcaaactgaggacagcggcatgcaatggcagatcaccctgctcattgtgatcgggttggtcattctggccgtgttgctctactacatcttctgccgccgcattcccaacgcgcaccgcaagccggtctacaagcccatcgttgacgggcaaccggagccgcttcaggtggaagggggtctaaggaatcttctcttctcttttacagtatggtgattgaactatgattcctagacaattcttgatcactattcttatctgcctcctccaagtctgtgccaccctcgctctggtggccaacgccagtccagactgtattgggcccttcgcctcctacgtgctctttgccttcgtcacctgcatctgctgctgtagcatagtctgcctgcttatcaccttcttccagttcattgactggatctttgtgcgcatcgcctacctgcgccaccacccccagtaccgcgaccagcgagtggcgcggctgctcaggctcctctgataagcatgcgggctctgctacttctcgcgcttctgctgttagtgctcccccgtcccgtcaacccccggtcccccactcagtcccccgaggaggtccgcaaatgcaaattccaagaaccctggaaattcctcaaatgctaccgccaaaaatcagacatgcatcccagctggatcatgatcattgggatcgtgaacattctggcctgcaccctcatctcctttgtgatttacccctgctttgactttggttggaactcgccagaggcgctctatctcccgcctgaacctgacacaccaccacagcaacctcaggcacacgcactaccaccaccacagcctaggccacaatacatgcccatattagactatgaggccgagccacagcgacccatgctccccgctattagttacttcaatctaaccggcggagatgactgacccactggccaacaacaacgtcaacgaccttctcctggacatggacggccgcgcctcggagcagcgactcgcccaacttcgcattcgccagcagcaggagagagccgtcaaggagctgcaggacggcatagccatccaccagtgcaagaaaggcatcttctgcctggtgaaacaggccaagatctcctacgaggtcacccagaccgaccatcgcctctcctacgagctcctgcagcagcgccagaagttcacctgcctggtcggagtcaaccccatcgtcatcacccagcagtcgggcgataccaaggggtgcatccactgctcctgcgactcccccgactgcgtccacactctgatcaagaccctctgcggcctccgcgacctcctccccatgaactaatcacccccttatccagtgaaataaagatcatattgatgatgattttacagaaataaagatacaatcatattgatgatttgagtttaataaaaaataaagaatcacttacttgaaatctgataccaggtctctgtccatgttttctgccaacaccacttcactcccctcttcccagctctggtactgcaggccccggcgggctgcaaacttcctccacacgctgaaggggatgtcaaattcctcctgtccctcaatcttcattttatcttctatcagatgtccaaaaagcgcgtccgggtggatgatgacttcgaccccgtctacccctacgatgcagacaacgcaccgaccgtgcccttcatcaacccccccttcgtctcttcagatggattccaagagaagcccctgggggtgctgtccctgcgactggccgaccccgtcaccaccaagaacggggaaatcaccctcaagctgggagagggggtggacctcgactcctcgggaaaactcatctccaacacggccaccaaggccgccgcccctctcagtttttccaacaacaccatttcccttaacatggatcaccccttttacactaaagatggaaaattatccttacaagtttctccaccattaaatatactgagaacaagcattctaaacacactagctttaggttttggatcaggtttaggactccgtggctctgccttggcagtacagttagtctctccacttacatttgatactgatggaaacataaagcttaccttagacagaggtttgcatgttacaacaggagatgcaattgaaagcaacataagctgggctaaaggtttaaaatttgaagatggagccatagcaaccaacattggaaatgggttagagtttggaagcagtagtacagaaacaggtgttgatgatgcttacccaatccaagttaaacttggatctggccttagctttgacagtacaggagccataatggctggtaacaaagaagacgataaactcactttgtggacaacacctgatccatcgccaaactgtcaaatactcgcagaaaatgatgcaaaactaacactttgcttgactaaatgtggtagtcaaatactggccactgtgtcagtcttagttgtaggaagtggaaacctaaaccccattactggcaccgtaagcagtgctcaggtgtttctacgttttgatgcaaacggtgttcttttaacagaacattctacactaaaaaaatactgggggtataggcagggagatagcatagatggcactccatataccaatgctgtaggattcatgcccaatttaaaagcttatccaaagtcacaaagttctactactaaaaataatatagtagggcaagtatacatgaatggagatgtttcaaaacctatgcttctcactataaccctcaatggtactgatgacagcaacagtacatattcaatgtcattttcatacacctggactaatggaagctatgttggagcaacatttggggctaactcttataccttctcatacatcgcccaagaatgaacactgtatcccaccctgcatgccaacccttcccaccccactctgtggaaaaaactctgaaacacaaaataaaataaagttcaagtgttttattgattcaacagttttacaggattcgagcagttatttttcctccaccctcccaggacatggaatacaccaccctctccccccgcacagccttgaacatctgaacgccattggtgatggacatgcttttggtctccacgttccacacagtttcagagcgagccagtctcgggtcggtcagggagatgaaaccctccgggcactcccgcatctgcacctcacagctcaacagctgaggattgtcctcggtggtcgggatcacggttatctggaagaagcagaagagcggcggtgggaatcatagtccgcgaacgggatcggccggtggtgtcgcatcaggccccgcagcagtcgctgtcgccgccgctccgtcaagctgctgctcagggggtccgggtccagggactccctcagcatgatgcccacggccctcagcatcagtcgtctggtgcggcgggcgcagcagcgcatgcggatctcgctcaggtcgctgcagtacgtgcaacacaggaccaccaggttgttcaacagtccatagttcaacacgctccagccgaaactcatcgcgggaaggatgctacccacgtggccgtcgtaccagatcctcaggtaaatcaagtggcgccccctccagaacacgctgcccatgtacatgatctccttgggcatgtggcggttcaccacctcccggtaccacatcaccctctggttgaacatgcagccccggatgatcctgcggaaccacagggccagcaccgccccgcccgccatgcagcgaagagaccccgggtcccggcaatggcaatggaggacccaccgctcgtacccgtggatcatctgggagctgaacaagtctatgttggcacagcacaggcacacgctcatgcatctcttcagcactctcagctcctcgggggtcaaaaccatatcccagggcacggggaactcttgcaggacagcgaaccccgcagaacagggcaatcctcgcacagaacttacattgtgcatggacagggtatcgcaatcaggcagcaccgggtgatcctccaccagggaagcgcgggtctcggtctcctcacagcgtggtaagggggccggccgatacgggtgatggcgggacgcggctgatcgtgctcgcgaccgtgtcatgatgcagttgctttcggacattttcgtacttgctgtagcagaacctggtccgggcgctgcacaccgatcgccggcggcggtcccggcgcttggaacgctcggtgttgaagttgtaaaacagccactctctcagaccgtgcagcagatctagggcctcaggagtgatgaaaatcccatcatgcctgatagctctgatcacatcgaccaccgtggaatgggccagacccagccagatgatgcaattttgttgggtttcggtaacggcgggggagggaagaacaggaagaaccatgattaacttttaatccaaacggtctcggagcacttcaaaatgaagatcgcggagatggcacctctcgcccccgctgtgttggtggaaaataacagccaggtcaaaggtgatacggttctcgagatgttccacggtggcttccagcaaagcctccacgcgcacatccagaaacaagacaatagcgaaagcgggagggttctctaattcctcaatcatcatgttacactcctgcaccatccccagataattttcatttttccagccttgaatgattcgaactagttcctgaggtaaatccaagccagccatgataaagagctcgcgcagagcgccctccaccggcattcttaagcacaccctcataattccaagatattctgctcctggttcacctgcagcagattgacaagcggaatatcaaactctctgccgcgatccctaagctcctccctcagcaataactgtaagtactctttcatatcctctccgaaatttttagccataggaccgccaggaataagattagggcaagccacagtacagataaaccgaagtcctccccagtgagcattgccaaatgcaagactgctataagcatgctggctagacccggtgatatcttccagataactggacagaaaatcgcccaggcaatttttaagaaaatcaacaaaagaaaaatcctccaggtgcacgtttagagcctcgggaacaacgatggagtaaatgcaagcggtgcgttccagcatggttagttagctgatctgtagaaaaaacaaaaatgaacattaaaccatgctagcctggcgaacaggtgggtaaatcgttctttccagcaccaggcaggccacggggtctccggcacgaccctcgtaaaaattgtcgctatgattgaaaaccatcacagagagacgttcccggtggccggcgtgaatgattcgacaagatgaatacacccccggaacattggcgtccgcgagtgaaaaaaagcgcccgaggaagcaataaggcactacaatgctcagtctcaagtccagcaaagcgatgccatgcggatgaagcacaaaattctcaggtgcgtacaaaatgtaattactcccctcctgcacaggcagcaaagcccccgatccctccaggtacacatacaaagcctcagcgtccatagcttaccgagcagcagcagcagcacacaacaggcgcaagagtcagagaaaggctgagctctaacctgtccacccgctctctgctcaatatatagcccagatctacactgacgtaaaggccaaagtctaaaaatacccgccaaatagtcacacacgcccagcacacgcccagaaaccggtgacacactcaaaaaaatacgcgcacttcctcaaacgcccaaactgccgtcatttccgggttcccacgctacgtcatcaaaacacgactttcaaattccgtcgaccgttaaaaacgtcacccgccccgcccctaacggtcgcccgtctctcagccaatcagcgccccgcatccccaaattcaaacacctcatttgcatattaacgcgcaccaaaagtttgaggtatattattgatgatg

SEQ ID NO: 16 - protein, 1985 aa, Artificial Sequence
  met-NS3-NS5B
MAPITAYSQQTRGLLGCIITSLTGRDKNQVEGEVQVVSTATQSFLATCVNGVCWTVYHGAGSKTLAGPKGPITQMYTNVDQDLVGWQAPPGARSLTPCTCGSSDLYLVTRHADVIPVRRRGDSRGSLLSPRPVSYLKGSSGGPLLCPSGHAVGIFRAAVCTRGVAKAVDFVPVESMETTMRSPVFTDNSSPPAVPQSFQVAHLHAPTGSGKSTKVPAAYAAQGYKVLVLNPSVAATLGFGAYMSKAHGIDPNIRTGVRTITTGAPVTYSTYGKFLADGGCSGGAYDIIICDECHSTDSTTILGIGTVLDQAETAGARLVVLATATPPGSVTVPHPNIEEVALSNTGEIPFYGKAIPIEAIRGGRHLIFCHSKKKCDELAAKLSGLGINAVAYYRGLDVSVIPTIGDVVVVATDALMTGYTGDFDSVIDCNTCVTQTVDFSLDPTFTIETTTVPQDAVSRSQRRGRTGRGRRGIYRFVTPGERPSGMFDSSVLCECYDAGCAWYELTPAETSVRLRAYLNTPGLPVCQDHLEFWESVFTGLTHIDAHFLSQTKQAGDNFPYLVAYQATVCARAQAPPPSWDQMWKCLIRLKPTLHGPTPLLYRLGAVQNEVTLTHPITKYIMACMSADLEVVTSTWVLVGGVLAALAAYCLTTGSVVIVGRIILSGRPAIVPDREFLYQEFDEMEECASHLPYIEQGMQLAEQFKQKALGLLQTATKQAEAAAPVVESKWRALETFWAKHMWNFISGIQYLAGLSTLPGNPAIASLMAFTASITSPLTTQSTLLFNILGGWVAAQLAPPSAASAFVGAGIAGAAVGSIGLGKVLVDILAGYGAGVAGALVAFKVMSGEMPSTEDLVNLLPAILSPGALVVGVVCAAILRRHVGPGEGAVQWMNRLIAFASRGNHVSPTHYVPESDAAARVTQILSSLTITQLLKRLHQWINEDCSTPCSGSWLRDVWDWICTVLTDFKTWLQSKLLPQLPGVPFFSCQRGYKGVWRGDGIMQTTCPCGAQITGHVKNGSMRIVGPKTCSNTWHGTFPINAYTTGPCTPSPAPNYSRALWRVAAEEYVEVTRVGDFHYVTGMTTDNVKCPCQVPAPEFFTEVDGVRLHRYAPACRPLLREEVTFQVGLNQYLVGSQLPCEPEPDVAVLTSMLTDPSHITAETAKRRLARGSPPSLASSSASQLSAPSLKATCTTHHVSPDADLIEANLLWRQEMGGNITRVESENKVVVLDSFDPLRAEEDEREVSVPAEILRKSKKFPAAMPIWARPDYNPPLLESWKDPDYVPPVVHGCPLPPIKAPPIPPPRRKRTVVLTESSVSSALAELATKTFGSSESSAVDSGTATALPDQASDDGDKGSDVESYSSMPPLEGEPGDPDLSDGSWSTVSEEASEDVVCCSMSYTWTGALITPCAAEESKLPINALSNSLLRHHNMVYATTSRSAGLRQKKVTFDRLQVLDDHYRDVLKEMKAKASTVKAKLLSVEEACKLTPPHSAKSKFGYGAKDVRNLSSKAVNHIHSVWKDLLEDTVTPIDTTIMAKNEVFCVQPEKGGRKPARLIVFPDLGVRVCEKMALYDVVSTLPQVVMGSSYGFQYSPGQRVEFLVNTWKSKKNPMGFSYDTRCFDSTVTENDIRVEESIYQCCDLAPEARQAIKSLTERLYIGGPLTNSKGQNCGYRRCRASGVLTTSCGNTLTCYLKASAACRAAKLQDCTMLVNAAGLVVICESAGTQEDAASLRVFTEAMTRYSAPPGDPPQPEYDLELITSCSSNVSVAHDASGKRVYYLTRDPTTPLARAAWETARHTPVNSWLGNIIMYAPTLWARMILMTHFFSILLAQEQLEKALDCQIYGACYSIEPLDLPQIIERLHGLSAFSLHSYSPGEINRVASCLRKLGVPPLRVWRHRARSVRARLLSQGGRAATCGKYLFNWAVKTKLKLTPIPAASQLDLSGWFVAGYSGGDIYHSLSRARPRWFMLCLLLLSVGVGIYLLPNR

SEQ ID NO: 17 - DNA, 34658 bp, Artificial Sequence
  ChAd63 delta E1,3,4, Ad5 E4orf6, NSmut
catcatcaataatatacctcaaacttttggtgcgcgttaatatgcaaatgaggtgtttgaatttggggatgcggggcgctgattggctgagagacgggcgaccgttaggggcggggcgggtgacgttttgatgacgtggccgtgaggcggagccggtttgcaagttctcgtgggaaaagtgacgtcaaacgaggtgtggtttgaacacggaaatactcaattttcccgcgctctctgacaggaaatgaggtgtttctgggcggatgcaagtgaaaacgggccattttcgcgcgaaaactgaatgaggaagtgaaaatctgagtaattccgcgtttatggcagggaggagtatttgccgagggccgagtagactttgaccgattacgtgggggtttcgattaccgtatttttcacctaaatttccgcgtacggtgtcaaagtccggtgtttttacgatcccattgcatacgttgtatccatatcataatatgtacatttatattggctcatgtccaacattaccgccatgttgacattgattattgactagttattaatagtaatcaattacggggtcattagttcatagcccatatatggagttccgcgttacataacttacggtaaatggcccgcctggctgaccgcccaacgacccccgcccattgacgtcaataatgacgtatgttcccatagtaacgccaatagggactttccattgacgtcaatgggtggagtatttacggtaaactgcccacttggcagtacatcaagtgtatcatatgccaagtacgccccctattgacgtcaatgacggtaaatggcccgcctggcattatgcccagtacatgaccttatgggactttcctacttggcagtacatctacgtattagtcatcgctattaccatggtgatgcggttttggcagtacatcaatgggcgtggatagcggtttgactcacggggatttccaagtctccaccccattgacgtcaatgggagtttgttttggcaccaaaatcaacgggactttccaaaatgtcgtaacaactccgccccattgacgcaaatgggcggtaggcgtgtacggtgggaggtctatataagcagagctcgtttagtgaaccgtcagatcgcctggagacgccatccacgctgttttgacctccatagaagacaccgggaccgatccagcctccgcggccgggaacggtgcattggaacgcggattccccgtgccaagagtgagatctgccaccatggcgcccatcacggcctactcccaacagacgcggggcctacttggttgcatcatcactagccttacaggccgggacaagaaccaggtcgagggagaggttcaggtggtttccaccgcaacacaatccttcctggcgacctgcgtcaacggcgtgtgttggaccgtttaccatggtgctggctcaaagaccttagccggcccaaaggggccaatcacccagatgtacactaatgtggaccaggacctcgtcggctggcaggcgccccccggggcgcgttccttgacaccatgcacctgtggcagctcagacctttacttggtcacgagacatgctgacgtcattccggtgcgccggcggggcgacagtagggggagcctgctctcccccaggcctgtctcctacttgaagggctcttcgggtggtccactgctctgcccttcggggcacgctgtgggcatcttccgggctgccgtatgcacccggggggttgcgaaggcggtggactttgtgcccgtagagtccatggaaactactatgcggtctccggtcttcacggacaactcatcccccccggccgtaccgcagtcatttcaagtggcccacctacacgctcccactggcagcggcaagagtactaaagtgccggctgcatatgcagcccaagggtacaaggtgctcgtcctcaatccgtccgttgccgctaccttagggtttggggcgtatatgtctaaggcacacggtattgaccccaacatcagaactggggtaaggaccattaccacaggcgcccccgtcacatactctacctatggcaagtttcttgccgatggtggttgctctgggggcgcttatgacatcataatatgtgatgagtgccattcaactgactcgactacaatcttgggcatcggcacagtcctggaccaagcggagacggctggagcgcggcttgtcgtgctcgccaccgctacgcctccgggatcggtcaccgtgccacacccaaacatcgaggaggtggccttgtctaatactggagagatccccttctatggcaaagccatccccattgaagccatcagggggggaaggcatctcattttctgtcattccaagaagaagtgcgacgagctcgccgcaaagctgtcaggcctcggaatcaacgctgtggcgtattaccgggggctcgatgtgtccgtcataccaactatcggagacgtcgttgtcgtggcaacagacgctctgatgacgggctatacgggcgactttgactcagtgatcgactgtaacacatgtgtcacccagacagtcgacttcagcttggatcccaccttcaccattgagacgacgaccgtgcctcaagacgcagtgtcgcgctcgcagcggcggggtaggactggcaggggtaggagaggcatctacaggtttgtgactccgggagaacggccctcgggcatgttcgattcctcggtcctgtgtgagtgctatgacgcgggctgtgcttggtacgagctcacccccgccgagacctcggttaggttgcgggcctacctgaacacaccagggttgcccgtttgccaggaccacctggagttctgggagagtgtcttcacaggcctcacccacatagatgcacacttcttgtcccagaccaagcaggcaggagacaacttcccctacctggtagcataccaagccacggtgtgcgccagggctcaggccccacctccatcatgggatcaaatgtggaagtgtctcatacggctgaaacctacgctgcacgggccaacacccttgctgtacaggctgggagccgtccaaaatgaggtcaccctcacccaccccataaccaaatacatcatggcatgcatgtcggctgacctggaggtcgtcactagcacctgggtgctggtgggcggagtccttgcagctctggccgcgtattgcctgacaacaggcagtgtggtcattgtgggtaggattatcttgtccgggaggccggctattgttcccgacagggagtttctctaccaggagttcgatgaaatggaagagtgcgcctcgcacctcccttacatcgagcagggaatgcagctcgccgagcaattcaagcagaaagcgctcgggttactgcaaacagccaccaaacaagcggaggctgctgctcccgtggtggagtccaagtggcgagcccttgagacattctgggcgaagcacatgtggaatttcatcagcgggatacagtacttagcaggcttatccactctgcctgggaaccccgcaatagcatcattgatggcattcacagcctctatcaccagcccgctcaccacccaaagtaccctcctgtttaacatcttgggggggtgggtggctgcccaactcgccccccccagcgccgcttcggctttcgtgggcgccggcatcgccggtgcggctgttggcagcataggccttgggaaggtgcttgtggacattctggcgggttatggagcaggagtggccggcgcgctcgtggccttcaaggtcatgagcggcgagatgccctccaccgaggacctggtcaatctacttcctgccatcctctctcctggcgccctggtcgtcggggtcgtgtgtgcagcaatactgcgtcgacacgtgggtccgggagagggggctgtgcagtggatgaaccggctgatagcgttcgcctcgcggggtaatcatgtttcccccacgcactatgtgcctgagagcgacgccgcagcgcgtgttactcagatcctctccagccttaccatcactcagctgctgaaaaggctccaccagtggattaatgaagactgctccacaccgtgttccggctcgtggctaagggatgtttgggactggatatgcacggtgttgactgacttcaagacctggctccagtccaagctcctgccgcagctaccgggagtcccttttttctcgtgccaacgcgggtacaagggagtctggcggggagacggcatcatgcaaaccacctgcccatgtggagcacagatcaccggacatgtcaaaaacggttccatgaggatcgtcgggcctaagacctgcagcaacacgtggcatggaacattccccatcaacgcatacaccacgggcccctgcacaccctctccagcgccaaactattctagggcgctgtggcgggtggccgctgaggagtacgtggaggtcacgcgggtgggggatttccactacgtgacgggcatgaccactgacaacgtaaagtgcccatgccaggttccggctcctgaattcttcacggaggtggacggagtgcggttgcacaggtacgctccggcgtgcaggcctctcctacgggaggaggttacattccaggtcgggctcaaccaatacctggttgggtcacagctaccatgcgagcccgaaccggatgtagcagtgctcacttccatgctcaccgacccctcccacatcacagcagaaacggctaagcgtaggttggccagggggtctcccccctccttggccagctcttcagctagccagttgtctgcgccttccttgaaggcgacatgcactacccaccatgtctctccggacgctgacctcatcgaggccaacctcctgtggcggcaggagatgggcgggaacatcacccgcgtggagtcggagaacaaggtggtagtcctggactctttcgacccgcttcgagcggaggaggatgagagggaagtatccgttccggcggagatcctgcggaaatccaagaagttccccgcagcgatgcccatctgggcgcgcccggattacaaccctccactgttagagtcctggaaggacccggactacgtccctccggtggtgcacgggtgcccgttgccacctatcaaggcccctccaataccacctccacggagaaagaggacggttgtcctaacagagtcctccgtgtcttctgccttagcggagctcgctactaagaccttcggcagctccgaatcatcggccgtcgacagcggcacggcgaccgcccttcctgaccaggcctccgacgacggtgacaaaggatccgacgttgagtcgtactcctccatgcccccccttgagggggaaccgggggaccccgatctcagtgacgggtcttggtctaccgtgagcgaggaagctagtgaggatgtcgtctgctgctcaatgtcctacacatggacaggcgccttgatcacgccatgcgctgcggaggaaagcaagctgcccatcaacgcgttgagcaactctttgctgcgccaccataacatggtttatgccacaacatctcgcagcgcaggcctgcggcagaagaaggtcacctttgacagactgcaagtcctggacgaccactaccgggacgtgctcaaggagatgaaggcgaaggcgtccacagttaaggctaaactcctatccgtagaggaagcctgcaagctgacgcccccacattcggccaaatccaagtttggctatggggcaaaggacgtccggaacctatccagcaaggccgttaaccacatccactccgtgtggaaggacttgctggaagacactgtgacaccaattgacaccaccatcatggcaaaaaatgaggttttctgtgtccaaccagagaaaggaggccgtaagccagcccgccttatcgtattcccagatctgggagtccgtgtatgcgagaagatggccctctatgatgtggtctccacccttcctcaggtcgtgatgggctcctcatacggattccagtactctcctgggcagcgagtcgagttcctggtgaatacctggaaatcaaagaaaaaccccatgggcttttcatatgacactcgctgtttcgactcaacggtcaccgagaacgacatccgtgttgaggagtcaatttaccaatgttgtgacttggcccccgaagccagacaggccataaaatcgctcacagagcggctttatatcgggggtcctctgactaattcaaaagggcagaactgcggttatcgccggtgccgcgcgagcggcgtgctgacgactagctgcggtaacaccctcacatgttacttgaaggcctctgcagcctgtcgagctgcgaagctccaggactgcacgatgctcgtgaacgccgccggccttgtcgttatctgtgaaagcgcgggaacccaagaggacgcggcgagcctacgagtcttcacggaggctatgactaggtactctgccccccccggggacccgccccaaccagaatacgacttggagctgataacatcatgttcctccaatgtgtcggtcgcccacgatgcatcaggcaaaagggtgtactacctcacccgtgatcccaccacccccctcgcacgggctgcgtgggaaacagctagacacactccagttaactcctggctaggcaacattatcatgtatgcgcccactttgtgggcaaggatgattctgatgactcacttcttctccatccttctagcacaggagcaacttgaaaaagccctggactgccagatctacggggcctgttactccattgagccacttgacctacctcagatcattgaacgactccatggccttagcgcattttcactccatagttactctccaggtgagatcaatagggtggcttcatgcctcaggaaacttggggtaccacccttgcgagtctggagacatcgggccaggagcgtccgcgctaggctactgtcccagggggggagggccgccacttgtggcaagtacctcttcaactgggcagtgaagaccaaactcaaactcactccaatcccggctgcgtcccagctggacttgtccggctggttcgttgctggttacagcgggggagacatatatcacagcctgtctcgtgcccgaccccgctggttcatgctgtgcctactcctactttctgtaggggtaggcatctacctgctccccaaccgataaatctagagctgtgccttctagttgccagccatctgttgtttgcccctcccccgtgccttccttgaccctggaaggtgccactcccactgtcctttcctaataaaatgaggaaattgcatcgcattgtctgagtaggtgtcattctattctggggggtggggtggggcagcacagcaagggggaggattgggaagacaatagcaggcatgctggggatgcggtgggctctagatgtagcgatcgcgtgagtagtgtttgggggtgggtgggagcctgcatgatgggcagaatgactaaaatctgtgtttttctgtgtgttgcagcagcatgagcggaagcgcctcctttgagggaggggtattcagcccttatctgacggggcgtctcccctcctgggcgggagtgcgtcagaatgtgatgggatccacggtggacggccggcccgtgcagcccgcgaactcttcaaccctgacctacgcgaccctgagctcctcgtccgtggacgcagctgccgccgcagctgctgcttccgccgccagcgccgtgcgcggaatggccctgggcgccggctactacagctctctggtggccaactcgagttccaccaataatcccgccagcctgaacgaggagaagctgttgctgctgatggcccagctcgaggccctgacccagcgcctgggcgagctgacccagcaggtggctcagctgcaggcggagacgcgggccgcggttgccacggtgaaaaccaaataaaaaatgaatcaataaataaacggagacggttgttgattttaacacagagtcttgaatctttatttgatttttcgcgcgcggtaggccctggaccaccggtctcgatcattgagcacccggtggatcttttccaggacccggtagaggtgggcttggatgttgaggtacatgggcatgagcccgtcccgggggtggaggtagctccattgcagggcctcgtgctcgggggtggtgttgtaaatcacccagtcatagcaggggcgcagggcgtggtgctgcacgatgtctttgaggaggagactgatggccacgggcagccccttggtgtaggtgttgacgaacctattgagctgggagggatgcatgcggggggagatgagatgcatcttggcctggatcttgagattggcgatgttcccgcccagatcccgccgggggttcatgttgtgcaggaccaccagcacggtgtatccggtgcacttggggaatttgtcatgcaacttggaagggaaggcgtgaaagaatttggagacgcccttgtgaccgcccaggttttccatgcactcatccatgatgatggcgatgggcccgtgggcggcggcctgggcaaagacgtttcgggggtcggacacatcgtagttgtggtcctgggtgagctcgtcataggccattttaatgaatttggggcggagggtacccgactgggggacaaaggtgccctcgatcccgggggcgtagttcccctcgcagatctgcatctcccaggccttgagctcggagggggggatcatgtccacctgcggggcgatgaaaaaaacggtttccggggcgggggagatgagctgcgccgaaagcaggttccggagcagctgggacttgccgcagccggtggggccgtagatgaccccgatgaccggctgcaggtggtagttgagggagagacagctgccgtcctcgcggaggaggggggccacctcgttcatcatctcgcgcacatgcatgttctcgcgcacgagttccgccaggaggcgctcgccccccagcgagaggagctcttgcagcgaggcgaagtttttcagcggcttgagcccgtcggccatgggcattttggagagggtctgttgcaagagttccagacggtcccagagctcggtgatgtgctctagggcatctcgatccagcagacctcctcgtttcgcgggttggggcgactgcgggagtagggcaccaggcgatgggcgtccagcgaggccagggtccggtccttccagggtcgcagggtccgcgtcagcgtggtctccgtcacggtgaaggggtgcgcgccgggctgggcgcttgcgagggtgcgcttcaggctcatccggctggtcgagaaccgctcccggtcggcgccctgcgcgtcggccaggtagcaattgagcatgagttcgtagttgagcgcctcggccgcgtggcccttggcgcggagcttacctttggaagtgtgtccgcagacgggacagaggagggacttgagggcgtagagcttgggggcgaggaagacggactcgggggcgtaggcgtccgcgccgcagctggcgcagacggtctcgcactccacgagccaggtgaggtcggggcggtcggggtcaaaaacgaggtttcctccgtgctttttgatgcgtttcttacctctggtctccatgagctcgtgtccccgctgggtgacaaagaggctgtccgtgtccccgtagaccgactttatgggccggtcctcgagcggggtgccgcggtcctcgtcgtagaggaaccccgcccactccgagacgaaggcccgggtccaggccagcacgaaggaggccacgtgggaggggtagcggtcgttgtccaccagcgggtccaccttctccagggtatgcaagcacatgtccccctcgtccacatccaggaaggtgattggcttgtaagtgtaggccacgtgaccgggggtcccggccgggggggtataaaagggggcgggcccctgctcgtcctcactgtcttccggatcgctgtccaggagcgccagctgttggggtaggtattccctctcgaaggcgggcatgacctcggcactcaggttgtcagtttctagaaacgaggaggatttgatattgacggtgccgttggagacgcctttcatgagcccctcgtccatctggtcagaaaagacgatctttttgttgtcgagcttggtggcgaaggagccgtagagggcgttggagagcagcttggcgatggagcgcatggtctggttcttttccttgtcggcgcgctccttggcggcgatgttgagctgcacgtactcgcgcgccacgcacttccattcggggaagacggtggtgagctcgtcgggcacgattctgacccgccagccgcggttgtgcagggtgatgaggtccacgctggtggccacctcgccgcgcaggggctcgttggtccagcagaggcgcccgcccttgcgcgagcagaaggggggcagcgggtccagcatgagctcgtcgggggggtcggcgtccacggtgaagatgccgggcaggagctcggggtcgaagtagctgatgcaggtgcccagatcgtccagacttgcttgccagtcgcgcacggccagcgcgcgctcgtaggggctgaggggcgtgccccagggcatggggtgcgtgagcgcggaggcgtacatgccgcagatgtcgtagacgtagaggggctcctggaggacgccgatgtaggtggggtagcagcgccccccgcggatgctggcgcgcacgtagtcgtacagctcgtgcgagggcgcgaggagccccgtgccgagattggagcgctgcggcttttcggcgcggtagacgatctggcggaagatggcgtgggagttggaggagatggtgggcctctggaagatgttgaagtgggcatggggcagtccgaccgagtccctgatgaagtgggcgtaggagtcctgcagcttggcgacgagctcggcggtgacgaggacgtccagggcgcagtagtcgagggtctcttggatgatgtcgtacttgagctggcccttctgcttccacagctcgcggttgagaaggaactcttcgcggtccttccagtactcttcgagggggaacccgtcctgatcggcacggtaagagcccaccatgtagaactggttgacggccttgtaggcgcagcagcccttctccacggggagggcgtaagcttgcgcggccttgcgcagggaggtgtgggtgagggcgaaggtgtcgcgcaccatgactttgaggaactggtgcttgaagtcgaggtcgtcgcagccgccctgctcccagagctggaagtccgtgcgcttcttgtaggcggggttgggcaaagcgaaagtaacatcgttgaagaggatcttgcccgcgcggggcatgaagttgcgagtgatgcggaaaggctggggcacctcggcccggttgttgatgacctgggcggcgaggacgatctcgtcgaagccgttgatgttgtgcccgacgatgtagagttccacgaatcgcgggcggcccttgacgtggggcagcttcttgagctcgtcgtaggtgagctcggcggggtcgctgagcccgtgctgctcgagggcccagtcggcgacgtgggggttggcgctgaggaaggaagtccagagatccacggccagggcggtctgcaagcggtcccggtactgacggaactgctggcccacggccattttttcgggggtgacgcagtagaaggtgcgggggtcgccgtgccagcggtcccacttgagctggagggcgaggtcgtgggcgagctcgacgagcggcgggtccccggagagtttcatgaccagcatgaaggggacgagctgcttgccgaaggaccccatccaggtgtaggtttccacatcgtaggtgaggaagagcctttcggtgcgaggatgcgagccgatggggaagaactggatctcctgccaccagttggaggaatggctgttgatgtgatggaagtagaaatgccgacggcgcgccgagcactcgtgcttgtgtttatacaagcgtccgcagtgctcgcaacgctgcacgggatgcacgtgctgcacgagctgtacctgggttcctttgacgaggaatttcagtgggcagtggagcgctggcggctgcatctggtgctgtactacgtcctggccatcggcgtggccatcgtctgcctcgatggtggtcatgctgacgagcccgcgcgggaggcaggtccagacctcggctcggacgggtcggagagcgaggacgagggcgcgcaggccggagctgtccagggtcctgagacgctgcggagtcaggtcagtgggcagcggcggcgcgcggttgacttgcaggagcttttccagggcgcgcgggaggtccagatggtacttgatctccacggcgccgttggtggcgacgtccacggcttgcagggtcccgtgcccctggggcgccaccaccgtgccccgtttcttcttgggcggcggcggctccatgcttagaagcggcggcgaggacgcgcgccgggcggcaggggcggctcggggcccggaggcaggggcggcaggggcacgtcggcgccgcgcgcgggcaggttctggtactgcgcccggagaagactggcgtgagcgacgacgcgacggttgacgtcctggatctgacgcctctgggtgaaggccacgggacccgtgagtttgaacctgaaagagagttcgacagaatcaatctcggtatcgttgacggcggcctgccgcaggatctcttgcacgtcgcccgagttgtcctggtaggcgatctcggtcatgaactgctcgatctcctcctcctgaaggtctccgcggccggcgcgctcgacggtggccgcgaggtcgttggagatgcggcccatgagctgcgagaaggcgttcatgccggcctcgttccagacgcggctgtagaccacggctccgtcggggtcgcgcgcgcgcatgaccacctgggcgaggttgagctcgacgtggcgcgtgaagaccgcgtagttgcagaggcgctggtagaggtagttgagcgtggtggcgatgtgctcggtgacgaagaagtacatgatccagcggcggagcggcatctcgctgacgtcgcccagggcttccaagcgctccatggcctcgtagaagtccacggcgaagttgaaaaactgggagttgcgcgccgagacggtcaactcctcctccagaagacggatgagctcggcgatggtggcgcgcacctcgcgctcgaaggccccggggggctcctcttccatttcctcctcttcctcctccactaacatctcttctacttcctcctcaggaggcggcggcgggggaggggccctgcgtcgccggcggcgcacgggcagacggtcgatgaagcgctcgatggtctccccgcgccggcgacgcatggtctcggtgacggcgcgcccgtcctcgcggggccgcagcgtgaagacgccgccgcgcatctccaggtggccgccgggggggtctccgttgggcagggagagggcgctgacgatgcatcttatcaattgacccgtagggactccgcgcaaggacctgagcgtctcgagatccacgggatccgaaaaccgctgaacgaaggcttcgagccagtcgcagtcgcaaggtaggctgagcccggtttcttgttcttcgggtatttggtcgggaggcgggcgggcgatgctgctggtgatgaagttgaagtaggcggtcctgagacggcggatggtggcgaggagcaccaggtccttgggcccggcttgctggatgcgcagacggtcggccatgccccaggcgtggtcctgacacctggcgaggtccttgtagtagtcctgcatgagccgctccacgggcacctcctcctcgcccgcgcggccgtgcatgcgcgtgagcccgaacccgcgctgcggctggacgagcgccaggtcggcgacgacgcgctcggcgaggatggcctgctggatctgggtgagggtggtctggaagtcgtcgaagtcgacgaagcggtggtaggctccggtgttgatggtgtaggagcagttggccatgacggaccagttgacggtctggtggccggggcgcacgagctcgtggtacttgaggcgcgagtaggcgcgcgtgtcgaagatgtagtcgttgcaggtgcgcacgaggtactggtatccgacgaggaagtgcggcggcggctggcggtagagcggccatcgctcggtggcgggggcgccgggcgcgaggtcctcgagcatgaggcggtggtagccgtagatgtacctggacatccaggtgatgccggcggcggtggtggaggcgcgcgggaactcgcggacgcggttccagatgttgcgcagcggcaggaagtagttcatggtggccgcggtctggcccgtgaggcgcgcgcagtcgtggatgctctagacatacgggcaaaaacgaaagcggtcagcggctcgactccgtggcctggaggctaagcgaacgggttgggctgcgcgtgtaccccggttcgaatctcgaatcaggctggagccgcagctaacgtggtactggcactcccgtctcgacccaagcctgctaacgaaacctccaggatacggaggcgggtcgttttttggccttggtcgctggtcatgaaaaactagtaagcgcggaaagcggccgcccgcgatggctcgctgccgtagtctggagaaagaatcgccagggttgcgttgcggtgtgccccggttcgagcctcagcgctcggcgccggccggattccgcggctaacgtgggcgtggctgccccgtcgtttccaagaccccttagccagccgacttctccagttacggagcgagcccctctttttttcttgtgtttttgccagatgcatcccgtactgcggcagatgcgcccccaccctccaccacaaccgcccctaccgcagcagcagcaacagccggcgcttctgcccccgccccagcagcagcagccagccactaccgcggcggccgccgtgagcggagccggcgttcagtatgacctggccttggaagagggcgaggggctggcgcggctgggggcgtcgtcgccggagcggcacccgcgcgtgcagatgaaaagggacgctcgcgaggcctacgtgcccaagcagaacctgttcagagacaggagcggcgaggagcccgaggagatgcgcgcctcccgcttccacgcggggcgggagctgcggcgcggcctggaccgaaagcgggtgctgagggacgaggatttcgaggcggacgagctgacggggatcagccccgcgcgcgcgcacgtggccgcggccaacctggtcacggcgtacgagcagaccgtgaaggaggagagcaacttccaaaaatccttcaacaaccacgtgcgcacgctgatcgcgcgcgaggaggtgaccctgggcctgatgcacctgtgggacctgctggaggccatcgtgcagaaccccacgagcaagccgctgacggcgcagctgtttctggtggtgcagcacagtcgggacaacgagacgttcagggaggcgctgctgaatatcaccgagcccgagggccgctggctcctggacctggtgaacattctgcagagcatcgtggtgcaggagcgcgggctgccgctgtccgagaagctggcggccatcaacttctcggtgctgagcctgggcaagtactacgctaggaagatctacaagaccccgtacgtgcccatagacaaggaggtgaagatcgatgggttttacatgcgcatgaccctgaaagtgctgaccctgagcgacgatctgggggtgtaccgcaacgacaggatgcaccgcgcggtgagcgccagccgccggcgcgagctgagcgaccaggagctgatgcacagcctgcagcgggccctgaccggggccgggaccgagggggagagctactttgacatgggcgcggacctgcgctggcagcccagccgccgggccttggaagctgccggcggcgtgccctacgtggaggaggtggacgatgaggaggaggagggcgagtacctggaagactgatggcgcgaccgtatttttgctagatgcagcaacagccaccgccgccgcctcctgatcccgcgatgcgggcggcgctgcagagccagccgtccggcattaactcctcggacgattggacccaggccatgcaacgcatcatggcgctgacgacccgcaatcccgaagcctttagacagcagcctcaggccaaccggctctcggccatcctggaggccgtggtgccctcgcgctcgaaccccacgcacgagaaggtgctggccatcgtgaacgcgctggtggagaacaaggccatccgcggcgacgaggccgggctggtgtacaacgcgctgctggagcgcgtggcccgctacaacagcaccaacgtgcagacgaacctggaccgcatggtgaccgacgtgcgcgaggcggtgtcgcagcgcgagcggttccaccgcgagtcgaacctgggctccatggtggcgctgaacgccttcctgagcacgcagcccgccaacgtgccccggggccaggaggactacaccaacttcatcagcgcgctgcggctgatggtggccgaggtgccccagagcgaggtgtaccagtcggggccggactacttcttccagaccagtcgccagggcttgcagaccgtgaacctgagccaggctttcaagaacttgcagggactgtggggcgtgcaggccccggtcggggaccgcgcgacggtgtcgagcctgctgacgccgaactcgcgcctgctgctgctgctggtggcgcccttcacggacagcggcagcgtgagccgcgactcgtacctgggctacctgcttaacctgtaccgcgaggccatcgggcaggcgcacgtggacgagcagacctaccaggagatcacccacgtgagccgcgcgctgggccaggaggacccgggcaacctggaggccaccctgaacttcctgctgaccaaccggtcgcagaagatcccgccccagtacgcgctgagcaccgaggaggagcgcatcctgcgctacgtgcagcagagcgtggggctgttcttgatgcaggagggggccacgcccagcgccgcgctcgacatgaccgcgcgcaacatggagcccagcatgtacgcccgcaaccgcccgttcatcaataagctgatggactacttgcatcgggcggccgccatgaactcggactactttaccaacgccatcttgaacccgcactggctcccgccgcccgggttctacacgggcgagtacgacatgcccgaccccaacgacgggttcctgtgggacgacgtggacagcagcgtgttctcgccgcggcccaccaccaccaccgtgtggaagaaagagggcggggaccggcggccgtcctcggcgctgtccggtcgcgcgggtgctgccgcggcggtgcccgaggctgccagccccttcccgagcctgcccttttcgctgaacagcgtgcgcagcagcgagctgggtcggctgacgcggccgcgcctgctgggcgaggaggagtacctgaacgactccttgttgaagcccgagcgcgagaagaacttccccaataacgggatagagagcctggtggacaagatgagccgctggaagacgtacgcgcacgagcacagggacgagccccgagctagcagcgcaggcacccgtagacgccagcggcacgacaggcagcggggactggtgtgggacgatgaggattccgccgacgacagcagcgtgttggacttgggtgggagtggtggtggtaacccgttcgctcacctgcgcccccgtatcgggcgcctgatgtaagaatctgaaaaaataaaagacggtactcaccaaggccatggcgaccagcgtgcgttcttctctgttgtttgtagtagtatgatgaggcgcgtgtacccggagggtcctcctccctcgtacgagagcgtgatgcagcaggcggtggcggcggcgatgcagcccccgctggaggcgccttacgtgcccccgcggtacctggcgcctacggaggggcggaacagcattcgttactcggagctggcacccttgtacgataccacccggttgtacctggtggacaacaagtcggcggacatcgcctcgctgaactaccagaacgaccacagcaacttcctgaccaccgtggtgcagaacaacgatttcacccccacggaggccagcacccagaccatcaactttgacgagcgctcgcggtggggcggccagctgaaaaccatcatgcacaccaacatgcccaacgtgaacgagttcatgtacagcaacaagttcaaggcgcgggtgatggtctcgcgcaagacccccaacggggtcacggtaggggatgattatgatggtagtcaggacgagctgacctacgagtgggtggagtttgagctgcccgagggcaacttctcggtgaccatgaccatcgatctgatgaacaacgccatcatcgacaactacttggcggtggggcggcagaacggggtgctggagagcgacatcggcgtgaagttcgacacgcgcaacttccggctgggctgggaccccgtgaccgagctggtgatgccgggcgtgtacaccaacgaggccttccaccccgacatcgtcctgctgcccggctgcggcgtggacttcaccgagagccgcctcagcaacctgctgggcatccgcaagcggcagcccttccaggagggcttccagatcctgtacgaggacctggaggggggcaacatccccgcgctcttggatgtcgaagcctatgaagaaagtaaggaaaaagcagaggctgaggcaactacagccgtggctaccgccgcgactgtggcagatgccactgtcaccaggggcgatacattcgccacccaggcggaggaagcagccgccctagcggcgaccgatgatagtgaaagtaagatagtcatcaagccggtggagaaggacagcaagaacaggagctacaacgttctaccggatggaaagaacaccgcctaccgcagctggtacctggcctacaactacggcgaccccgagaagggcgtgcgctcctggacgctgctcaccacctcggacgtcacctgcggcgtggagcaagtctactggtcgctgcccgacatgatgcaagacccggtcaccttccgctccacgcgacaagttagcaactacccggtggtgggcgccgagctcctgcccgtctactccaagagcttcttcaacgagcaggccgtctactcgcagcagctgcgtgccttcacctcgctcacgcacgtcttcaaccgcttccccgagaaccagatcctcgtccgcccgcccgcgcccaccattaccaccgtcagtgaaaacgttcctgctctcacagatcacgggaccctgccgctgcgcagcagtatccggggagtccagcgcgtgaccgtcactgacgccagacgccgcacctgcccctacgtctacaaggccctgggcgtagtcgcgccgcgcgtcctctcgagccgcaccttctaaaaaatgtccattctcatctcgcccagtaataacaccggttggggcctgcgcgcgcccagcaagatgtacggaggcgctcgccaacgctccacgcaacaccccgtgcgcgtgcgcgggcacttccgcgctccctggggcgccctcaagggccgcgtgcgctcgcgcaccaccgtcgacgacgtgatcgaccaggtggtggccgacgcgcgcaactacacgcccgccgccgcgcccgcctccaccgtggacgccgtcatcgacagcgtggtggccgacgcgcgccggtacgcccgcgccaagagccggcggcggcgcatcgcccggcggcaccggagcacccccgccatgcgcgcggcgcgagccttgctgcgcagggccaggcgcacgggacgcagggccatgctcagggcggccagacgcgcggcctccggcagcagcagcgccggcaggacccgcagacgcgcggccacggcggcggcggcggccatcgccagcatgtcccgcccgcggcgcggcaacgtgtactgggtgcgcgacgccgccaccggtgtgcgcgtgcccgtgcgcacccgcccccctcgcacttgaagatgctgacttcgcgatgttgatgtgtcccagcggcgaggaggatgtccaagcgcaaatacaaggaagagatgctccaggtcatcgcgcctgagatctacggccccgcggcggcggtgaaggaggaaagaaagccccgcaaactgaagcgggtcaaaaaggacaaaaaggaggaggaagatgacggactggtggagtttgtgcgcgagttcgccccccggcggcgcgtgcagtggcgcgggcggaaagtgaaaccggtgctgcggcccggcaccacggtggtcttcacgcccggcgagcgttccggctccgcctccaagcgctcctacgacgaggtgtacggggacgaggacatcctcgagcaggcggtcgagcgtctgggcgagtttgcttacggcaagcgcagccgccccgcgcccttgaaagaggaggcggtgtccatcccgctggaccacggcaaccccacgccgagcctgaagccggtgaccctgcagcaggtgctgccgagcgcggcgccgcgccggggcttcaagcgcgagggcggcgaggatctgtacccgaccatgcagctgatggtgcccaagcgccagaagctggaggacgtgctggagcacatgaaggtggaccccgaggtgcagcccgaggtcaaggtgcggcccatcaagcaggtggccccgggcctgggcgtgcagaccgtggacatcaagatccccacggagcccatggaaacgcagaccgagcccgtgaagcccagcaccagcaccatggaggtgcagacggatccctggatgccagcggcttccaccaccaccactcgccgaagacgcaagtacggcgcggccagcctgctgatgcccaactacgcgctgcatccttccatcatccccacgccgggctaccgcggcacgcgcttctaccgcggctacaccagcagccgccgccgcaagaccaccacccgccgccgtcgtcgcagccgccgcagcagcaccgcgacttccgccttggtgcggagagtgtatcgcagcgggcgcgagcctctgaccctgccgcgcgcgcgctaccacccgagcatcgccatttaactaccgcctcctacttgcagatatggccctcacatgccgcctccgcgtccccattacgggctaccgaggaagaaagccgcgccgtagaaggctgacggggaacgggctgcgtcgccatcaccaccggcggcggcgcgccatcagcaagcggttggggggaggcttcctgcccgcgctgatccccatcatcgccgcggcgatcggggcgatccccggcatagcttccgtggcggtgcaggcctctcagcgccactgagacacaaaaaagcatggatttgtaataaaaaaatggactgacgctcctggtcctgtgatgtgtgtttttagatggaagacatcaatttttcgtccctggcaccgcgacacggcacgcggccgtttatgggcacctggagcgacatcggcaacagccaactgaacgggggcgccttcaattggagcagtctctggagcgggcttaagaatttcgggtccacgctcaaaacctatggcaacaaggcgtggaacagcagcacagggcaggcgctgagggaaaagctgaaagagcagaacttccagcagaaggtggtcgatggcctggcctcgggcatcaacggggtggtggacctggccaaccaggccgtgcagaaacagatcaacagccgcctggacgcggtcccgcccgcggggtccgtggagatgccccaggtggaggaggagctgcctcccctggacaagcgcggcgacaagcgaccgcgtcccgacgcggaggagacgctgctgacgcacacggacgagccgcccccgtacgaggaggcggtgaaactgggtctgcccaccacgcggcccgtggcgcctctggccaccggggtgctgaaacccagcagcagcagccagcccgcgaccctggacttgcctccgcctgcttcccgcccctccacagtggctaagcccctgccgccggtggccgtcgcgtcgcgcgccccccgaggccgcccccaggcgaactggcagagcactctgaacagcatcgtgggtctgggagtgcagagtgtgaagcgccgccgctgctattaaaagacactgtagcgcttaacttgcttgtctgtgtgtgtatatgtatgtccgccgaccagaaggaggaagaggcgcgtcgccgagttgcaagatggccaccccatcgatgctgccccagtgggcgtacatgcacatcgccggacaggacgcttcggagtacctgagtccgggtctggtgcagttcgcccgcgccacagacacctacttcagtctggggaacaagtttaggaaccccacggtggcgcccacgcacgatgtgaccaccgaccgcagccagcggctgacgctgcgcttcgtgcccgtggaccgcgaggacaacacctactcgtacaaagtgcgctacacgctggccgtgggcgacaaccgcgtgctggacatggccagcacctactttgacatccgcggcgtgctggatcggggccccagcttcaaaccctactccggcaccgcctacaacagcctagctcccaagggagcgcccaacacctcacagtggaaggattccgacagcaaaatgcatacttttggagttgctgccatgcccggtgttgttggtaaaaaaatagaagccgatggtctgcctattggaatagattcatcctctggaactgacaccataatttatgctgataaaactttccaaccagagccacaggttggaagtgacagttgggtcgacaccaatggtgcagaggaaaaatatggaggtagagctcttaaggacactacaaacatgaagccctgctacggttcttttgccaggcctaccaacaaagaaggtggacaggctaacataaaagattctgaaactgccagcactactcctaactatgatatagatttggcattctttgacagcaaaaatattgcagctaactacgatccagatattgtaatgtacacagaaaatgttgagttgcaaactccagatactcatattgtgtttaagccaggaacttcagatgaaagttcagaagccaatttgggccagcaggccatgcccaacagacccaactacatcgggttcagagacaactttatcgggctcatgtactacaacagcactggcaatatgggtgtactggctggtcaggcctcccagctaaatgctgtggtggacttgcaggacagaaacaccgaactgtcctaccagctcttgcttgactctctgggtgacagaaccaggtatttcagtatgtggaatcaggcggtggacagctatgaccccgatgtgcgcattattgaaaatcacggtgtggaggatgaactccccaattattgcttccctttgaatggtgtaggctttacagatacttaccagggtgttaaagttaagacagatacagccgctactggtaccaatggaacgcagtgggacaaagatgataccacagtcagcactgccaatgagatccactcaggcaatcctttcgccatggagatcaacatccaggccaacctgtggcggaacttcctctacgcgaacgtggcgctgtacctgcccgactcctacaagtacacgccggccaacatcacgctgccgaccaacaccaacacctacgattacatgaacggccgcgtggtggcgccctcgctggtggacgcctacatcaacatcggggcgcgctggtcgctggaccccatggacaacgtcaaccccttcaaccaccaccgcaacgcgggcctgcgctaccgctccatgctcctgggcaacgggcgctacgtgcccttccacatccaggtgccccaaaagtttttcgccatcaagagcctcctgctcctgcccgggtcctacacctacgagtggaacttccgcaaggacgtcaacatgatcctgcagagctccctcggcaacgacctgcgcacggacggggcctccatcgccttcaccagcatcaacctctacgccaccttcttccccatggcgcacaacaccgcctccacgctcgaggccatgctgcgcaacgacaccaacgaccagtccttcaacgactacctctcggcggccaacatgctctaccccatcccggccaacgccaccaacgtgcccatctccatcccctcgcgcaactgggccgccttccgcggatggtccttcacgcgcctcaagacccgcgagacgccctcgctcggctccgggttcgacccctacttcgtctactcgggctccatcccctacctcgacggcaccttctacctcaaccacaccttcaagaaggtctccatcaccttcgactcctccgtcagctggcccggcaacgaccgcctcctgacgcccaacgagttcgaaatcaagcgcaccgtcgacggagagggatacaacgtggcccagtgcaacatgaccaaggactggttcctggtccagatgctggcccactacaacatcggctaccagggcttctacgtgcccgagggctacaaggaccgcatgtactccttcttccgcaacttccagcccatgagccgccaggtcgtggacgaggtcaactacaaggactaccaggccgtcaccctggcctaccagcacaacaactcgggcttcgtcggctacctcgcgcccaccatgcgccagggccagccctaccccgccaactacccctacccgctcatcggcaagagcgccgtcgccagcgtcacccagaaaaagttcctctgcgaccgggtcatgtggcgcatccccttctccagcaacttcatgtccatgggcgcgctcaccgacctcggccagaacatgctctacgccaactccgcccacgcgctagacatgaatttcgaagtcgaccccatggatgagtccacccttctctatgttgtcttcgaagtcttcgacgtcgtccgagtgcaccagccccaccgcggcgtcatcgaggccgtctacctgcgcacgcccttctcggccggcaacgccaccacctaaagccccgctcttgcttcttgcaagatgacggcctgtggctccggcgagcaggagctcagggccatcctccgcgacctgggctgcgggccctgcttcctgggcaccttcgacaagcgcttcccgggattcatggccccgcacaagctggcctgcgccatcgtcaacacggccggccgcgagaccgggggcgagcactggctggccttcgcctggaacccgcgctcccacacctgctacctcttcgaccccttcgggttctcggacgagcgcctcaagcagatctaccagttcgagtacgagggcctgctgcgccgcagcgccctggccaccgaggaccgctgcatcaccctggaaaagtccacccagaccgtgcagggtccgcgctcggccgcctgcgggctcttctgctgcatgttcctgcacgccttcgtgcactggcccgaccgccccatggacaagaaccccaccatgaacttgctgacgggggtgcccaacggcatgctccagtcgccccaggtggaacccaccctgcgccgcaaccaggaggcgctctaccgcttcctcaacgcccactccgcctactttcgctcccaccgcgcgcgcatcgagaaggccaccgccttcgaccgcatgaatcaagacatgtaaactgtgtgtatgtgaatgctttattcatcataataaacagcacatgtttatgccaccttctctgaggctctgactttatttagaaatcgaaggggttctgccggctctcggcgtgccccgcgggcagggatacgttgcggaactggtacttgggcagccacttgaactcggggatcagcagcttcggcacggggaggtcggggaacgagtcgctccacagcttgcgcgtgagttgcagggcgcccagcaggtcgggcgcggagatcttgaaatcgcagttgggacccgcgttctgcgcgcgagagttgcggtacacggggttgcagcactggaacaccatcagggccgggtgcttcacgctcgccagcaccgtcgcgtcggtgatgccctccacgtccagatcctcggcgttggccatcccgaagggggtcatcttgcaggtctgccgccccatgctgggcacgcagccgggcttgtggttgcaatcgcagtgcagggggatcagcatcatctgagcctgctcggagctcatgcccgggtacatggccttcatgaaagcctccagctggcggaaggcctgctgcgccttgccgccctcggtgaagaagaccccacaggacttgctagagaactggttggtggcgcagcccgcgtcgtgcacgcagcagcgcgcgtcgttgttggccagctgcaccacgctgcgcccccagcggttctgggtgatcttggcccggtcggggttctccttcagcgcgcgctgcccgttctcgctcgccacatccatctcgatcgtgtgctccttctggatcatcacggtcccgtgcaggcaccgcagcttgccctcggcctcggtgcacccgtgcagccacagcgcgcagccggtgcactcccagttcttgtgggcgatctgggagtgcgagtgcacgaagccctgcaggaagcggcccatcatcgtggtcagggtcttgttgctggtgaaggtcagcgggatgccgcggtgctcctcgttcacatacaggtggcagatgcggcggtacacctcgccctgctcgggcatcagctggaaggcggacttcaggtcgctctccacgcggtaccgctccatcagcagcgtcatcacttccatgcccttctcccaggccgaaacgatcggcaggctcagggggttcttcaccgtcatcttagtcgccgccgccgaagtcagggggtcgttctcgtccagggtctcaaacactcgcttgccgtccttctcggtgatgcgcacggggggaaagctgaagcccacggccgccagctcctcctcggcctgcctttcgtcctcgctgtcctggctgatgtcttgcaaaggcacatgcttggtcttgcggggtttctttttgggcggcagaggcggcggcggagacgtgctgggcgagcgcgagttctcgctcaccacgactatttcttcttcttggccgtcgtccgagaccacgcggcggtaggcatgcctcttctggggcagaggcggaggcgacgggctctcgcggttcggcgggcggctggcagagccccttccgcgttcgggggtgcgctcctggcggcgctgctctgactgacttcctccgcggccggccattgtgttctcctagggagcaacaagcatggagactcagccatcgtcgccaacatcgccatctgcccccgccgccgacgagaaccagcagcagcagaatgaaagcttaaccgccccgccgcccagccccacctccgacgccgccgcggccccagacatgcaagagatggaggaatccatcgagattgacctgggctacgtgacgcccgcggagcacgaggaggagctggcagcgcgcttttcagccccggaagagaaccaccaagagcagccagagcaggaagcagagagcgagcagcagcaggctgggctcgagcatggcgactacctgagcggggcagaggacgtgctcatcaagcatctggcccgccaaagcatcatcgtcaaggacgcgctgctcgaccgcgccgaggtgcccctcagcgtggcggagctcagccgcgcctacgagcgcaacctcttctcgccgcgcgtgccccccaagcgccagcccaacggcacctgcgagcccaacccgcgcctcaacttctacccggtcttcgcggtgcccgaggccctggccacctaccacctctttttcaagaaccaaaggatccccgtctcctgccgcgccaaccgcacccgcgccgacgccctgctcaacctgggtcccggcgcccgcctacctgatatcacctccttggaagaggttcccaagatcttcgagggtctgggcagcgacgagactcgggccgcgaacgctctgcaaggaagcggagaggagcatgagcaccacagcgccctggtggagttggaaggcgacaacgcgcgcctggcggtgctcaagcgcacggtcgagctgacccacttcgcctacccggcgctcaacctgccccccaaggtcatgagcgccgtcatggaccaggtgctcatcaagcgcgcctcgcccctctcagaggaggagatgcaggaccccgagagctcggacgagggcaagcccgtggtcagcgacgagcagctggcgcgctggctgggagcgagcagcaccccccagagcctggaagagcggcgcaagctcatgatggccgtggtcctggtgaccgtggagctggagtgtctgcgccgcttcttcgccgacgcggagaccctgcgcaaggtcgaggagaacctgcactacctcttcaggcacgggttcgtgcgccaggcctgcaagatctccaacgtggagctgaccaacctggtctcctacatgggcatcctgcacgagaaccgcctggggcagaacgtgctgcacaccaccctgcgcggggaggcccgccgcgactacatccgcgactgcgtctacctgtacctctgccacacctggcagacgggcatgggcgtgtggcagcagtgcctggaggagcagaacctgaaagagctctgcaagctcctgcagaagaacctcaaggccctgtggaccgggttcgacgagcgcaccaccgcctcggacctggccgacctcatcttccccgagcgcctgcggctgacgctgcgcaacgggctgcccgactttatgagccaaagcatgttgcaaaactttcgctctttcatcctcgaacgctccgggatcctgcccgccacctgctccgcactgccctcggacttcgtgccgctgaccttccgcgagtgccccccgccgctctggagccactgctacttgctgcgcctggccaactacctggcctaccactcggacgtgatcgaggacgtcagcagcgagggtctgctcgagtgccactgccgctgcaacctctgcacgccgcaccgctccttggcctgcaacccccagctgctgagcgagacccagatcatcggcaccttcgagttgcaaggccccggcgagggcaaggggggtctcaaactcaccccggggctgtggacctcggcctacttgcgcaagttcgtgcccgaggactaccatcccttcgagatcaggttctacgaggaccaatcccagccgcccaaggccgagctgtcggcctgcgtcatcacccagggggccatcctggcccaattgcaagccatccagaaatcccgccaagaatttctgctgaaaaagggccacggggtctacttggacccccagaccggagaggagctcaaccccagcttcccccaggatgccccgaggaagcagcaagaagctgaaagtggagctgccgctgccgccggaggatttggaggaagactgggagagcagtcaggcagaggagatggaagactgggacagcactcaggcagaggaggacagcctgcaagacagtctggaggaggaagacgaggtggaggaggaggcagaggaagaagcagccgccgccagaccgtcgtcctcggcggaggagaaagcaagcagcacggataccatctccgctccgggtcggggtcgcggcggccgggcccacagtagatgggacgagaccgggcgcttcccgaaccccaccacccagaccggtaagaaggagcggcagggatacaagtcctggcgggggcacaaaaacgccatcgtctcctgcttgcaagcctgcgggggcaacatctccttcacccggcgctacctgctcttccaccgcggggtgaacttcccccgcaacatcttgcattactaccgtcacctccacagcccctactactgtttccaagaagaggcagaaacccagcagcagcagcagaaaaccagcggcagcagcagcagctagaaaatccacagcggcggcaggtggactgaggatcgcggcgaacgagccggcgcagacccgggagctgaggaaccggatctttcccaccctctatgccatcttccagcagagtcgggggcaggagcaggaactgaaagtcaagaaccgttctctgcgctcgctcacccgcagttgtctgtatcacaagagcgaagaccaacttcagcgcactctcgaggacgccgaggctctcttcaacaagtactgcgcgctcactcttaaagagtagcccgcgcccgcccacacacggaaaaaggcgggaattacgtcaccacctgcgcccttcgcccgaccatcatcatgagcaaagagattcccacgccttacatgtggagctaccagccccagatgggcctggccgccggcgccgcccaggactactccacccgcatgaactggctcagtgccgggcccgcgatgatctcacgggtgaatgacatccgcgcccaccgaaaccagatactcctagaacagtcagcgatcaccgccacgccccgccatcaccttaatccgcgtaattggcccgccgccctggtgtaccaggaaattccccagcccacgaccgtactacttccgcgagacgcccaggccgaagtccagctgactaactcaggtgtccagctggccggcggcgccgccctgtgtcgtcaccgccccgctcagggtataaagcggctggtgatccgaggcagaggcacacagctcaacgacgaggtggtgagctcttcgctgggtctgcgacctgacggagtcttccaactcgccggatcggggagatcttccttcacgcctcgtcaggccgtcctgactttggagagttcgtcctcgcagccccgctcgggcggcatcggcactctccagttcgtggaggagttcactccctcggtctacttcaaccccttctccggctcccccggccactacccggacgagttcatcccgaacttcgacgccatcagcgagtcggtggacggctacgattgaatgtcccatggtggcgcggctgacctagctcggcttcgacacctggaccactgttaattaatcgcctctcctacgagctcctgcagcagcgccagaagttcacctgcctggtcggagtcaaccccatcgtcatcacccagcagtcgggcgataccaaggggtgcatccactgctcctgcgactcccccgactgcgtccacactctgatcaagaccctctgcggcctccgcgacctcctccccatgaactaatcacccccttatccagtgaaataaagatcatattgatgatgattttacagaaataaagatacaatcatattgatgatttgagtttaataaaaaataaagaatcacttacttgaaatctgataccaggtctctgtccatgttttctgccaacaccacttcactcccctcttcccagctctggtactgcaggccccggcgggctgcaaacttcctccacacgctgaaggggatgtcaaattcctcctgtccctcaatcttcattttatcttctatcagatgtccaaaaagcgcgtccgggtggatgatgacttcgaccccgtctacccctacgatgcagacaacgcaccgaccgtgcccttcatcaacccccccttcgtctcttcagatggattccaagagaagcccctgggggtgctgtccctgcgactggccgaccccgtcaccaccaagaacggggaaatcaccctcaagctgggagagggggtggacctcgactcctcgggaaaactcatctccaacacggccaccaaggccgccgcccctctcagtttttccaacaacaccatttcccttaacatggatcaccccttttacactaaagatggaaaattatccttacaagtttctccaccattaaatatactgagaacaagcattctaaacacactagctttaggttttggatcaggtttaggactccgtggctctgccttggcagtacagttagtctctccacttacatttgatactgatggaaacataaagcttaccttagacagaggtttgcatgttacaacaggagatgcaattgaaagcaacataagctgggctaaaggtttaaaatttgaagatggagccatagcaaccaacattggaaatgggttagagtttggaagcagtagtacagaaacaggtgttgatgatgcttacccaatccaagttaaacttggatctggccttagctttgacagtacaggagccataatggctggtaacaaagaagacgataaactcactttgtggacaacacctgatccatcgccaaactgtcaaatactcgcagaaaatgatgcaaaactaacactttgcttgactaaatgtggtagtcaaatactggccactgtgtcagtcttagttgtaggaagtggaaacctaaaccccattactggcaccgtaagcagtgctcaggtgtttctacgttttgatgcaaacggtgttcttttaacagaacattctacactaaaaaaatactgggggtataggcagggagatagcatagatggcactccatataccaatgctgtaggattcatgcccaatttaaaagcttatccaaagtcacaaagttctactactaaaaataatatagtagggcaagtatacatgaatggagatgtttcaaaacctatgcttctcactataaccctcaatggtactgatgacagcaacagtacatattcaatgtcattttcatacacctggactaatggaagctatgttggagcaacatttggggctaactcttataccttctcatacatcgcccaagaatgaacactgtatcccaccctgcatgccaacccttcccaccccactctgtggaaaaaactctgaaacacaaaataaaataaagttcaagtgttttattgattcaacagttttacaggattcgagcagttatttttcctccaccctcccaggacatggaatacaccaccctctccccccgcacagccttgaacatctgaacgccattggtgatggacatgcttttggtctccacgttccacacagtttcagagcgagccagtctcgggtcggtcagggagatgaaaccctccgggcacaattgggagaagtactcgcctacatgggggtagagtcataatcgtgcatcaggatagggcggtggtgctgcagcagcgcgcgaataaactgctgccgccgccgctccgtcctgcaggaatacaacatggcagtggtctcctcagcgatgattcgcaccgcccgcagcataaggcgccttgtcctccgggcacagcagcgcaccctgatctcacttaaatcagcacagtaactgcagcacagcaccacaatattgttcaaaatcccacagtgcaaggcgctgtatccaaagctcatggcggggaccacagaacccacgtggccatcataccacaagcgcaggtagattaagtggcgacccctcataaacacgctggacataaacattacctcttttggcatgttgtaattcaccacctcccggtaccatataaacctctgattaaacatggcgccatccaccaccatcctaaaccagctggccaaaacctgcccgccggctatacactgcagggaaccgggactggaacaatgacagtggagagcccaggactcgtaaccatggatcatcatgctcgtcatgatatcaatgttggcacaacacaggcacacgtgcatacacttcctcaggattacaagctcctcccgcgttagaaccatatcccagggaacaacccattcctgaatcagcgtaaatcccacactgcagggaagacctcgcacgtaactcacgttgtgcattgtcaaagtgttacattcgggcagcagcggatgatcctccagtatggtagcgcgggtttctgtctcaaaaggaggtagacgatccctactgtacggagtgcgccgagacaaccgagatcgtgttggtcgtagtgtcatgccaaatggaacgccggacgtagtcatatttcctgaagtcttggcgcgccaaagtctagacagcgtccatagcttaccgagcagcagcagcagcacacaacaggcgcaagagtcagagaaaggctgagctctaacctgtccacccgctctctgctcaatatatagcccagatctacactgacgtaaaggccaaagtctaaaaatacccgccaaatagtcacacacgcccagcacacgcccagaaaccggtgacacactcaaaaaaatacgcgcacttcctcaaacgcccaaactgccgtcatttccgggttcccacgctacgtcatcaaaacacgactttcaaattccgtcgaccgttaaaaacgtcacccgccccgcccctaacggtcgcccgtctctcagccaatcagcgccccgcatccccaaattcaaacacctcatttgcatattaacgcgcaccaaaagtttgaggtatattattgatgatg

SEQ ID NO: 18 - DNA, 10 bp, Artificial Sequence
  Ribosome binding site
gccaccaugg

SEQ ID NO: 19 - DNA, 49 bp, Artificial Sequence
  Synthetic polyadenylation signal
aauaaaagaucuuuauuuucauuagaucuguguguugguuuuuugugug

SEQ ID NO: 20 - DNA, 33 bp, Artificial Sequence
  PCR Primer
tattctgcgatcgctgaggtgggtgagtgggcg

SEQ ID NO: 21 - DNA, 31 bp, Artificial Sequence
  PCR Primer
taggcgcgcccttaaacggcatttgtgggag

SEQ ID NO: 22 - DNA, 27 bp, Artificial Sequence
  PCR Primer
cgtctagaagacccgagtcttaccagt

SEQ ID NO: 23 - DNA, 39 bp, Artificial Sequence
  PCR Primer
cgggatccgtttaaaccatcatcaataatataccttatt

SEQ ID NO: 24 - DNA, 37 bp, Artificial Sequence
  PCR Primer
atggaattcgtttaaaccatcatcaataatatacctt

SEQ ID NO: 25 - DNA, 45 bp, Artificial Sequence
  PCR Primer
atgacgcgatcgctgatatcctataataataaaacgcagactttg

SEQ ID NO: 26 - DNA, 27 bp, Artificial Sequence
  PCR Primer
cgtctagacagcgtccatagcttaccg

SEQ ID NO: 27 - DNA, 40 bp, Artificial Sequence
  PCR Primer
cgggatccgtttaaaccatcatcaataatatacctcaaac

SEQ ID NO: 28 - DNA, 32 bp, Artificial Sequence
  PCR Primer
atgcgcgatcgcgtgagtagtgtttgggggtg

SEQ ID NO: 29 - DNA, 32 bp, Artificial Sequence
  PCR Primer
taggcgcgccgcttctcctcgttcaggctggc

SEQ ID NO: 30 - DNA, 41 bp, Artificial Sequence
  PCR Primer
atggaattcgtttaaaccatcatcaataatatacctcaaac

SEQ ID NO: 31 - DNA, 32 bp, Artificial Sequence
  PCR Primer
tcaagatatccgtaaaaacaccggactttgac

SEQ ID NO: 32 - DNA, 32 bp, Artificial Sequence
  PCR Primer
tgatatcccattgcatacgttgtatccatatc

SEQ ID NO: 33 - DNA, 25 bp, Artificial Sequence
  PCR Primer
tgatatctagagcccaccgcatccc